European Patent Application EP 4 692 367 A1, published February 11, 2026. Title: Method for screening compounds capable of inducing autophagy. Applicant: 国立大学法人東北大学. The sequence listing filed with the application follows.

SEQUENCE LISTING (93 sequences)

SEQ ID NO: 1 - protein, 614 aa, Homo sapiens
MSGYSSDRDRGRDRGFGAPRFGGSRAGPLSGKKFGNPGEKLVKKKWNLDELPKFEKNFYQEHPDLARRTAQEVETYRRSKEITVRGHNCPKPVLNFYEANFPANVMDVIARQNFTEPTAIQAQGWPVALSGLDMVGVAQTGSGKTLSYLLPAIVHINHQPFLERGDGPICLVLAPTRELAQQVQQVAAEYCRACRLKSTCIYGGAPKGPQIRDLERGVEICIATPGRLIDFLECGKTNLRRTTYLVLDEADRMLDMGFEPQIRKIVDQIRPDRQTLMWSATWPKEVRQLAEDFLKDYIHINIGALELSANHNILQIVDVCHDVEKDEKLIRLMEEIMSEKENKTIVFVETKRRCDELTRKMRRDGWPAMGIHGDKSQQERDWVLNEFKHGKAPILIATDVASRGLDVEDVKFVINYDYPNSSEDYIHRIGRTARSTKTGTAYTFFTPNNIKQVSDLISVLREANQAINPKLLQLVEDRGSGRSRGRGGMKDDRRDRYSAGKRGGFNTFRDRENYDRGYSSLLKRDFGAKTQNGVYSAANYTNGSFGSNFVSAGIQTSFRTGNPTGTYQNGYDSTQQYGSNVPNMHNGMNQQAYAYPATAAAPMIGYPMPTGYSQ

SEQ ID NO: 2 - DNA, 1845 bp, Homo sapiens
  source 1..1845: mol_type = genomic DNA
atgtcgggttattcgagtgaccgagaccgcggccgggaccgagggtttggtgcacctcgatttggaggaagtagggcagggcccttatctggaaagaagtttggaaaccctggggagaaattagttaaaaagaagtggaatcttgatgagctgcctaaatttgagaagaatttttatcaagagcaccctgatttggctaggcgcacagcacaagaggtggaaacatacagaagaagcaaggaaattacagttagaggtcacaactgcccgaagccagttctaaatttttatgaagccaatttccctgcaaatgtcatggatgttattgcaagacagaatttcactgaacccactgctattcaagctcagggatggccagttgctctaagtggattggatatggttggagtggcacagactggatctgggaaaacattgtcttatttgcttcctgccattgtccacatcaatcatcagccattcctagagagaggcgatgggcctatttgtttggtgctggcaccaactcgggaactggcccaacaggtgcagcaagtagctgctgaatattgtagagcatgtcgcttgaagtctacttgtatctacggtggtgctcctaagggaccacaaatacgtgatttggagagaggtgtggaaatctgtattgcaacacctggaagactgattgactttttagagtgtggaaaaaccaatctgagaagaacaacctaccttgtccttgatgaagcagatagaatgcttgatatgggctttgaaccccaaataaggaagattgtggatcaaataagacctgataggcaaactctaatgtggagtgcgacttggccaaaagaagtaagacagcttgctgaagatttcctgaaagactatattcatataaacattggtgcacttgaactgagtgcaaaccacaacattcttcagattgtggatgtgtgtcatgacgtagaaaaggatgaaaaacttattcgtctaatggaagagatcatgagtgagaaggagaataaaaccattgtttttgtggaaaccaaaagaagatgtgatgagcttaccagaaaaatgaggagagatgggtggcctgccatgggtatccatggtgacaagagtcaacaagagcgtgactgggttctaaatgaattcaaacatggaaaagctcctattctgattgctacagatgtggcctccagagggctagatgtggaagatgtgaaatttgtcatcaattatgactaccctaactcctcagaggattatattcatcgaattggaagaactgctcgcagtaccaaaacaggcacagcatacactttctttacacctaataacataaagcaagtgagcgaccttatctctgtgcttcgtgaagctaatcaagcaattaatcccaagttgcttcagttggtcgaagacagaggttcaggtcgttccaggggtagaggaggcatgaaggatgaccgtcgggacagatactctgcgggcaaaaggggtggatttaatacctttagagacagggaaaattatgacagaggttactctagcctgcttaaaagagattttggggcaaaaactcagaatggtgtttacagtgctgcaaattacaccaatgggagctttggaagtaattttgtgtctgctggtatacagaccagttttaggactggtaatccaacagggacttaccagaatggttatgatagcactcagcaatacggaagtaatgttccaaatatgcacaatggtatgaaccaacaggcatatgcatatcctgctactgcagctgcacctatgattggttatccaatgccaacaggatattcccaataa

SEQ ID NO: 3 - protein, 729 aa, Homo sapiens
MPTGFVAPILCVLLPSPTREAATVASATGDSASERESAAPAAAPTAEAPPPSVVTRPEPQALPSPAIRAPLPDLYPFGTMRGGGFGDRDRDRDRGGFGARGGGGLPPKKFGNPGERLRKKKWDLSELPKFEKNFYVEHPEVARLTPYEVDELRRKKEITVRGGDVCPKPVFAFHHANFPQYVMDVLMDQHFTEPTPIQCQGFPLALSGRDMVGIAQTGSGKTLAYLLPAIVHINHQPYLERGDGPICLVLAPTRELAQQVQQVADDYGKCSRLKSTCIYGGAPKGPQIRDLERGVEICIATPGRLIDFLESGKTNLRRCTYLVLDEADRMLDMGFEPQIRKIVDQIRPDRQTLMWSATWPKEVRQLAEDFLRDYTQINVGNLELSANHNILQIVDVCMESEKDHKLIQLMEEIMAEKENKTIIFVETKRRCDDLTRRMRRDGWPAMCIHGDKSQPERDWVLNEFRSGKAPILIATDVASRGLDVEDVKFVINYDYPNSSEDYVHRIGRTARSTNKGTAYTFFTPGNLKQARELIKVLEEANQAINPKLMQLVDHRGGGGGGGGRSRYRTTSSANNPNLMYQDECDRRLRGVKDGGRRDSASYRDRSETDRAGYANGSGYGSPNSAFGAQAGQYTYGQGTYGAAAYGTSSYTAQEYGAGTYGASSTTSTGRSSQSSSQQFSGIGRSGQQPQPLMSQQFAQPPGATNMIGYMGQTAYQYPPPPPPPPPSRK

SEQ ID NO: 4 - DNA, 2190 bp, Homo sapiens
  source 1..2190: mol_type = genomic DNA
atgcccaccggctttgtagccccgattctctgtgttttgctcccgtctccgacgagagaggcggcgacggtggcgtctgcgacgggagacagcgcgtcggagcgagagagcgctgcgcctgccgccgccccaacagcggaggcgccgccgccatcggtcgtcaccagaccggagccgcaggccctcccgagcccggccatccgtgccccgctcccagatctctatccttttgggaccatgcgcggaggaggctttggggaccgggaccgggatcgtgaccgtggaggatttggagcaagaggtggtggtggccttcccccgaagaaatttggtaatcctggggagcgtttgcgtaaaaaaaagtgggatttgagtgagctccccaagtttgagaaaaatttttatgtggaacatccggaagtagcaaggctgacaccatatgaggttgatgagctacgccgaaagaaggagattacagtgagggggggagatgtttgtcctaaacccgtgtttgccttccatcatgctaacttcccacaatatgtaatggatgtgttgatggatcagcactttacagaaccaactccaattcagtgccagggatttccgttggctcttagtggccgggatatggtgggcattgctcagactggctctgggaagacgttggcgtatctcctgcctgcaattgttcatattaaccaccagccatacttggaaaggggagatggcccaatctgtctagttctggctcctaccagagagcttgcccagcaagtacagcaggtggccgatgactatggcaaatgttctagattgaagagtacttgtatttatggaggtgctcctaaaggtccccagattcgagacttggaaagaggtgttgagatctgcatagccactcctggacgtctgatagatttcctggagtcaggaaagacaaatcttcgccgatgtacttaccttgtattggacgaagctgacagaatgcttgatatggggtttgaaccccagatccgtaaaattgttgaccaaatcaggcctgataggcagacactgatgtggagtgcaacctggccaaaagaagtaagacagcttgcagaggatttccttcgtgattacacccagatcaacgtaggcaatctggagttgagtgccaaccacaacatcctccagatagtggatgtctgcatggaaagtgaaaaagaccacaagttgatccaactaatggaagaaataatggctgaaaaggaaaacaaaacaataatatttgtggagacaaagagacgctgtgatgatctgactcgaaggatgcgcagagatggttggccagctatgtgtatccatggagacaagagtcaaccagaaagagattgggtacttaatgagttccgttctggaaaggcacccatccttattgctacagatgtagcctcccgtgggctagatgtggaagatgtcaagtttgtgatcaactatgactatccaaacagctcagaggattatgtgcaccgtattggccgaacagcccgtagcaccaacaagggtaccgcctataccttcttcaccccagggaacctaaaacaggccagagagcttatcaaagtgctggaagaggccaatcaggctatcaatccaaaactgatgcagcttgtggaccacagaggaggcggcggaggcgggggtggtcgttctcgttaccggaccacttcttcagccaacaatcccaatctgatgtatcaggatgagtgtgaccgaaggcttcgaggagtcaaggatggtggccggagagactctgcaagctatcgggatcgtagtgaaaccgatagagctggttatgctaatggcagtggctatggaagtccaaattctgcctttggagcacaagcaggccaatacacctatggtcaaggcacctatggggcagctgcttatggcaccagtagctatacagctcaagaatatggtgctggcacttatggagctagtagcaccacctcaactgggagaagttcacagagctctagccagcagtttagtgggataggccggtctgggcagcagccacagccactgatgtcacaacagtttgcacagcctccgggagctaccaatatgataggttacatggggcagactgcctaccaataccctcctcctcctccccctcctcctccttcacgtaaatga

SEQ ID NO: 5 - protein, 440 aa, Homo sapiens
MASLTVKAYLLGKEDAAREIRRFSFCCSPEPEAEAEAAAGPGPCERLLSRVAALFPALRPGGFQAHYRDEDGDLVAFSSDEELTMAMSYVKDDIFRIYIKEKKECRRDHRPPCAQEAPRNMVHPNVICDGCNGPVVGTRYKCSVCPDYDLCSVCEGKGLHRGHTKLAFPSPFGHLSEGFSHSRWLRKVKHGHFGWPGWEMGPPGNWSPRPPRAGEARPGPTAESASGPSEDPSVNFLKNVGESVAAALSPLGIEVDIDVEHGGKRSRLTPVSPESSSTEEKSSSQPSSCCSDPSKPGGNVEGATQSLAEQMRKIALESEGRPEEQMESDNCSGGDDDWTHLSSKEVDPSTGELQSLQMPESEGPSSLDPSQEGPTGLKEAALYPHLPPEADPRLIESLSQMLSMGFSDEGGWLTRLLQTKNYDIGAALDTIQYSKHPPPL

SEQ ID NO: 6 - DNA, 1323 bp, Homo sp.
  source 1..1323: mol_type = genomic DNA
atggcgtcgctcaccgtgaaggcctaccttctgggcaaggaggacgcggcgcgcgagattcgccgcttcagcttctgctgcagccccgagcctgaggcggaagccgaggctgcggcgggtccgggaccctgcgagcggctgctgagccgggtggccgccctgttccccgcgctgcggcctggcggcttccaggcgcactaccgcgatgaggacggggacttggttgccttttccagtgacgaggaattgacaatggccatgtcctacgtgaaggatgacatcttccgaatctacattaaagagaaaaaagagtgccggcgggaccaccgcccaccgtgtgctcaggaggcgccccgcaacatggtgcaccccaatgtgatctgcgatggctgcaatgggcctgtggtaggaacccgctacaagtgcagcgtctgcccagactacgacttgtgtagcgtctgcgagggaaagggcttgcaccgggggcacaccaagctcgcattccccagccccttcgggcacctgtctgagggcttctcgcacagccgctggctccggaaggtgaaacacggacacttcgggtggccaggatgggaaatgggtccaccaggaaactggagcccacgtcctcctcgtgcaggggaggcccgccctggccccacggcagaatcagcttctggtccatcggaggatccgagtgtgaatttcctgaagaacgttggggagagtgtggcagctgcccttagccctctgggcattgaagttgatatcgatgtggagcacggagggaaaagaagccgcctgacccccgtctctccagagagttccagcacagaggagaagagcagctcacagccaagcagctgctgctctgaccccagcaagccgggtgggaatgttgagggcgccacgcagtctctggcggagcagatgaggaagatcgccttggagtccgaggggcgccctgaggaacagatggagtcggataactgttcaggaggagatgatgactggacccatctgtcttcaaaagaagtggacccgtctacaggtgaactccagtccctacagatgccagaatccgaagggccaagctctctggacccctcccaggagggacccacagggctgaaggaagctgccttgtacccacatctcccgccagaggctgacccgcggctgattgagtccctctcccagatgctgtccatgggcttctctgatgaaggcggctggctcaccaggctcctgcagaccaagaactatgacatcggagcggctctggacaccatccagtattcaaagcatcccccgccgttgtag

SEQ ID NO: 7 - DNA, 14 bp, synthetic construct
  source 1..14: mol_type = other DNA
gcctccacctgctc

SEQ ID NO: 8 - DNA, 21 bp, synthetic construct
  source 1..21: mol_type = other DNA
gctagcagatcttagagtcgg

SEQ ID NO: 9 - DNA, 26 bp, synthetic construct
  source 1..26: mol_type = other DNA
agcggtaggcatggcgtcgctcaccg

SEQ ID NO: 10 - DNA, 30 bp, synthetic construct
  source 1..30: mol_type = other DNA
agaagatctgctagtacaacggcgggatgc

SEQ ID NO: 11 - DNA, 22 bp, synthetic construct
  source 1..22: mol_type = other DNA
ggtggctttaccaacagtaccg

SEQ ID NO: 12 - DNA, 21 bp, synthetic construct
  source 1..21: mol_type = other DNA
gctagcagatcttctagtcgg

SEQ ID NO: 13 - DNA, 30 bp, synthetic construct
  source 1..30: mol_type = other DNA
agcggtggcatgtcgggattcgagtgaccg

SEQ ID NO: 14 - DNA, 39 bp, synthetic construct
  source 1..39: mol_type = other DNA
agaagatctgctagcttattgggaatcctgttggcattg

SEQ ID NO: 15 - DNA, 1024 bp, synthetic construct
  source 1..1024: mol_type = other DNA
ggcctaactggccggtacctgagtctaaatgagtcttcggacctcgcgggggccgcttaagcggtggttagggtttgtctgacgcggggggagggggaaggaacgaaacactctcattcggaggcggctcggggtttggtcttggtggccacgggcacgcagaagagcgccgcgatcctcttaagcacccccccgccctccgtggaggcgggggtttggtcggcgggtggtaactggcgggccgctgactcgggcgggtcgcgcgccccagagtgtgaccttttcggtctgctcgcagacccccgggcggcgccgccgcggcggcgacgggctcgctgggtcctaggctccatggggaccgtatacgtggacaggctctggagcatccgcacgactgcggtgatattaccggagaccttctgcgggacgagccgggtcacgcggctgacgcggagcgtccgttgggcgacaaacaccaggacggggcacaggtacactatcttgtcacccggaggcgcgagggactgcaggagcttcagggagtggcgcagctgcttcatccccgtggcccgttgctcgcgtttgctggcggtgtccccggaagaaatatatttgcatgtctttagttctatgatgacacaaaccccgcccagcgtcttgtcattggcgaagtcgaacacgcagatgcagtcggggcggcgcggtcccaggtccacttcgcatattaaggtgacgcgtgtggcctcgaacaccgagcgaccctgcagcgacccgcttaaaagcttggcaatccggtactgttggtaaagccaccatggtcttcacactcgaagatttcgttggggactgggaacagacagccgcctacaacctggaccaagtccttgaacagggaggtgtgtccagtttgctgcagaatctcgccgtgtccgtaactccgatccaaaggattgtccggagcggtgaaaatgccctgaagatcgacatccatgtcatcatcccgtatgaaggtctgagcgccgac

SEQ ID NO: 16 - DNA, 1024 bp, synthetic construct
  source 1..1024: mol_type = other DNA
ggcctaactggccggtacctgagtctaaatgagtcttcggacctcgcgggggccgcttaagcggtggttagggtttgtctgacgcggggggagggggaaggaacgaaacactctcattcggaggcggctcggggtttggtcttggtggccacgggcacgcagaagagcgccgcgatcctcttaagcacccccccgccctccgtggaggcgggggtttggtcggcgggtggtaactggcgggccgctgactcgggcgggtcgcgcgccccagagtgtgaccttttcggtctgctcgcagacccccgggcggcgccgccgcggcggcgacgggctcgctgggtcctaggctccatggggaccgtatacgtggacaggctctggagcatccgcacgactgcggtgatattaccggagaccttctgcgggacgagccgggtcacgcggctgacgcggagcgtccgttgggcgacaaacaccaggacggggcacaggtacactatcttgtcacccggaggcgcgagggactgcaggagcttcagggagtggcgcagctgcttcatccccgtggcccgttgctcgcgtttgctggcggtgtccccggaagaaatatatttgcatgtctttagttctatgatgacacaaaccccgcccagcgtcttgtcattggcgaagtcgaacacgcagatgcagtcggggcggcgcggtcccaggtccacttcgcatattaaggtgacgcgtgtggcctcgaacaccgagcgaccctgcagcgacccgcttaaaagcttggcaatccggtactgttggtaaagccaccatggtgaccggctaccggctgttcgaggagattctcgggagttccggtggtggcgggagcggaggtggaggcatgtcgggttattcgagtgaccgagaccgcggccgggaccgagggtttggtgcacctcgatttggaggaagtagggcagggcccttatctggaaagaagtttggaaaccctggggagaaattagttaaaaagaagtgg

SEQ ID NO: 17 - DNA, 28 bp, synthetic construct
  source 1..28: mol_type = other DNA
cgcaaatctagacttgtacagctcgtcc

SEQ ID NO: 18 - DNA, 18 bp, synthetic construct
  source 1..18: mol_type = other DNA
ggccgcttcgagcagatg

SEQ ID NO: 19 - DNA, 31 bp, synthetic construct
  source 1..31: mol_type = other DNA
aagtctagatttgcgatgggagtgcaggtgg

SEQ ID NO: 20 - DNA, 32 bp, synthetic construct
  source 1..32: mol_type = other DNA
ctgctcgaagcggcctcattccagttagaagc

SEQ ID NO: 21 - DNA, 1024 bp, synthetic construct
  source 1..1024: mol_type = other DNA
tcaatattggccattagccatattattcattggttatatagcataaatcaatattggctattggccattgcatacgttgtatctatatcataatatgtacatttatattggctcatgtccaatatgaccgccatgttggcattgattattgactagttattaatagtaatcaattacggggtcattagttcatagcccatatatggagttccgcgttacataacttacggtaaatggcccgcctggctgaccgcccaacgacccccgcccattgacgtcaataatgacgtatgttcccatagtaacgccaatagggactttccattgacgtcaatgggtggagtatttacggtaaactgcccacttggcagtacatcaagtgtatcatatgccaagtccgccccctattgacgtcaatgacggtaaatggcccgcctggcattatgcccagtacatgaccttacgggactttcctacttggcagtacatctacgtattagtcatcgctattaccatggtgatgcggttttggcagtacaccaatgggcgtggatagcggtttgactcacggggatttccaagtctccaccccattgacgtcaatgggagtttgttttggcaccaaaatcaacgggactttccaaaatgtcgtaataaccccgccccgttgacgcaaatgggcggtaggcgtgtacggtgggaggtctatataagcagagctggtttagtgaaccgtcagatcactagaagctttattgcggtagtttatcacagttaaattgctaacgcagtcagtgcttctgacacaacagtctcgaacttaagctgcagaagttggtcgtgaggcactgggcaggtaagtatcaaggttacaagacaggtttaaggagaccaatagaaactgggcttgtcgagacagagaagactcttgcgtttctgataggcacctattggtcttactgacatccactttgcctttctctccacaggtgtccactcccagttcaattacagctcttaaggc

SEQ ID NO: 22 - DNA, 2220 bp, Homo sapiens
  source 1..2220: mol_type = genomic DNA
gcggccttctccgagatgggtgtaatgcctgagattgcacaagctgtggaagagatggattggctcctcccaactgatatccaggctgaatctatcccattgatcttaggaggaggtgatgtacttatggctgcagaaacaggaagtggcaaaactggtgcttttagtattccagttatccagatagtttatgaaactctgaaagaccaacaggaaggcaaaaaaggaaaaacaacaattaaaactggtgcttcagtgctgaacaaatggcagatgaacccatatgacagaggatctgcttttgcaattgggtcagatggtctttgttgtcaaagcagagaagtaaaggaatggcatgggtgtagagctactaaaggattaatgaaagggaaacactactatgaagtatcctgtcatgaccaagggttatgcagggtcgggtggtctaccatgcaggcctctttggacctaggtactgacaagtttggatttggctttggtggaacaggaaagaaatcccataacaaacaatttgataattatggagaggaattcactatgcatgataccattggatgttacctggatatagataagggacatgtcaagttctccaaaaatggaaaagatcttggtctggcatttgaaataccaccacatatgaaaaaccaagccctctttcctgcctgtgttttgaagaatgctgaactgaaatttaacttcggtgaagaggaatttaagtttccaccaaaagatggctttgttgctctttccaaggcaccggatggttacattgtcaaatcacagcactcaggtaatgcacaggtgacacaaacaaagtttctccccaatgctccgaaagctctcattgttgaaccttcccgggagttagctgaacaaactttgaacaacatcaagcagtttaagaaatacattgataatcctaaattaagggagcttctgataattggaggtgttgcagcccgggatcagctctctgttttggaaaatggagtagatatagttgtaggtactccgggaagactagatgacttggtgtcaactggaaagctgaacttatctcaagttagattcctggtcctggatgaagctgatgggcttctttctcaaggttattctgattttataaataggatgcacaatcagattcctcaggttacctctgatggaaaaagacttcaggtgattgtttgctctgccactttgcattctttcgatgtaaagaaactgtccgagaagataatgcattttcctacatgggttgacttaaaaggagaagactctgttccagatactgtacaccatgttgttgtcccagtaaatcccaaaactgacagactctgggaaaggcttggaaagagccacattagaactgatgatgtacatgcaaaagataacacaagacctggtgctaatagtccagagatgtggtctgaagctattaaaatcctgaaaggggagtatgctgtccgggcaatcaaggaacataagatggatcaagcaattatcttctgtagaaccaaaattgactgtgataacttggagcagtactttatacaacaaggaggaggacctgataaaaaaggacaccagttctcatgtgtttgtcttcatggtgacagaaagcctcatgagagaaagcaaaacttggaaagatttaagaaaggagatgtaagattcttgatttgcacagatgtagctgctagaggaattgatatccacggtgttccttatgttataaatgtcactctgcccgatgaaaagcaaaactacgtacatcgaattggcagagtaggaagagctgaaaggatgggtctggcaatttccctggtggcaacagaaaaagaaaaggtttggtaccatgtatgtagcagccgtggaaaagggtgttataacacaagactcaaggaagatggaggctgtaccatatggtacaacgagatgcagttactatctgagatagaagaacacctgaactgtaccatttctcaggttgagccggatataaaggtaccagtggatgaatttgatgggaaagttacctacggtcagaaaagggctgctggtggtggaagctataaaggccatgtggatattttggcacctactgttcaagagttggctgcccttgaaaaggaggcgcagacatctttcctgcatcttggctaccttcctaaccagctgttcagaaccttctga

SEQ ID NO: 23 - DNA, 1218 bp, Homo sapiens
  source 1..1218: mol_type = genomic DNA
tctgcgagccaggattcccgatccagagacaatggccccgatgggatggagcccgaaggcgtcatcgagagtaactggaatgagattgttgacagctttgatgacatgaacctctcggagtcccttctccgtggcatctacgcgtatggttttgagaagccctctgccatccagcagcgagccattctaccttgtatcaagggttatgatgtgattgctcaagcccaatctgggactgggaaaacggccacatttgccatatcgattctgcagcagattgaattagatctaaaagccacccaggccttggtcctagcacccactcgagaattggctcagcagatacagaaggtggtcatggcactaggagactacatgggcgcctcctgtcacgcctgtatcgggggcaccaacgtgcgtgctgaggtgcagaaactgcagatggaagctccccacatcatcgtgggtacccctggccgtgtgtttgatatgcttaaccggagatacctgtcccccaaatacatcaagatgtttgtactggatgaagctgacgaaatgttaagccgtggattcaaggaccagatctatgacatattccaaaagctcaacagcaacacccaggtagttttgctgtcagccacaatgccttctgatgtgcttgaggtgaccaagaagttcatgagggaccccattcggattcttgtcaagaaggaagagttgaccctggagggtatccgccagttctacatcaacgtggaacgagaggagtggaagctggacacactatgtgacttgtatgaaaccctgaccatcacccaggcagtcatcttcatcaacacccggaggaaggtggactggctcaccgagaagatgcatgctcgagatttcactgtatccgccatgcatggagatatggaccaaaaggaacgagacgtgattatgagggagtttcgttctggctctagcagagttttgattaccactgacctgctggccagaggcattgatgtgcagcaggtttctttagtcatcaactatgaccttcccaccaacagggaaaactatatccacagaatcggtcgaggtggacggtttggccgtaaaggtgtggctattaacatggtgacagaagaagacaagaggactcttcgagacattgagaccttctacaacacctccattgaggaaatgcccctcaatgttgctgacctcatctga

SEQ ID NO: 24 - DNA, 1986 bp, Homo sapiens
  source 1..1986: mol_type = genomic DNA
agtcatgtggcagtggaaaatgcgctcgggctggaccagcagtttgctggcctagacctgaactcttcagataatcagagtggaggaagtacagccagcaaagggcgctatattcctcctcatttaaggaaccgagaagctactaaaggtttctacgataaagacagttcagggtggagttctagcaaagataaggatgcgtatagcagttttggatctcgtagtgattcaagagggaagtctagcttcttcagtgatcgtggaagtggatcaaggggaaggtttgatgatcgtggacggagtgattacgatggcattggcagccgtggtgacagaagtggctttggcaaatttgaacgtggtggaaacagtcgctggtgtgacaaatcagatgaagatgattggtcaaaaccactcccaccaagtgaacgcttggaacaggaactcttttctggaggcaacactgggattaattttgagaaatacgatgacattccagttgaggcaacaggcaacaactgtcctccacatattgaaagtttcagtgatgttgagatgggagaaattatcatgggaaacattgagcttactcgttatactcgcccaactccagtgcaaaagcatgctattcctattatcaaagagaaaagagacttgatggcttgtgcccaaacagggtctggaaaaactgcagcatttctgttgcccatcttgagtcagatttattcagatggtccaggcgaggctttgagggccatgaaggaaaatggaaggtatgggcgccgcaaacaatacccaatctccttggtattagcaccaacgagagagttggcagtacagatctacgaggaagccagaaaattttcataccgatctagagttcgtccttgcgtggtttatggtggtgccgatattggtcagcagattcgagacttggaacgtggatgccatttgttagtagccactccaggacgtctagtggatatgatggaaagaggaaagattggattagacttttgcaaatacttggtgttagatgaagctgatcggatgttggatatggggtttgagcctcagattcgtagaatagtcgaacaagatactatgcctccaaagggtgtccgccacactatgatgtttagtgctacttttcctaaggaaatacagatgctggctcgtgatttcttagatgaatatatcttcttggctgtaggaagagttggctctacctctgaaaacatcacacagaaagtagtttgggtggaagaatcagacaaacggtcatttctgcttgacctcctaaatgcaacaggcaaggattcactgaccttagtgtttgtggagaccaaaaagggtgcagattctctggaggatttcttataccatgaaggatacgcatgtaccagcatccatggagaccgttctcagagggatagagaagaggcccttcaccagttccgctcaggaaaaagcccaattttagtggctacagcagtagcagcaagaggactggacatttcaaatgtgaaacatgttatcaattttgacttgccaagtgatattgaagaatatgtacatcgtattggtcgtacgggacgtgtaggaaaccttggcctggcaacctcattctttaacgagaggaacataaatattactaaggatttgttggatcttcttgttgaagctaaacaagaagtgccgtcttggttagaaaacatggcttatgaacaccactacaagggtagcagtcgtggacgttctaagagtagcagatttagtggagggtttggtgccagagactaccgacaaagtagcggtgccagcagttccagcttcagcagcagccgcgcaagcagcagccgcagtggcggaggtggccacggtagcagcagaggatttggtggaggtggctatggaggcttttacaacagtgatggatatggaggaaattataactcccagggggttgactggtggggtaactga

SEQ ID NO: 25 - DNA, 2172 bp, Homo sapiens
  source 1..2172: mol_type = genomic DNA
ggagatgaagattgggaagcagaaatcaaccctcatatgtcttcctatgttcccatatttgagaaggataggtattctggagaaaatggagacaattttaacaggactccagcttcatcatcagaaatggatgatggaccttctcgaagagatcatttcatgaaaagtggatttgcctctgggcggaattttggaaacagagatgctggtgagtgtaataagcgagataatacatccacaatgggtggttttggagttggaaagagttttggaaacagaggtttttcaaacagcaggtttgaagatggtgatagctctggtttctggagagagtctagtaatgactgcgaagataatccaacacggaacagagggttttccaagagaggcggctatcgagatggaaataattcagaagcttcagggccatacagaagaggtggaagaggtagtttccgaggttgccgtggaggatttggtctaggaagtccaaataatgacttagacccagacgaatgtatgcagcgcactggtggcctttttggttctagaagaccagtattaagtggcacaggtaatggtgatacttctcaaagcagaagtggcagtggaagtgaacgaggtggttacaaaggtttaaatgaagaagtaataacaggctctggaaagaattcttggaagtcagaagcagaaggaggagaaagtagtgatactcaaggaccaaaagtgacctacataccccctcctccacctgaggatgaggactccatctttgcacattatcagacaggcataaacttcgacaaatacgacactattcttgtggaagtgtctggacatgatgcaccaccagcaattctgacttttgaagaagctaatctctgtcagacactgaataacaacattgctaaagctggttatactaagcttactcctgtgcaaaaatacagtattcctatcatacttgcaggacgagatttgatggcttgcgctcaaacagggtctgggaagactgcggcttttctcctaccaattttggctcatatgatgcatgatggaataactgccagtcgttttaaagagttgcaggaaccagagtgtattattgtagcaccaactcgagaattggtcaaccagatttatttggaagccagaaaattttcttttgggacttgtgtaagagctgttgttatatatgggggaacccagctgggacattcaattcgacaaatagtacaaggctgtaatatattatgtgctactcctggaagactgatggatatcataggcaaagaaaagattggtctcaaacagatcaaatacttagttttggatgaagctgatcgcatgttggatatgggttttggtccagaaatgaagaagttaatttcttgcccaggaatgccatcaaaggaacagcgccaaacccttatgttcagtgcaacttttccagaggaaattcaaaggttggctgcagagtttttaaagtcaaattatctgtttgttgctgttggacaagtgggtggagcatgtagagatgttcagcagaccgttctccaagttggccagttctcaaaaagagaaaagctcgttgaaattctgcgaaacataggggatgaaagaactatggtctttgttgaaactaagaaaaaagcagattttattgcaacttttctttgtcaagaaaaaatatcaactacaagtattcatggtgatcgggaacagagagagcgggagcaagctcttggagattttcgctttggaaagtgcccagttcttgttgctacttcagtagctgccagagggctggatattgaaaatgtgcaacatgttatcaattttgatcttccttctaccattgatgaatatgttcatcgaattgggcgtactggtcgttgtgggaatactggcagagcaatttccttttttgatcttgaatcggataaccatttagcacagcctctagtaaaagtattgacagatgctcaacaggatgttcctgcatggttggaagaaattgcctttagtacatacattcctggcttcagtggtagtacaagaggaaacgtgtttgcatcagttgataccagaaagggcaagagcactttgaacacagctgggttttcttcttcacaagctcccaatccagtagatgatgagtcatgggattaa

SEQ ID NO: 26 - DNA, 1842 bp, Homo sapiens
  source 1..1842: mol_type = genomic DNA
tcgggttattcgagtgaccgagaccgcggccgggaccgagggtttggtgcacctcgatttggaggaagtagggcagggcccttatctggaaagaagtttggaaaccctggggagaaattagttaaaaagaagtggaatcttgatgagctgcctaaatttgagaagaatttttatcaagagcaccctgatttggctaggcgcacagcacaagaggtggaaacatacagaagaagcaaggaaattacagttagaggtcacaactgcccgaagccagttctaaatttttatgaagccaatttccctgcaaatgtcatggatgttattgcaagacagaatttcactgaacccactgctattcaagctcagggatggccagttgctctaagtggattggatatggttggagtggcacagactggatctgggaaaacattgtcttatttgcttcctgccattgtccacatcaatcatcagccattcctagagagaggcgatgggcctatttgtttggtgctggcaccaactcgggaactggcccaacaggtgcagcaagtagctgctgaatattgtagagcatgtcgcttgaagtctacttgtatctacggtggtgctcctaagggaccacaaatacgtgatttggagagaggtgtggaaatctgtattgcaacacctggaagactgattgactttttagagtgtggaaaaaccaatctgagaagaacaacctaccttgtccttgatgaagcagatagaatgcttgatatgggctttgaaccccaaataaggaagattgtggatcaaataagacctgataggcaaactctaatgtggagtgcgacttggccaaaagaagtaagacagcttgctgaagatttcctgaaagactatattcatataaacattggtgcacttgaactgagtgcaaaccacaacattcttcagattgtggatgtgtgtcatgacgtagaaaaggatgaaaaacttattcgtctaatggaagagatcatgagtgagaaggagaataaaaccattgtttttgtggaaaccaaaagaagatgtgatgagcttaccagaaaaatgaggagagatgggtggcctgccatgggtatccatggtgacaagagtcaacaagagcgtgactgggttctaaatgaattcaaacatggaaaagctcctattctgattgctacagatgtggcctccagagggctagatgtggaagatgtgaaatttgtcatcaattatgactaccctaactcctcagaggattatattcatcgaattggaagaactgctcgcagtaccaaaacaggcacagcatacactttctttacacctaataacataaagcaagtgagcgaccttatctctgtgcttcgtgaagctaatcaagcaattaatcccaagttgcttcagttggtcgaagacagaggttcaggtcgttccaggggtagaggaggcatgaaggatgaccgtcgggacagatactctgcgggcaaaaggggtggatttaatacctttagagacagggaaaattatgacagaggttactctagcctgcttaaaagagattttggggcaaaaactcagaatggtgtttacagtgctgcaaattacaccaatgggagctttggaagtaattttgtgtctgctggtatacagaccagttttaggactggtaatccaacagggacttaccagaatggttatgatagcactcagcaatacggaagtaatgttccaaatatgcacaatggtatgaaccaacaggcatatgcatatcctgctactgcagctgcacctatgattggttatccaatgccaacaggatattcccaataa

SEQ ID NO: 27 - DNA, 1449 bp, Homo sapiens
  source 1..1449: mol_type = genomic DNA
agcacggccagaacagagaaccctgttataatgggtctgtccagtcaaaatggtcagctgagaggccctgtgaaacccactggtggccctggaggagggggcacacagacacagcaacagatgaaccagctgaaaaacaccaacacaatcaataatggcactcagcagcaagcacagagtatgaccaccactattaaacctggtgatgactggaaaaagactttaaaactccctccaaaggatctaagaatcaaaacttcggatgtgacctccacaaaaggaaatgagtttgaagattactgtttgaaacgggagttactgatgggaatttttgaaatgggctgggaaaagccatctcctattcaggaggagagcattcccattgctttatctggtagggatatcttagctagagcaaaaaatggaacaggcaagagcggtgcctacctcattcccttacttgaacggctagacctgaagaaggacaatatacaagcaatggtgattgttcccactagagaacttgctctacaggtcagtcaaatttgcatccaggtcagcaaacacatgggaggggccaaagtgatggcaaccacaggaggaaccaatttacgagatgacataatgaggcttgatgatacagtgcacgtggtgattgctacccctgggagaatcctggatcttattaagaaaggagtagcaaaggttgatcatgtccagatgatagtattggatgaggcagataagttgctgtcacaggattttgtgcagataatggaggatattattctcacgctacctaaaaacaggcagattttactatattccgctactttccctcttagtgtacagaagttcatgaattcccatttgcagaaaccctatgagattaacctgatggaggaactaactctgaagggagtaacccagtactacgcatatgtaactgagcgccaaaaagtacactgcctcaacacacttttctccaggcttcagataaaccagtcgatcattttctgtaactcctctcagcgagttgaattgctagccaagaagatttctcaactgggttattcttgcttctatattcatgctaaaatgaggcaggaacatcgaaatcgtgtatttcatgatttccgaaatggcttatgccgcaatcttgtttgcactgatctgtttacccgaggtattgatatacaagctgtgaatgtggtaataaactttgatttcccaaagctggcagagacctatctccatcgtattggaagatcaggtcgctttggtcatcttggcttagccatcaacttgatcacatatgatgatcgcttcaacctgaaaagtattgaggagcagctgggaacagaaattaaacctattccgagcaacattgataagagcctgtatgtggcagaataccacagcgagcctgtagaagatgagaaaccttaa

SEQ ID NO: 28 - DNA, 2625 bp, Homo sapiens
  source 1..2625: mol_type = genomic DNA
ggcaaaacggccaactctccgggttcgggagcccgacccgacccggtgcggagcttcaatcgctggaagaaaaaacacagccataggcagaacaaaaagaagcagttgaggaagcaactgaagaaacccgaatggcaggtcgagcgcgagagtatcagccgcctcatgcagaactatgaaaagataaatgtaaatgaaatcacaagattttcagattttcccttgtccaaaaaaacattgaaaggtttgcaagaagctcagtaccgtttggtgactgagatacagaagcagaccattggattggctttgcaaggtaaagatgtacttggagcggccaaaactggatctggcaagactctggcttttcttgttccagtgctggaagccttatatcgtctgcaatggacttcaacagatgggctgggggttctcataatatcacctacgagagaactggcctatcagacctttgaggttctccgaaaagtaggaaagaatcatgacttctcagctggtctcatcattggtggaaaggatctaaaacacgaagctgagaggatcaacaacataaatatactcgtgtgcacaccaggtcggcttcttcaacacatggatgaaacagtatcttttcatgctaccgacctccaaatgttagttcttgatgaagcagatagaatcttggatatgggctttgctgataccatgaatgctgttattgaaaatctccccaagaaacgtcagactttacttttctcagcaacacaaactaaatctgtaaaggaccttgcacgcttgagtttgaaaaaccctgagtatgtctgggttcatgaaaaagcaaaatatagcacccctgccactttggaacagaactacatagtctgtgagctgcagcaaaaaataagtgtgctgtattcctttttgagaagccatctgaagaagaagagcattgtatttttttccagttgcaaagaggtccagtatctgtaccgagtgttttgccggctacgtcctggtgtttctatccttgcactccatggtcgacagcagcaaatgagaagaatggaagtctataatgagtttgtccgtaagagagctgcagtactctttgctactgatattgcagccaggggtctggatttcccggccgtgaattgggttcttcagtttgattgtcctgaggatgccaacacatatattcacagagcaggtagaactgccaggtacaaagaggatggtgaagctttgctaattttgctaccctcagaaaaagctatggtgcagcagcttcttcagaagaaagtacctgtgaaggaaatcaaaatcaatccagaaaaacttatagatgtccagaaaaaattggaatctattttagctcaagatcaagatttaaaagaaagagctcaaaggtgtttcgtctcctatgtacgatctgtatatctgatgaaggataaagaagtatttgatgtgagcaagttacctatacctgaatatgccctgtctcttggtcttgctgtggcaccacgcgtaagatttcttcagaaaatgcagaaacaacccaccaaagaattggtaaggagccaagccgataaagtaattgagccaagggctccctccctcaccaatgacgaagtggaagaatttagagcctacttcaatgagaaaatgtccatccttcaaaaaggtggaaaaagactcgaagggacagagcacagacaggataatgatactggtaatgaagaacaggaagaagaagaagacgatgaagaagaaatggaagagaaactggcaaaagcaaaaggatctcaagccccatctcttcctaacaccagtgaggcacagaagatcaaggaagttcctacacagttcttggacagagatgaggaggaagaagatgctgatttcttgaaggtgaagcggcataatgtgtttggattggaccttaaagacgagaaaacattacagaagaaagaaccttctaaatccagcatcaagaaaaaaatgaccaaagttgcagaagcaaaaaaagtaatgaagagaaattttaaagtgaataagaagataacatttactgatgaaggggagttggttcagcagtggccacaaatgcagaaatctgccatcaaggatgctgaggaagatgatgacacaggtggtatcaacttacataaagcaaaggaaagacttcaggaagaggacaaatttgacaaagaagaatataggaaaaaaattaaggcaaagcatcgggagaaaagactgaaagaaagggaagccagaagagaagccaacaagagacaagcaaaggccaaagatgaagaggaagcctttctggattggagtgatgatgatgatgatgatgatgatggatttgatccaagcacactcccagatccagataaatacagaagctctgaagattcagatagtgaagatatggaaaataaaataagtgataccaagaagaagcaggggatgaagaagaggagcaacagtgaagtggaagacgtgggaccaacaagtcataacagaaagaaggccaggtgggacactttagagcctttggataccggcctgtctttagcagaggatgaagagctggtgttacatctgctaagaagtcaaagctaa

SEQ ID NO: 29 - DNA, 2710 bp, Homo sapiens
  source 1..2710: mol_type = genomic DNA
gctaatgaaacacagaaggttggtgccatccattttccttttcccttcacaccctattccatccaggaagacttcatggcagagctgtaccgggttttggaggctggcaagattgggatatttgagagtccaactggcactgggaagtccttaagtcttatttgtggggccctctcttggctccgtgactttgaacagaagaagcgtgaagaagaggcacgactccttgaaactggaactggccccttacatgatgagaaagatgaatccctgtgtctgtcttcttcctgcgaaggggctgcaggcaccccgaggcctgctggagaaccggcctgggttactcagtttgtgcagaagaaagaagagagggacctggtggaccgactaaaggcggagcaggccaggaggaagcagcgagaagaacgcctgcagcagctgcagcacagggtgcagctcaagtatgcagccaagcgcctgaggcaggaagaagaagaaagagagaatctcctccgcctcagcagggagatgctagagacaggcccggaggctgagcggctggagcagctggagtctggggaggaggagctggtcctcgccgaatacgagagtgatgaggagaaaaaggtggcgagcagagtggatgaggatgaggatgacctggaggaagaacacataactaagatttattactgtagtcggacacactcccagctggcccagtttgtgcatgaggtgaagaagagcccctttggcaaggatgttcggctggtctcccttggctcccggcagaacctttgtgtaaatgaagacgtgaaaagcctaggttctgtgcagcttatcaacgaccgctgtgtggacatgcagagaagcaggcacgagaagaagaaaggagctgaggaggagaagccaaagaggaggaggcaggagaagcaggcagcctgccccttctacaaccacgagcagatgggccttctccgggatgaggccctggcagaggtgaaggacatggagcagctgctggcccttgggaaggaggcccgggcctgtccctattacgggagccgccttgccatccctgcagcccagctggtggtgctgccctatcagatgctgctgcatgcggccactcggcaggccgcgggcatccggctgcaggaccaggtggtgatcatcgacgaggcgcacaacctgatcgacaccatcacgggcatgcacagcgtggaggtcagcggctcccagctctgccaggcccattcccagctgctgcagtacgtggagcgatacgggaagcgtttgaaggccaagaacctgatgtacctgaagcagatcctgtatttgctggagaaattcgtggctgtgctaggggggaacattaagcaaaatcccaatacacagagtctgtcacagacagggacggagctgaagaccatcaacgactttctcttccagagccagatcgacaacatcaacctgttcaaggtgcagcgatactgtgagaagagcatgatcagcagaaagctctttggattcactgaacggtacggagcagtgttctcatcccgggagcagcccaaactggctgggtttcagcaattcctgcagagcctgcagcccaggacgactgaagctcttgcagcccctgcagacgagagtcaggccagcaccctgcgaccagcttctccactgatgcacatccaaggcttcctggcagctctcactacggccaaccaggacggcagggtcatcctgagccgccaaggcagcctcagtcagagcaccctgaagtttttgctcctgaatccagctgtgcactttgcccaagtggtgaaggaatgccgggcagtggtcattgcggggggtaccatgcagccggtgtctgacttccggcagcagctgctggcctgtgccggggtggaagctgagcgcgtggtggagttttcctgtggtcacgtgatccctccagacaacatcctgcccctcgtcatctgcagcgggatctccaaccagccgctggaattcacgttccagaaaagagagctgcctcagatgatggacgaggtgggtcgcattctctgtaacctgtgcggtgtggttcctggaggggtggtctgtttcttcccctcctacgagtacctgcgccaggtccatgcccactgggagaagggtggcctgctgggccgtctggctgccaggaagaagatattccaggaacctaagagcgcacaccaggtggagcaggtgctgctggcatattccaggtgcatccaggcctgtggccaggagagaggccaggtgacaggggccctgctcctctctgtggttggaggaaagatgagtgaagggatcaacttctctgacaacctaggccggtgtgtggtgatggtgggcatgcccttccccaacatcaggtctgcagagctgcaggagaagatggcctacttggatcaaaccctcagcccccggccaggcacccccagggaaggctctggtggagaacctgtgcatgaaggccgtcaaccagtccataggcagggccatcaggcaccagaaggattttgccagcgtagtgctcctggaccagcgatatgcccggccccctgtcctggccaagctgccggcctggatccgagcccgtgtggaggtcaaagctacctttggccccgccattgctgctgtgcagaagtttcaccgggagaagtcggcctcttcc

SEQ ID NO: 30 - DNA, 2187 bp, Homo sapiens
  source 1..2187: mol_type = genomic DNA
cccaccggctttgtagccccgattctctgtgttttgctcccgtctccgacgagagaggcggcgacggtggcgtctgcgacgggagacagcgcgtcggagcgagagagcgctgcgcctgccgccgccccaacagcggaggcgccgccgccatcggtcgtcaccagaccggagccgcaggccctcccgagcccggccatccgtgccccgctcccagatctctatccttttgggaccatgcgcggaggaggctttggggaccgggaccgggatcgtgaccgtggaggatttggagcaagaggtggtggtggccttcccccgaagaaatttggtaatcctggggagcgtttgcgtaaaaaaaagtgggatttgagtgagctccccaagtttgagaaaaatttttatgtggaacatccggaagtagcaaggctgacaccatatgaggttgatgagctacgccgaaagaaggagattacagtgagggggggagatgtttgtcctaaacccgtgtttgccttccatcatgctaacttcccacaatatgtaatggatgtgttgatggatcagcactttacagaaccaactccaattcagtgccagggatttccgttggctcttagtggccgggatatggtgggcattgctcagactggctctgggaagacgttggcgtatctcctgcctgcaattgttcatattaaccaccagccatacttggaaaggggagatggcccaatctgtctagttctggctcctaccagagagcttgcccagcaagtacagcaggtggccgatgactatggcaaatgttctagattgaagagtacttgtatttatggaggtgctcctaaaggtccccagattcgagacttggaaagaggtgttgagatctgcatagccactcctggacgtctgatagatttcctggagtcaggaaagacaaatcttcgccgatgtacttaccttgtattggacgaagctgacagaatgcttgatatggggtttgaaccccagatccgtaaaattgttgaccaaatcaggcctgataggcagacactgatgtggagtgcaacctggccaaaagaagtaagacagcttgcagaggatttccttcgtgattacacccagatcaacgtaggcaatctggagttgagtgccaaccacaacatcctccagatagtggatgtctgcatggaaagtgaaaaagaccacaagttgatccaactaatggaagaaataatggctgaaaaggaaaacaaaacaataatatttgtggagacaaagagacgctgtgatgatctgactcgaaggatgcgcagagatggttggccagctatgtgtatccatggagacaagagtcaaccagaaagagattgggtacttaatgagttccgttctggaaaggcacccatccttattgctacagatgtagcctcccgtgggctagatgtggaagatgtcaagtttgtgatcaactatgactatccaaacagctcagaggattatgtgcaccgtattggccgaacagcccgtagcaccaacaagggtaccgcctataccttcttcaccccagggaacctaaaacaggccagagagcttatcaaagtgctggaagaggccaatcaggctatcaatccaaaactgatgcagcttgtggaccacagaggaggcggcggaggcgggggtggtcgttctcgttaccggaccacttcttcagccaacaatcccaatctgatgtatcaggatgagtgtgaccgaaggcttcgaggagtcaaggatggtggccggagagactctgcaagctatcgggatcgtagtgaaaccgatagagctggttatgctaatggcagtggctatggaagtccaaattctgcctttggagcacaagcaggccaatacacctatggtcaaggcacctatggggcagctgcttatggcaccagtagctatacagctcaagaatatggtgctggcacttatggagctagtagcaccacctcaactgggagaagttcacagagctctagccagcagtttagtgggataggccggtctgggcagcagccacagccactgatgtcacaacagtttgcacagcctccgggagctaccaatatgataggttacatggggcagactgcctaccaataccctcctcctcctccccctcctcctccttcacgtaaatga

SEQ ID NO: 31 - DNA, 2010 bp, Homo sapiens
  source 1..2010: mol_type = genomic DNA
tcacacctgccgatgaaactcctgcgtaagaagatcgagaagcggaacctcaaattgcggcagcggaacctaaagtttcagggggcctcaaatctgaccctatcggaaactcaaaatggagatgtatctgaagaaacaatgggaagtagaaaggttaaaaaatcaaaacaaaagcccatgaatgtgggcttatcagaaactcaaaatggaggcatgtctcaagaagcagtgggaaatataaaagttacaaagtctccccagaaatccactgtattaaccaatggagaagcagcaatgcagtcttccaattcagaatcaaaaaagaaaaagaagaaaaagagaaaaatggtgaatgatgctgagcctgatacgaaaaaagcaaaaactgaaaacaaagggaaatctgaagaagaaagtgccgagactactaaagaaacagaaaataatgtggagaagccagataatgatgaagatgagagtgaggtgcccagtctgcccctgggactgacaggagcttttgaggatacttcgtttgcttctctatgtaatcttgtcaatgaaaacactctgaaggcaataaaagaaatgggttttacaaacatgactgaaattcagcataaaagtatcagaccacttctggaaggcagggatcttctagcagctgcaaaaacaggcagtggtaaaaccctggcttttctcatccctgcagttgaactcattgttaagttaaggttcatgcccaggaatggaacaggagtccttattctctcacctactagagaactagccatgcaaacctttggtgttcttaaggagctgatgactcaccacgtgcatacctatggcttgataatgggtggcagtaacagatctgctgaagcacagaaacttggtaatgggatcaacatcattgtggccacaccaggccgtctgctggaccatatgcagaataccccaggatttatgtataaaaacctgcagtgtctggttattgatgaagctgatcgtatcttggatgtggggtttgaagaggaattaaagcaaattattaaacttttgccaacacgtagacagactatgctcttttctgccacccaaactcgaaaagttgaagacctggcaaggatttctctgaaaaaggagccattgtatgttggcgttgatgatgataaagcgaatgcaacagtggatggtcttgaacagggatatgttgtttgtccttctgaaaagagattccttctgctctttacattccttaagaagaaccgaaagaagaagcttatggtcttcttttcatcttgtatgtctgtgaaataccactatgagttgctgaactacattgatttgcccgtcttggccattcatggaaagcaaaagcaaaataagcgtacaaccacattcttccagttctgcaatgcagattcgggaacactattgtgtacggatgtggcagcgagaggactagacattcctgaagtcgactggattgttcagtatgaccctccggatgaccctaaggaatatattcatcgtgtgggtagaacagccagaggcctaaatgggagagggcatgccttgctcattttgcgcccagaagaattgggttttcttcgctacttgaaacaatccaaggttccattaagtgaatttgacttttcctggtctaaaatttctgacattcagtctcagcttgagaaattgattgaaaagaattactttcttcataagtcagcccaggaagcatataagtcatacatacgagcctatgattcccattctctgaaacagatctttaatgttaataacctaaatttgcctcaggttgctctgtcatttggtttcaaggtgcctcccttcgttgatctgaacgtcaacagtaatgaaggcaagcagaaaaagcgaggaggtggtggtggatttggctaccagaaaaccaagaaagttgagaaatccaaaatctttaaacacattagcaagaaatcatctgacagcaggcagttctctcactga

SEQ ID NO: 32 - DNA, 1437 bp, Homo sapiens
  source 1..1437: mol_type = genomic DNA
gccactgactcatgggccctggcggtggacgagcaggaagctgcggctgagtcgttgagcaacttgcatcttaaggaagagaaaatcaaaccagataccaatggtgctgttgtcaagaccaatgccaatgcagagaagacagatgaagaagagaaagaggacagagctgcccagtccttactcaacaagctgatcagaagcaaccttgttgataacacaaaccaagtggaagtcctgcaacgggatccaaactcccctctgtactcggtgaagtcgtttgaagagcttcggctgaaaccacagcttctccagggagtctatgccatgggcttcaatcgaccctccaagatacaagagaacgcattacccatgatgcttgctgaacccccacagaatctgattgcccagtctcagtctggcactggtaaaacagctgcctttgtcttagccatgctcagccgagtggagccatcagacagatacccccagtgtctgtgcctctccccaacatatgagctggcgcttcaaacaggaaaagtgattgagcagatgggcaaattttacccagaactgaagcttgcctatgccgttcgaggcaataaattggaaagaggccagaagatcagtgagcagattgtcattggcacccctgggaccgtgctggactggtgctccaagctcaagttcattgatcccaagaaaatcaaggtgtttgttctggatgaggctgatgtcatgatagccactcagggccaccaagatcagagcatccgcatccagaggatgctgcccaggaactgccagatgctgcttttctccgccacctttgaagactctgtgtggaagtttgcccagaaagtggtcccagacccaaatgttatcaaactgaagcgtgaggaagagaccctggataccatcaagcagtactatgtcctgtgcagcagcagagacgagaagttccaggccttgtgtaacctctacggggccatcaccattgctcaagccatgatcttctgccatactcgcaaaacagctagttggctggcagcagagctctcaaaagaaggccaccaggtggctctgctgagtggggagatgatggtggagcagagggctgcggtgattgagcgcttccgagagggcaaagagaaggttttggtgaccaccaacgtgtgtgcccgcggcattgatgttgaacaagtgtctgtcgtcatcaactttgatcttcccgtggacaaggacgggaatcctgacaatgagacctacctgcaccggatcgggcgcacgggccgctttggcaagaggggcctggcagtgaacatggtggacagcaagcacagcatgaacatcctgaacagaatccaggagcattttaataagaagatagaaagattggacacagatgatttggacgagattgagaaaatagccaactga

SEQ ID NO: 33 - DNA, 2472 bp, Homo sapiens
  source 1..2472: mol_type = genomic DNA
gcggcggcatttgaagcctcgggagccttagcagcagtggcgactgctatgccggctgagcatgtggccgtgcaggtcccggccccagagccaacacccgggcctgtgaggatcctgcggaccgctcaggatctcagcagcccgcggacccgcacgggggatgtgctgttggcggagccggccgacttcgagtcactgctgctttcgcggccggtgctggaggggctgcgggcggccggcttcgagaggccctcgccggtgcagctcaaggccatcccgttggggcgctgcgggctcgatttaattgttcaagctaaatctggcaccgggaaaacctgtgtgttctccaccatagctttggactctcttgttcttgaaaacttaagtacccagattttgatcttggctcctacaagagaaattgctgtacagatacattctgttattacagccattggaataaaaatggaaggcttagagtgtcatgtctttattggagggaccccattatcacaagacaaaaccagacttaaaaagtgtcatattgctgttggatctcctggcagaattaagcaactcatagaacttgactacttgaacccaggcagtatacgcctctttattcttgatgaagcagataagcttttagaagaaggcagcttccaggagcaaataaattggatttattcttccttgcctgccagtaaacagatgctggcagtatcagctacttatcccgaatttttggctaatgctttgacaaagtacatgagagatcccacttttgtaagactgaattccagtgatccaagtctcataggtttgaagcagtattacaaagttgtcaattcataccctttggcacataaggtttttgaggaaaagactcagcatttacaggaactgttcagcagaattccatttaatcaagctttagtcttttctaatttgcacagcagagcacaacatttggctgatatcctttcttctaaaggctttcctgctgagtgcatttcaggcaatatgaatcagaatcagcgtcttgatgctatggctaaactgaagcactttcattgcagagtcctcatttccacagatttgacttctcgtgggattgatgctgagaaggtgaatctggttgtaaatctggatgtaccattggattgggagacatacatgcatcggattgggagagctggccgttttggtacattggggctgacagtgacctactgttgccggggagaggaagaaaatatgatgatgagaattgcccagaaatgtaatatcaaccttctccctttaccagatcccattccttctggtctgatggaagaatgtgtggattgggatgtggaagttaaagctgctgtgcatacatatggtatagcaagtgtacctaaccaacccttaaaaaagcaaattcagaaaatagagagaacccttcaaattcagaaagctcatggtgaccacatggcttcctctagaaataattctgtatctggactatcagtcaaatcaaaaaataataccaaacaaaagcttcctgtgaaaagccactcagaatgtggaatcatagaaaaagcaacgtcaccaaaagaactgggctgtgacaggcaatccgaagagcaaatgaagaattctgttcagactcccgttgaaaactccaccaacagtcagcaccaggtcaaagaagctttacctgtgtcactcccccagattccttgtctgtcttcctttaaaatccatcagccatacacgttgacttttgctgaattggtagaggattatgaacattatattaaagaggggttagagaaacctgtggaaatcatcaggcactacacaggccctggggatcagactgtgaatcctcaaaatggttttgtgagaaataaagttattgaacagagagtccctgtgttggcaagtagtagccaatctggagactctgagagtgacagtgattcttacagctcaagaacctcttcccagagcaaaggaaataagtcatacttggaaggctcttctgataatcagctgaaagactctgaatctacgcctgtggatgatcgtatttctttggaacaaccaccaaatggaagtgacacccccaatccagagaaatatcaagaatcacctggaatccagatgaagacaagacttaaagagggggctagccagagagctaagcagagccggagaaacctacccaggcggtcttccttcagattgcagactgaagcccaggaagatgattggtatgactgtcatagggaaatacgtctgagtttttctgatacctatcaggattatgaggagtactggagagcttactacagggcatggcaagaatattatgctgccgcttctcattcatattattggaatgctcagagacatccaagttggatggcagcttatcacatgaataccatttatctacaagaaatgatgcatagtaaccagtga

SEQ ID NO: 34 - DNA, 2349 bp, Homo sapiens
  source 1..2349: mol_type = genomic DNA
ccgggaaaactccgtagtgacgctggtttggaatcagacaccgcaatgaaaaaaggggagacactgcgaaagcaaaccgaggagaaagagaaaaaagagaagccaaaatctgataagactgaagagatagcagaagaggaagaaactgttttccccaaagctaaacaagttaaaaagaaagcagagccttctgaagttgacatgaattctcctaaatccaaaaaggcaaaaaagaaagaggagccatctcaaaatgacatttctcctaaaaccaaaagtttgagaaagaaaaaggagcccattgaaaagaaagtggtttcttctaaaaccaaaaaagtgacaaaaaatgaggagccttctgaggaagaaatagatgctcctaagcccaagaagatgaagaaagaaaaggaaatgaatggagaaactagagagaaaagccccaaactgaagaatggatttcctcatcctgaaccggactgtaaccccagtgaagctgccagtgaagaaagtaacagtgagatagagcaggaaatacctgtggaacaaaaagaaggcgctttctctaattttcccatatctgaagaaactattaaacttctcaaaggccgaggagtgaccttcctatttcctatacaagcaaagacattccatcatgtttacagcgggaaggacttaattgcacaggcacggacaggaactgggaagacattctcctttgccatccctttgattgagaaacttcatggggaactgcaagacaggaagagaggccgtgcccctcaggtactggttcttgcacctacaagagagttggcaaatcaagtaagcaaagacttcagtgacatcacaaaaaagctgtcagtggcttgtttttatggtggaactccctatggaggtcaatttgaacgcatgaggaatgggattgatatcctggttggaacaccaggtcgtatcaaagaccacatacagaatggcaaactagatctcaccaaacttaagcatgttgtcctggatgaagtggaccagatgttggatatgggatttgctgatcaagtggaagagattttaagtgtggcatacaagaaagattctgaagacaatccccaaacattgcttttttctgcaacttgccctcattgggtatttaatgttgccaagaaatacatgaaatctacatatgaacaggtggacctgattggtaaaaagactcagaaaacggcaataactgtggagcatctggctattaagtgccactggactcagagggcagcagttattggggatgtcatccgagtatatagtggtcatcaaggacgcactatcatcttttgtgaaaccaagaaagaagcccaggagctgtcccagaattcagctataaagcaggatgctcagtccttgcatggagacattccacagaagcaaagggaaatcaccctgaaaggttttagaaatggtagttttggagttttggtggcaaccaatgttgctgcacgtgggttagacatccctgaggttgatttggttatacaaagctctccaccaaaggatgtagagtcctacattcatcgatccgggcggacaggcagagctggaaggacgggggtgtgcatctgcttttatcagcacaaggaagaatatcagttagtacaagtggagcaaaaagcgggaattaagttcaaacgaataggtgttccttctgcaacagaaataataaaagcttccagcaaagatgccatcaggcttttggattccgtgcctcccactgccattagtcacttcaaacaatcagctgagaagctgatagaggagaagggagctgtggaagctctggcagcagcactggcccatatttcaggtgccacgtccgtagaccagcgctccttgatcaactcaaatgtgggttttgtgaccatgatcttgcagtgctcaattgaaatgccaaatattagttatgcttggaaagaacttaaagagcagctgggcgaggagattgattccaaagtgaagggaatggtttttctcaaaggaaagctgggtgtttgctttgatgtacctaccgcatcagtaacagaaatacaggagaaatggcatgattcacgacgctggcagctctctgtggccacagagcaaccagaactggaaggaccacgggaaggatatggaggcttcaggggacagcgggaaggcagtcgaggcttcaggggacagcgggacggaaacagaagattcagaggacagcgggaaggcagtagaggcccgagaggacagcgatcaggaggtggcaacaaaagtaacagatcccaaaacaaaggccagaagcggagtttcagtaaagcatttggtcaataa

SEQ ID NO: 35 - DNA, 2460 bp, Homo sapiens
  source 1..2460: mol_type = genomic DNA
gcaggagagctggctgacaaaaaggaccgtgatgcatcaccttccaaggaggaaaggaagcgatcacggactcctgacagagagcgggatagagaccgggaccggaagtcttccccatctaaagatagaaagcggcatcgttcaagggatagacgtcgaggaggcagccgttctcgctctcgttcccgttccaaatctgcagaaagagaacgacggcacaaagaacgagaacgagataaggagcgggatcggaataagaaggaccgagatcgagacaaggatgggcacagacgggacaaggaccgtaaacgatccagcttatctcctggtcgaggaaaagactttaaatctcggaaggacagagactctaagaaggatgaagaggatgaacatggtgataagaagcctaaggcccagccattatccctggaggagcttctggccaagaaaaaggctgaggaagaagctgaggctaagcccaagttcctctctaaagcagaacgagaggctgaagctctaaagcgacggcagcaggaggtggaagagcggcagaggatgcttgaagaagagaggaagaaaaggaaacagttccaagacttgggcaggaagatgttggaagatcctcaggaacgggaacgtcgggaacgcagggagaggatggaacgggagaccaatggaaatgaggatgaggaagggcggcagaagatccgggaagagaaggataagagcaaggaactgcatgccattaaggagcgttacctgggtggcatcaaaaagcggcgccgaacgagacatctcaatgaccggaaatttgtttttgagtgggatgcatctgaggacacatccattgactacaaccccctgtacaaagaacggcaccaggtgcagttgttagggcgaggcttcattgcaggcattgacctcaagcagcagaagcgagagcagtcacgtttctatggagacctaatggagaagaggcgaaccctggaagaaaaggagcaggaggaggcaagactccgcaaacttcgtaagaaggaagccaagcagcgctgggatgatcgtcattggtctcagaaaaagttagatgagatgacggacagggactggcggatcttccgtgaggactacagcatcaccaccaaaggtggcaagatccccaatcccatccgatcctggaaagactcttctctgcccccacacatcttggaggtcattgataagtgtggctacaaggaaccaacacctatacagcgtcaggcaattcccattgggctacagaatcgtgacatcattggtgtggctgagactggcagtggcaagacagcagccttcctcatccctctgctggtctggatcaccacacttcccaaaattgacaggatcgaagagtcagaccaaggcccttatgccatcatcctggctcccacccgtgagttggctcaacagattgaggaagagaccatcaagtttgggaaaccgctaggtatccgcactgtggctgtcattggtggcatctccagagaagaccagggcttcaggctgcgcatgggttgtgagattgtgattgctacccctgggcgtttgattgatgtgctggagaaccgctacctggtgctgagccgctgtacctatgtggttctggatgaggcagataggatgattgacatgggctttgagccagatgtccagaagatcctggagcacatgcctgtcagcaaccagaagccagacacggatgaggctgaggaccctgagaagatgctggccaactttgagtcgggaaaacataagtaccgccaaacagtcatgttcacggccaccatgcccccagcggtggagcgtctggccaggagctatcttcggcgacctgctgtggtgtacattggctccgcaggcaagccccatgagcgtgtggaacagaaggtcttcctcatgtcagagtcagaaaagaggaaaaagctgctggcaatcttggagcaaggctttgacccacccatcattatttttgtcaaccagaagaagggctgcgacgtgttggccaaatccctggagaagatggggtacaatgcttgcacactgcacggtggaaaaggccaggagcagcgagagtttgcgttgtccaacctcaaggctggggccaaggatattttggtggctacagatgtggctggtcgtggtattgacatccaagatgtgtctatggttgtcaactatgatatggccaaaaatattgaagattacatccaccgcattggccgcacgggacgagcaggcaagagtggggtggccatcaccttcctcacaaaagaggactctgctgtgttctacgagctgaagcaagctatcctggaaagcccagtgtcttcctgtccccccgaactagccaaccacccagatgcccagcataagccaggcaccatcctcaccaagaagcgccgggaagagaccatctttgcctga

SEQ ID NO: 36 - DNA, 2577 bp, Homo sapiens
  source 1..2577: mol_type = genomic DNA
aagttgaaggacacaaaatcaaggccaaagcagtcaagctgtggcaaatttcagacaaagggaatcaaagttgtgggaaaatggaaggaagtgaagattgacccaaatatgtttgcagatggacagatggatgacttggtgtgctttgaggaattgacagattaccagttggtctcccctgccaagaatccctccagtctcttctcaaaggaagcacccaagagaaaggcacaagctgtttcagaagaagaggaggaggaggagggaaagtctagctcaccaaagaaaaagatcaagttgaagaaaagtaaaaatgtagcaactgaaggaaccagtacccagaaagaatttgaagtgaaagatcctgagctggaggcccagggagatgacatggtttgtgatgatccggaggctggggagatgacatcagaaaacctggtccaaactgctccaaaaaagaagaaaaataaagggaaaaaagggttggagccttctcagagcactgctgccaaggtgcccaaaaaagcgaagacatggattcctgaagttcatgatcagaaagcagatgtgtcagcttggaaggacctgtttgttcccaggccggttctccgagcactcagctttctaggcttctctgcacccacaccaatccaagccctgaccttggcacctgccatccgtgacaaactggacatccttggggctgctgagacaggaagtgggaaaactcttgcctttgccatcccaatgattcatgcggtgttgcagtggcagaagaggaatgctgcccctcctccaagtaacaccgaagcaccacctggagagaccagaactgaggccggagctgagactagatcaccaggcaaggctgaagctgagtctgatgcattgcctgacgatactgtaattgagagtgaagcactgcccagtgatattgcagccgaggccagagccaagactggaggcactgtctcagaccaggcgttgctctttggtgacgatgatgctggtgaagggccttcttccctgatcagggagaaacctgttcccaaacagaatgagaatgaggaggaaaatcttgataaagagcagactggaaatctaaaacaggagttggatgacaaaagcgccacctgtaaggcatatccaaagcgtcctctgcttggactggttctgactcccactcgagagctggccgtccaggtcaaacagcacattgatgctgtggccaggtttacaggaattaaaactgctattttggttggtggaatgtccacgcagaaacagcagaggatgctgaaccgtcgtcctgagattgtggttgctactccaggccggctgtgggaattaattaaagaaaagcattatcatttgaggaaccttcggcagctcaggtgcctggtagtggatgaggctgaccggatggttgagaaaggccattttgctgagctctcacagctgctagagatgctcaatgactcccaatacaacccaaagagacaaacgcttgttttttctgccacactcaccctggtgcatcaggctcctgctcgaatccttcataagaagcacaccaagaaaatggataaaacagccaaacttgacctccttatgcagaaaattggcatgaggggcaagcccaaggtcattgacctcacaaggaatgaggccacggtggagacgctaacagagaccaagatccattgtgagactgatgagaaagacttctacttgtactacttcctgatgcagtatccaggccgcagcttagtgtttgccaacagtatctcctgcatcaaacgcctctctgggctcctcaaagtccttgatatcatgcccttgaccctgcatgcctgtatgcaccagaagcagaggctcagaaacctggagcagtttgcccgtctggaagactgtgttctcttggcaacagatgtggcagctcggggtctggatattcctaaagtccagcatgtcatccattaccaggtcccacgtacctcggagatttatgtccaccgaagtggtcgaactgctcgagctaccaatgaaggcctcagtctgatgctcattgggcctgaggatgtgatcaactttaagaagatttacaaaacgctcaagaaagatgaggatatcccactgttccccgtgcagacaaaatacatggatgtggtcaaggagcgaatccgtttagctcgacagattgagaaatctgagtatcggaacttccaggcttgcctgcacaactcttggattgagcaggcagcagctgccctggagattgagctggaagaagacatgtataagggaggaaaagctgaccagcaagaagaacgtcggagacaaaagcagatgaaggttctgaagaaggagctgcgccacctgctgtcccagccactgtttacggagagccagaaaaccaagtatcccactcagtctggcaagccgcccctgcttgtgtctgccccaagtaagagcgagtctgctttgagctgtctctccaagcagaagaagaagaagacaaagaagccgaaggagccacagccggaacagccacagccaagtacaagtgcaaattaa

SEQ ID NO: 37 - DNA, 1449 bp, Homo sapiens
  source 1..1449: mol_type = genomic DNA
gcgtcgttactgtggggaggcgacgcaggggcggcggagagcgagcggctgaacagccacttttcaaacctcagccaaccccggaagaacctttggggtattaagagtactgcagtccgaaacatagatggttctattaataacatcaatgaagatgatgaagaagatgtagtggatttggcagctaattcactcttaaacaagttaatccatcaatccttagtagaatccagtcaccgtgtggaagttttacagaaggatcccagctctccactttactcagtaaagacatttgaagagctgcggctaaaggaagagttactaaaaggaatctatgcaatgggatttaataggccatctaaaatccaagagatggctctccctatgatgctggcacatccaccccagaacctcatagcacagagccagtctggaacaggaaagacagcggcatttgtgttggcaatgttaagcagagttaatgccttggaattgttcccacagtgcctctgcctagctcctacttatgaattggctctgcaaactggccgtgtggttgagcagatgggaaaattctgtgtggatgttcaagtgatgtatgccattcgagggaatcgaattcccagaggcaccgacatcactaaacagattataattggcactcctgggactgtcctagattggtgttttaaactaaaattgattgatttgactaagattcgtgtgtttgtcctggatgaagcagatgtgatgattgacactcaaggattctcagatcatagtattcgtattcaaagagctctaccctccgaatgccaaatgctcctcttttcagcaacctttgaggactctgtgtggcactttgctgagcgaatcatccctgaccctaatgttatcaagttacgcaaagaggagctcacactgaacaacatccggcaatattacgtgctgtgtgagcacaggaaagacaaataccaagctctgtgcaacatttatggcagcatcaccattggtcaggccatcatcttctgccagactcgtcgaaacgctaagtggttgaccgtggagatgatacaggatggccaccaggtgtctttgttaagcggggagctgaccgtggagcagcgagcttccatcattcagaggtttcgggatgggaaagagaaggttctcataacaactaatgtttgtgcccgagggattgatgtgaagcaggtcacaattgttgtgaactttgatctccctgtaaaacaaggagaggagccggactatgagacctacctccaccgcatagggcggacggggcgctttgggaaaaaaggccttgccttcaacatgattgaagtagatgagctgccctcgctcatgaaaatccaggaccactttaacagcagtattaagcaactcaacgctgaagacatggatgaaattgaaaagattgactattga

SEQ ID NO: 38 - DNA, 2295 bp, Homo sapiens
  source 1..2295: mol_type = genomic DNA
cttgcggacctcggcttaatcggaaccataggcgaggatgacgaggtgccggtggagcccgagtctgactccggggacgaggaagaggaggggcccattgtgctgggcagacgacaaaaagctttggggaagaaccgcagtgctgatttcaaccctgatttcgttttcactgagaaggaggggacgtacgatggcagctgggccctggctgatgtcatgagccaactcaagaagaagagggcagccactacattagatgagaagattgagaaagttcgaaagaaaaggaaaacagaggataaagaagccaagtctgggaagttggaaaaggagaaagaagcaaaggaaggctctgaaccaaaggagcaggaagaccttcaagagaatgatgaggaaggctcagaagatgaagcctcggagactgactactcatcagctgatgagaacatcctcaccaaagcagatacactcaaagtaaaggatcggaagaagaagaagaagaaaggacaggaagcaggaggattttttgaagatgcatctcagtacgatgaaaacctctcgttccaggacatgaacctttcccgccctcttctgaaggccattacagccatgggcttcaagcagcccaccccgatccagaaggcgtgcatacctgtgggtctattggggaaggacatctgtgcctgtgcagccactgggacaggtaaaactgccgcctttgccctgcctgttttggagcgtctgatttataaaccccgccaggctccagtcacccgcgtgctggtgctagtgcccacccgagagctgggcatccaggtgcactctgtcaccagacagctggcccagttctgcaacatcaccacctgcctggctgtgggcggcttggatgtgaagtctcaggaagcagctcttcgggcagcgcctgacatcctcatcgccaccccaggccggctcatcgatcacctccacaactgcccttccttccacctgagcagcatcgaggtgctcatcctggacgaggctgacaggatgctggatgagtactttgaggagcagatgaaggagatcatccgaatgtgttcccaccaccgccagaccatgctcttctcggccaccatgacagacgaggtgaaagatctggcttctgtctccttgaagaatcctgtccggatatttgtgaacagcaacacagatgtggctcccttcctgcggcaggagttcatccggatccggcctaatcgtgaaggagaccgggaagccatcgtggcagctttgttgacgaggaccttcactgaccatgtgatgctgttcacgcaaaccaagaagcaggcccaccgcatgcacatcctcctggggctcatggggctgcaggtgggtgagctccatggcaacttgtcacagacgcagcggctggaggccctccggcgttttaaggatgaacagattgacatcctcgtggccactgatgtggcagcccgtggacttgacattgagggggtcaaaacggtaatcaacttcacaatgcctaataccatcaaacattatgtccaccgggtggggcgaacagcacgtgctggcagggctgggcgctcagtctctctggtgggagaagatgagcggaagatgctgaaggagattgtaaaagctgccaaggcccctgtgaaggccaggatacttccccaagatgtcatcctcaaattccgggacaagattgagaaaatggagaaagatgtgtatgcagttctgcagctagaggcggaggaaaaagagatgcagcagtcagaagcccagatcaatacagcaaagcggctcctggagaaggggaaggaggcagtggtccaagagcccgagaggagctggttccagaccaaagaagagaggaagaaggagaaaattgccaaagctctgcaggaatttgacttggccttaagaggaaagaagaaaaggaagaagtttatgaaggatgccaaaaaaaagggggagatgacagcagaggaaaggtctcagtttgaaatcctcaaggcgcagatgtttgctgaacggctagcgaagaggaatcgcagagccaagcgggcccgagcaatgcccgaggaggagccagtgagaggtcctgccaagaagcaaaagcaggggaagaaatctgtatttgatgaagaactcaccaacacaagcaagaaggccctgaaacagtatcgagctggcccttcctttgaagaaaggaaacagttgggcttgccccaccagagacgaggaggaaactttaaatctaaatccagatacaagaggaggaagtag

SEQ ID NO: 39 - DNA, 1620 bp, Homo sapiens
  source 1..1620: mol_type = genomic DNA
gctctaacgcggccggtgcggctcttttccctcgtgactcggttgctcctggcgccgcgacggggcctcacggtccgcagtcccgacgaacccctgccggtggtgcgcatcccagtggctctacagcggcagttggaacagcggcagagcaggcggcggaacctcccgaggccggtgctggttcgacccggaccgctgctggtttcggcgcggcggccggagttgaaccagccggcgcgcctcacactgggccgttgggagcgcgcgccgctagcctctcaaggctggaagagtcgacgcgcgcgtcgggaccacttctccatcgagcgcgcgcaacaggaggcgccagcggtgcgaaagctctcgtctaagggcagctttgctgacctgggcctggagccccgtgtgctgcacgcactacaggaggctgcgcctgaagtcgttcagcccacaaccgtgcagtctagcaccatcccctcactacttcgcggccgccatgtcgtttgcgccgcagaaaccggcagtggcaagactctcagctacctcctgccgctgcttcaacggctcttgggccagccaagcctggactcccttcctatccccgcgccccgaggcctggtccttgttccttcccgagaattggcccaacaggtgcgggctgtggcccaacccttgggccgctccttgggcctgctggtgcgggacctggagggaggccacggcatgcgtaggatcaggctgcagctgtccagacagccttcagcagatgtgcttgtggccactccaggggctctgtggaaggccctgaaaagtcgactgatcagtctggagcaactctccttcttggtgttggatgaggcagacacactgctggatgaaagcttcctggaactggtggactacatcttagagaagagccacatagcagaaggcccagctgacttggaagaccccttcaatcccaaagctcagttagtgctggtaggagccacatttcccgaaggtgtaggccagttgctgaataaagtcgccagcccagatgctgtcaccaccatcaccagctccaagctccactgtatcatgcctcatgtgaaacagacatttctgagactgaagggagcagataaggtggccgagctggtgcacatcctcaagcatcgtgacagagcagaaaggactggtccctcaggaactgttctggtgttctgtaatagctccagcactgtgaactggctgggatatattctggatgaccacaaaatccaacacctaaggttgcaggggcaaatgccagccttgatgagggtaggaatcttccagtccttccagaagagctcccgagacatacttctctgcacagacatagcctctcggggcctggacagcactggtgtggagctggttgtcaattatgatttccccccaacgctgcaagattacatccacagagcagggagagtgggccgtgtggggagcgaggtgccaggcaccgtcatcagttttgtgacccatccctgggatgtgagcctggttcagaagattgagctggcggctcgccgaaggagaagtcttccaggactagcatcctcggtgaaagagcctttgccccaagcaacctga

SEQ ID NO: 40 - DNA, 2238 bp, Homo sapiens
  source 1..2238: mol_type = genomic DNA
gcagccgccgacggttcgctcttcgacaaccccaggacgttctccagacgtcccccagcccaggcgagtcggcaagcaaaggctacgaaaagaaaataccaagcgtccagtgaggctcccccagcgaaacggaggaacgaaacttcatttctcccagccaagaaaactagtgttaaagaaactcagaggacttttaaggggaacgcacaaaaaatgttttctccaaagaagcattcggttagcacaagtgatagaaaccaggaggagagacagtgcattaagacttcatcactgtttaaaaacaaccctgacattccagaactccacagacctgtggtaaagcaggtgcaagaaaaagtgtttacttcagctgcttttcatgagctgggcctccacccacatttaatttccacaataaatacggtcttaaaaatgtctagtatgaccagtgttcagaagcaaagtattcctgtgttgctggaaggcagagatgctctcgtgagatcccagacgggctcaggtaaaactcttgcctattgcatccctgtggtccagtcccttcaagcaatggagtcaaaaatacagcgcagtgatggcccctatgccctggtgctcgtgccaacgagagagctagctctacaaagctttgacactgtccagaaactgcttaagcctttcacctggattgtgcctggagtgttaatgggaggagagaagagaaaatcagaaaaggccagactccgcaaaggaataaatatccttatctcaactcctggacgcctggtggatcatataaaatccacaaagaacattcattttagtcggctgcggtggttggtgtttgatgaagcagacagaatcttggatttgggttttgaaaaggacatcacagtgatacttaatgctgtaaatgctgaatgccaaaaacgacagaatgtcttgctatcagcgacactcacagaaggtgtaacgcggctagctgatatcagtttgcatgatccagtcagtatttctgtcctggacaagagccatgaccagttgaacccaaaggacaaagcggtccaggaggtctgtcctccaccagctggcgacaagctggacagctttgcaataccagagagtctcaagcagcatgtgactgtggttcccagcaaactgaggcttgtctgcctagcggccttcatccttcagaaatgcaagtttgaggaagaccagaagatggttgtctttttctcaagttgcgagctggtggagttccactacagcctcttcctacagaccctgctgagcagctcaggggcgccggcatcagggcagttgccatctgcctccatgcgattaaaattcctacggctgcatggcggcatggagcaggaggaaagaacagcagtgtttcaggaattttcacattccagaagaggcgtccttctttgcacggatgttgcagctcggggcttagatctccctcaagtcacgtggattgttcagtacaacgctccatcttcacctgcagaatacatccaccggattggaagaaccgcccggattggctgccatgggagcagcctgctcattttggctccttcggaggcagaatatgtcaactcgttggcttctcacaaaatcaacgtttctgagattaagatggaagatattttgtgtgttctgacaagagatgattgttttaaagggaaacgatggggagcccagaaatcccatgctgttggcccccaggaaatccgagagcgagccacagtcttgcagacggtatttgaagattacgtgcactccagtgagaggagggtctcctgggcaaagaaagctctgcagtccttcatccaagcctacgccacctaccccagggagctgaagcacatcttccacgtccgatccctccaccttgggcatgtggcgaagagcttcggactaagagatgcccccaggaatcttagtgccttgactagaaagaagaggaaagcacacgtgaaaaggcctgaccttcataagaagacccagagtaaacacagcctcgctgaaatcctacgttcggaatactcaagcggcatggaggccgacatcgccaaggtcaaaaagcaaaacgcacctggagagcctggtggccggcccctgcagcacagtctgcagccgacaccctgctttggccgtgggaaaacattaaaatggagaaaaacccaaaaaggtgtacagcgggacagcaagacttcccagaaagtttaa

SEQ ID NO: 41 - DNA, 1284 bp, Homo sapiens
  source 1..1284: mol_type = genomic DNA
gcagagaacgatgtggacaatgagctcttggactatgaagatgatgaggtggagacagcagctgggggagatggggctgaggcccctgccaagaaggatgtcaagggctcctatgtctccatccacagctctggctttcgtgacttcctgctcaagccagagttgctccgggccattgtcgactgtggctttgagcatccgtcagaagtccagcatgagtgcatccctcaggccattctgggaatggatgtcctgtgccaggccaagtcgggcatgggaaagacagcagtgtttgtcttggccacactgcaacagctggagccagttactgggcaggtgtctgtactggtgatgtgtcacactcgggagttggcttttcagatcagcaaggaatatgagcgcttctctaaatacatgcccaatgtcaaggttgctgttttttttggtggtctgtctatcaagaaggatgaagaggtgctgaagaagaactgcccgcatatcgtcgtggggactccaggccgtatcctagccctggctcgaaataagagcctcaacctcaaacacattaaacactttattttggatgaatgtgataagatgcttgaacagctcgacatgcgtcgggatgtccaggaaatttttcgcatgaccccccacgagaagcaggtcatgatgttcagtgctaccttgagcaaagagatccgtccagtctgccgcaagttcatgcaagatccaatggagatcttcgtggatgatgagacgaagttgacgctgcatgggttgcagcagtactacgtgaaactgaaggacaacgagaagaaccggaagctctttgaccttctggatgtccttgagttcaaccaggtggtgatctttgtgaagtctgtgcagcggtgcattgccttggcccagctactagtggagcagaacttcccagccattgccatccaccgtgggatgccccaggaggagaggctttctcggtatcagcagtttaaagattttcaacgacgaattcttgtggctaccaacctatttggccgaggcatggacatcgagcgggtgaacattgcttttaattatgacatgcctgaggattctgacacctacctgcatcgggtggccagagcaggccggtttggcaccaagggcttggctatcacatttgtgtccgatgagaatgatgccaagatcctcaatgatgtgcaggatcgctttgaggtcaatattagtgagctgcctgatgagatagacatctcctcctacattgaacagacacggtag

SEQ ID NO: 42 - DNA, 1866 bp, Homo sapiens
  source 1..1866: mol_type = genomic DNA
gaggagtcggaacccgaacggaagcgggctcgcaccgacgaggtgcctgccggaggaagccgctccgaggcggaagatgaggacgacgaggactacgtgccctatgtgccgttacggcagcgccggcagctactgctccagaagctgctgcagcgaagacgcaagggagctgcggaggaagagcagcaggacagcggtagtgaaccccggggagatgaggacgacatcccgctaggccctcagtccaacgtcagcctcctggatcagcaccagcaccttaaagagaaggctgaagcgcgcaaagagtctgccaaggagaagcagctgaaggaagaagagaagatcctggagagtgttgccgagggccgagcattgatgtcagtgaaggagatggctaagggcattacgtatgatgaccccatcaaaaccagctggactccaccccgttatgttctgagcatgtctgaagagcgacatgagcgcgtgcggaagaaataccacatcctggtggagggagacggtatcccaccacccatcaagagcttcaaggaaatgaagtttcctgcagccatcctgagaggcctgaagaagaaaggcattcaccacccaacacccattcagatccagggcatccccaccattctatctggccgtgacatgataggcatcgctttcacgggttcaggcaagacactggtgttcacgttgcccgtcatcatgttctgcctggaacaagagaagaggttacccttctcaaagcgcgaggggccctatggactcatcatctgcccctcgcgggagctggcccggcagacccatggcatcctggagtactactgccgcctgctgcaggaggacagctcaccactcctgcgctgcgccctctgcattgggggcatgtccgtgaaagagcagatggagaccatccgacacggtgtacacatgatggtggccaccccggggcgcctcatggatttgctgcagaagaagatggtcagcctagacatctgtcgctacctggccctggacgaggctgaccgcatgatcgacatgggcttcgagggtgacatccgtaccatcttctcctacttcaagggccagcgacagaccctgctcttcagtgccaccatgccgaagaagattcagaactttgctaagagtgcccttgtaaagcctgtgaccatcaatgtggggcgcgctggggctgccagcctggatgtcatccaggaggtagaatatgtgaaggaggaggccaagatggtgtacctgctcgagtgcctgcagaagacacccccgcctgtactcatctttgcagagaagaaggcagacgtggacgccatccacgagtacctgctgctcaagggggttgaggccgtagccatccatgggggcaaagaccaggaggaacggactaaggccatcgaggcattccgggagggcaagaaggatgtcctagtagccacagacgttgcctccaagggcctggacttccctgccatccagcacgtcatcaattatgacatgccagaggagattgagaactatgtacaccggattggccgcaccgggcgctcgggaaacacaggcatcgccactaccttcatcaacaaagcgtgtgatgagtcagtgctgatggacctcaaagcgctgctgctagaagccaagcagaaggtgccgcccgtgctgcaggtgctgcattgcggggatgagtccatgctggacattggaggagagcgcggctgtgccttctgcgggggcctgggtcatcggatcactgactgccccaaactcgaggctatgcagaccaagcaggtcagcaacatcggtcgcaaggactacctggcccacagctccatggacttctga

SEQ ID NO: 43 - DNA, 2814 bp, Homo sapiens
  source 1..2814: mol_type = genomic DNA
aactggaataaaggtggtcctggcactaagcgaggatttggctttggaggttttgccatcagtgctgggaaaaaggaggaacccaaactcccacagcagtcccacagtgcctttggggcaaccagctcttcttctggatttggaaagtcagctccaccacagcttccttctttctacaaaattggatctaagcgggccaactttgatgaagaaaatgcctattttgaagatgaggaagaagattctagcaacgttgatttaccttacattcctgctgaaaactcaccaactcgccagcaattccattccaagccagtagattctgacagcgatgatgatcccttggaggcattcatggctgaagtggaggatcaggcagctagagacatgaagaggcttgaagaaaaggacaaggaaagaaaaaacgtaaagggtattcgagatgacattgaagaggaagatgaccaagaagcttattttcgatacatggcagaaaacccaactgctggtgtggttcaggaggaagaggaagacaatctagaatatgatagtgacggaaatccaattgcacctaccaaaaaaatcattgatcctcttccccccattgatcattcagagattgactatccaccatttgaaaaaaacttttacaatgagcatgaagagataaccaacctcactccacagcagttaatagatctccggcataagctcaatcttcgggtctctggtgctgcacctcctagaccaggaagtagctttgctcattttgggtttgacgaacaacttatgcaccagattcggaaatctgaatacacacagcccactccaatacagtgccagggtgtgcctgtggcattaagtggtagagacatgattggtattgccaaaacaggtagtgggaaaactgcagccttcatttggcccatgttgattcatataatggaccagaaggagttggaaccaggtgatggaccaattgcagtgattgtgtgtcctaccagggagctttgccagcagatccatgcagaatgtaagcggtttggaaaagcatataatcttcgatcagtggccgtatatggaggagggagtatgtgggagcaggccaaggcccttcaggagggggcagagattgttgtgtgtaccccaggtcgactgatagatcatgtgaaaaagaaagctaccaatcttcaaagagtctcttaccttgtgtttgatgaagcagatcgaatgtttgacatgggatttgagtaccaagttcgatccatagcaagtcatgttcgtcctgacaggcagactctcttatttagtgcaacttttcggaagaagattgaaaagttggccagagacatcctgatcgaccctattcgagtggtgcagggagatattggagaggcaaatgaagatgtgacacagattgtggagattctccattctggacctagtaaatggaactggcttacccggcgtctggtagaatttacctcttcagggagtgtcctcctctttgttactaaaaaagccaatgctgaagagctagcgaataaccttaaacaggagggtcataatcttgggctgctccatggggatatggatcagagtgagagaaacaaggtcatttcagactttaagaaaaaggacatcccagtcctggtggccacagatgttgcagcccgtggtctggacattccttcaattaagactgtcattaactatgatgtggcacgagacattgatacccacacgcataggattggccgcacaggaagagcgggtgagaaaggtgtggcctataccctactcactcccaaggacagcaattttgctggtgacctggtccggaacttggaaggagccaatcaacacgtttctaaggaactcctagatctggcaatgcagaatgcctggtttcggaaatctcgattcaaaggagggaaaggaaaaaagctgaacattggtggaggaggcctaggctacagggagcggcctggcctgggctctgagaacatggatcgaggaaataacaatgtaatgagcaattatgaggcctacaagccttccacaggagctatgggagatcgactaacggcaatgaaagcagctttccagtcacagtacaagagtcactttgttgcagccagtttaagtaatcagaaggctggaagttctgctgctggggcaagtgggtggactagtgcagggagcttgaattctgttccaactaactcagcacaacagggccataacagtcctgacagccccgtcaccagtgccgccaagggcatcccaggctttggcaatactggcaacatcagtggtgcccctgtgacctacccgtctgccggagcccaaggagtcaacaacacagcttcagggaataacagccgagaagggactgggggcagcaacgggaaaagagagagatatactgagaaccggggcagcagccgtcacagtcacggagagactggcaatcggcatagcgatagtccacgtcacggagatggtggtcgccatggagatggataccgccatccagaaagcagcagccgtcatactgatggccatcggcacggggagaacagacatggaggaagcgcaggccggcatggggagaaccggggtgcaaatgatggtcggaatggggaaagcaggaaagaagcttttaatcgtgagagcaagatggagcccaagatggaacccaaagtggacagcagcaagatggacaaggtggacagcaagacagataagacagctgacggctttgctgtcccagagccgcctaaacgcaagaaaagtcgatgggacagttag

SEQ ID NO: 44 - DNA, 1944 bp, Homo sapiens
  source 1..1944: mol_type = genomic DNA
tcccaccacggaggagctcccaaggcctctacgtgggtcgttgctagtcggcgaagctcgacagtgtcccgagcgccagagaggaggccggcggaggagttgaatcgaacaggtcctgagggatatagtgtcggcagaggtggtcgctggagaggcacctctaggcccccggaggccgtggccgctggtcacgaggaactgccgctgtgttttgctttgaagagccactttgttggcgcggtaatcggtcgtggtgggtcaaaaataaagaatatacaaagtacaacaaacaccacaatccaaataatacaagaacaaccagaatcattagtcaaaatttttggcagcaaggcaatgcaaacgaaagcaaaagcagtgatagacaattttgttaaaaagctagaagaaaattacaattcagaatgcggaattgatactgcattccaaccttctgttggaaaagatggaagcacagataacaatgttgttgcaggagatcggccattgatagattgggatcaaattagagaggaaggtttgaaatggcaaaaaacaaagtgggcagatttaccaccaattaagaaaaacttttataaagagtccactgccacaagtgccatgtcaaaagtagaagcagatagttggaggaaagaaaattttaatataacgtgggatgacttgaaggatggggagaaacgacctatccccaatcctacctgcacatttgatgacgcctttcaatgttatcctgaggttatggaaaacattaaaaaggcaggttttcaaaagccaacacctattcagtcacaggcatggcccattgtgttgcaaggaatagatcttataggagtagcccagactggaacaggaaagacattgtgttatttaatgcctggatttattcatctggtccttcaacccagccttaaaggtcaaaggaatagacccggcatgttagttctaactcccactcgggaattagcacttcaagtagaaggagaatgttgcaaatattcatataaagggcttcggagtgtttgtgtatatggtggtggaaatagagatgaacaaatagaagagcttaaaaaaggtgtagatatcataattgcaactcccggaagattgaatgatctgcaaatgagtaacttcgtcaatctgaagaatataacctacttggttttagatgaagcagacaagatgttggacatgggatttgaaccccagataatgaagattttgttagatgtgcgcccagataggcagacagttatgaccagtgctacatggcctcattcagttcatcgcctcgcacaatcttatttgaaagaaccaatgattgtctatgttggtacattggatctagttgctgtaagttcagtgaagcaaaatataattgtaaccaccgaggaagagaaatggagtcacatgcaaacttttctacagagtatgtcatccacagacaaagtcattgtcttcgtttctcgaaaagctgttgcggatcacttatcaagtgacctaatacttggaaatatatcagtagagtctctgcatggagatagagaacagagagatcgggagaaagcattagagaactttaaaacaggcaaagtgagaatactaattgcaactgatctagcctctagaggacttgatgtccatgacgttacacatgtctataattttgactttccacggaatattgaagaatacgtacaccgaatagggcgcacgggaagagcagggaggactggtgtttccattacaactttgactagaaatgattggagggttgcctctgaattgattaatattctggaaagagcaaatcagagtattccagaggagcttgtatcaatggctgagaggtttaaggcacatcaacagaaaagggaaatggaaagaaaaatggaaagacctcaaggaaggcccaagaagtttcattaa

SEQ ID NO: 45 - DNA, 3096 bp, Homo sapiens
  source 1..3096: mol_type = genomic DNA
ggtcgggagtcacgccactatcgaaaacgatcggcatcccggggtcgctctggaagtcggtctagaagtcgctcaccctcagacaaaagaagtaaacgtggagatgacagacggtctagaagtagagatagagataggaggagagagaggtctcgtagcagggataaaagaagatctcggtcaagggacaggaagcgtctgagacgttccagaagtagagagagagacagaagccgagagcgaagaagatctcgaagtagagacaggagacgctcaaggagtagaagccggggccggcgatcccgatcctccagtcctggaaataaaagcaagaaaactgagaatagatctaggtccaaagagaaaactgatggtggggaaagttctaaagagaagaaaaaagacaaagatgacaaggaggatgaaaaagaaaaagatgctggcaactttgaccagaataagctggaagaagaaatgagaaagcgaaaagaaagagtagaaaaatggcgagaagagcaacgtaaaaaggctatggaaaacataggagaactgaaaaaggaaatcgaagagatgaaacaagggaaaaagtggagtttagaggacgatgatgatgacgaagatgatcctgcagaagctgaaaaggagggaaatgaaatggagggtgaggagttagatccattagatgcttacatggaagaagtgaaagaggaagtaaaaaaatttaacatgagaagtgtaaaaggtggtgggggaaatgaaaagaagtctgggccaacggtcacaaaagttgtcactgttgtgacaaccaaaaaagcagttgtggattctgataagaagaaaggtgagctgatggagaatgaccaggatgccatggagtattcttcagaggaggaagaagttgatcttcagacagcccttacagggtatcaaacaaaacagcgaaagcttctagaaccagttgatcatggaaaaattgagtatgagccatttaggaaaaacttctatgttgaagttccagaactagcaaaaatgtctcaagaagaggtaaatgtgtttcgattggaaatggagggcattacagttaaaggaaaaggttgccccaaaccaattaaatcctgggtccagtgtggaatttccatgaagatcttaaattccctcaagaagcatggctatgaaaagcccacgcccatccaaacccaagctattcctgctataatgtctggacgagatttgattggcattgccaaaacaggaagtggaaagaccattgcttttctgttgcccatgtttagacacatcatggatcagaggtcattagaggaaggagaggggccaatagctgtcatcatgactccaactcgagaactggctttacagattactaaagagtgtaagaagttttccaagactttgggacttagagtggtctgtgtttacggaggaacaggaatcagtgagcagattgctgagctgaaaagaggtgctgaaattattgtttgcacacctggtcgaatgattgacatgttagccgctaacagtggtcgggtcacaaatcttcgaagagtgacatatgttgttttagatgaagcagacagaatgtttgacatgggttttgaaccccaggtcatgcgcatcgtggataatgttcgtcctgatcgacagacggttatgttttcagctactttccccagagctatggaggctttggctcgcaggatcctcagtaaacctattgaagtacaagttggaggcaggagtgtggtttgctcagatgtggagcaacaagtgattgtgattgaagaagaaaagaaattcttgaagttacttgagcttctaggccattatcaagagtcaggatctgtcattatatttgtggataagcaggaacatgctgatggtcttcttaaggatttaatgagagcatcttatccttgcatgtctcttcatggaggcattgatcaatatgacagagatagcatcataaatgactttaagaatgggacctgcaaacttcttgtggctacctctgttgctgcccgaggtctagatgtgaaacatctgattcttgtagtaaattatagctgccccaaccattatgaggattatgtacacagagcagggcggactggaagagcaggaaacaagggttatgcttatacttttatcacagaggatcaagctcgctatgctggtgacataattaaagctcttgaattgtcagggactgcagtacctcctgatttagagaaactgtggagtgatttcaaagatcagcagaaagctgaggggaaaataattaaaaagagtagtgggttctctggtaagggattcaagtttgatgaaacagaacaagctttggctaatgagaggaagaagttacaaaaagcagctcttggtctacaagattcagatgatgaggatgctgcagttgatattgatgagcaaattgaaagcatgtttaattcaaagaagagagtaaaggatatggctgctcctggaacatcaagtgttcctgctccaactgcaggaaatgctgagaaattagaaattgctaagagattggctcttagaatcaatgcccagaagaatttgggcatcgagtctcaggtagatgtgatgcagcaggccaccaatgcaattcttaggggtggcaccattctggctcccactgtttctgcaaaaaccattgcagaacaacttgctgaaaagatcaatgccaagctcaattatgtgccgttagagaaacaagaagaagagagacaggatggtggacagaatgaatcttttaagagatatgaagaagaattagagatcaatgacttcccacagactgctaggtggaaagttacctctaaggaagctctgcagagaatcagtgaatactctgaagccgcaattacaatcagaggaacctacttccctcctggcaaagaacccaaggaaggcgagcggaagatttacttggcaattgaaagtgccaatgaactggctgtgcagaaagcaaaggcagaaatcaccaggctcataaaagaagagctgatccggctgcaaaattcataccaaccaacaaataaaggaagatacaaagtcttatag

SEQ ID NO: 46 - DNA, 1365 bp, Homo sapiens
  source 1..1365: mol_type = genomic DNA
gcggcacccgaggaacacgattctccgaccgaagcgtcccagccgattgtggaagaggaggaaactaaaacatttaaagacctgggtgtgacagatgtgttgtgtgaagcttgtgaccagttgggatggacaaaacccaccaagatccagattgaagctattcctttggccttacaaggtcgtgatatcattgggcttgcagaaactggctctggaaagacaggcgcctttgctttgcccattctaaacgcactgctggagaccccgcagcgtttgtttgccctagttcttaccccgactcgggagctggcctttcagatctcagagcagtttgaagccctggggtcctctattggagtgcagagtgctgtgattgtaggtggaattgattcaatgtctcaatctttggcccttgcaaaaaaaccacatataataatagcaactcctggtcgactgattgaccacttggaaaatacgaaaggtttcaacttgagagctctcaaatacttggtcatggatgaagccgaccgaatactgaatatggattttgagacagaggttgacaagatcctcaaagtgattcctcgagatcggaaaacattcctcttctctgccaccatgaccaagaaggttcaaaaacttcagcgagcagctctgaagaatcctgtgaaatgtgccgtttcctctaaataccagacagttgaaaaattacagcaatattatatttttattccctctaaattcaaggatacctacctggtttatattctaaatgaattggctggaaactcctttatgatattctgcagcacctgtaataatacccagagaacagctttgctactgcgaaatcttggcttcactgccatccccctccatggacaaatgagtcagagtaagcgcctaggatcccttaataagtttaaggccaaggcccgttccattcttctagcaactgacgttgccagccgaggtttggacatacctcatgtagatgtggttgtcaactttgacattcctacccattccaaggattacatccatcgagtaggtcgaacagctagagctgggcgctccggaaaggctattacttttgtcacacagtatgatgtggaactcttccagcgcatagaacacttaattgggaagaaactaccaggttttccaacacaggatgatgaggttatgatgctgacagaacgcgtcgctgaagcccaaaggtttgcccgaatggagttaagggagcatggagaaaagaagaaacgctcgcgagaggatgctggagataatgatgacacagagggtgctattggtgtcaggaacaaggtggctggaggaaaaatgaagaagcggaaaggccgttaa

SEQ ID NO: 47 - DNA, 1233 bp, Homo sapiens
  source 1..1233: mol_type = genomic DNA
gcgaccacggccacgatggcgacctcgggctcggcgcgaaagcggctgctcaaagaggaagacatgactaaagtggaattcgagaccagcgaggaggtggatgtgacccccacgttcgacaccatgggcctgcgggaggacctgctgcggggcatctacgcttacggttttgaaaaaccatcagcaatccagcaacgagcaatcaagcagatcatcaaagggagagatgtcatcgcacagtctcagtccggcacaggaaaaacagccaccttcagtatctcagtcctccagtgtttggatattcaggttcgtgaaactcaagctttgatcttggctcccacaagagagttggctgtgcagatccagaaggggctgcttgctctcggtgactacatgaatgtccagtgccatgcctgcattggaggcaccaatgttggcgaggacatcaggaagctggattacggacagcatgttgtcgcgggcactccagggcgtgtttttgatatgattcgtcgcagaagcctaaggacacgtgctatcaaaatgttggttttggatgaagctgatgaaatgttgaataaaggtttcaaagagcagatttacgatgtatacaggtacctgcctccagccacacaggtggttctcatcagtgccacgctgccacacgagattctggagatgaccaacaagttcatgaccgacccaatccgcatcttggtgaaacgtgatgaattgactctggaaggcatcaagcaatttttcgtggcagtggagagggaagagtggaaatttgacactctgtgtgacctctacgacacactgaccatcactcaggcggtcatcttctgcaacaccaaaagaaaggtggactggctgacggagaaaatgagggaagccaacttcactgtatcctcaatgcatggagacatgccccagaaagagcgggagtccatcatgaaggagttccggtcgggcgccagccgagtgcttatttctacagatgtctgggccagggggttggatgtccctcaggtgtccctcatcattaactatgatctccctaataacagagaattgtacatacacagaattgggagatcaggtcgatacggccggaagggtgtggccattaactttgtaaagaatgacgacatccgcatcctcagagatatcgagcagtactattccactcagattgatgagatgccgatgaacgttgctgatcttatctga

SEQ ID NO: 48 - DNA, 1449 bp, Homo sapiens
  source 1..1449: mol_type = genomic DNA
gcaggcttcgcggagctcgggctgtcatcgtggctcgtggaacaatgtcggcagctgggtttgaagcagcccacgcccgtgcagctcggctgcatccccgccatcctggagggtcgagactgcttgggctgtgctaagacaggcagtgggaagacagcagcgtttgtccttcccatcttgcagaagctgtctgaggatccctatggcatcttctgcctcgtcctgacacccaccagggagctggcctaccagatcgcagagcagttccgggtcctggggaagcctctagggctgaaagactgcatcatcgtcggtggcatggacatggtggcccaggcgctggagctctctcggaaaccacacgtggtcatcgccacgccggggcgcctggcagatcacctgcgcagctccaacacttttagtataaagaagatccgcttcctggtgatggatgaggcagaccggctgctggaacagggctgcactgacttcaccgtggacctggaggccatcctggcggctgtgccggcccgcaggcagacactgctgttcagcgccacgctgaccgacacactccgggagctgcagggtctggccaccaaccagcccttcttctgggaagcacaggccccggtgagcaccgtggagcagctggaccagcgctacctgctggtgcctgagaaggtcaaggacgcctacctggtccacctgatccagcgcttccaggatgagcacgaggactggtccattatcatcttcaccaacacgtgcaagacctgccagattctgtgcatgatgctgcgcaaattcagcttccccaccgtggctctgcactccatgatgaagcagaaagaacgctttgccgccctagccaagttcaagtccagcatctaccggatcctgatcgcaacagacgtggcctcccggggcctggacatccctacggtacaggtggtcatcaaccacaacacccccgggctccccaagatctacatccaccgagtcggccggacggcccgtgcagggcggcagggtcaggccatcacgctggtgacacagtacgacatccacctggtgcacgccatcgaggagcagatcaagaagaagctggaggagttctccgtggaagaggccgaggtgctacagatcctcacacaggtcaacgtggtgcgaagagagtgtgagatcaaactggaggcggcccactttgacgaaaagaaggagatcaacaaacggaagcagctgatcctggaggggaaggaccctgacctggaggccaagcgcaaggctgagctggccaagatcaagcagaagaaccggcgcttcaaggagaaggtggaggagacgctgaagcgacagaaggctggcagggctggccacaaggggcgtccacccaggacaccgtctgggtcccactcaggcccagtcccctcccagggcctggtctga

SEQ ID NO: 49 - DNA, 2211 bp, Homo sapiens
  source 1..2211: mol_type = genomic DNA
cctgggaaactcctctggggggacattatggagctggaagcacccttggaggagtccgagagccagaagaaggagaggcaaaagagtgacagaaggaagtcaaggcaccattatgactcggatgagaaatcagaaacaagagaaaatggtgttacagatgacctggatgctcccaaggccaaaaaatctaaaatgaaagagaagctaaatggagacactgaagaaggatttaatagactttcagatgaattctccaaatctcataagtcaagaagaaaagatctaccaaatggagatatagatgaatatgaaaaaaaatcaaagcgagtatcatctttagatacttctactcataaatcaagtgataataaactagaggagaccttaacacgtgaacagaaagaaggagccttctccaattttcctatttctgaagagactataaagcttctgaaaggtcgaggggtaacatatctctttcctattcaagttaagacctttggtcctgtatatgaaggaaaagatttaatagctcaagcacggacaggaacaggaaagacattctcttttgccatccccttaattgaaagactccaaagaaatcaagaaacaattaaaaaaagccgctcaccaaaggtacttgttttggctccaacaagggaactggcaaaccaagtagccaaagacttcaaagatataactaggaaactcagcgtggcgtgtttttatggtggaacatcatatcaaagccaaattaatcatattcgaaatggtattgacatcttggttggaacacctggtcgtatcaaagaccatctgcagagtggccgattggatctttctaaactgcgacatgttgtgcttgatgaagtggatcagatgttagatttaggtttcgctgaacaagttgaagatattattcatgaatcctacaaaactgattctgaagacaatcctcagactttacttttttctgcaacttgcccacagtgggtatacaaagttgcaaaaaaatacatgaaatccagatatgaacaggttgaccttgttggaaaaatgactcaaaaggctgcaactactgtggaacatttggccatccagtgtcattggtctcagaggccagcagttattggagatgtccttcaagtctacagtgggtctgaagggagggctattattttctgtgagaccaagaagaatgtaactgaaatggccatgaatccacacataaaacagaatgcccagtgtttacatggggacattgcacagtcacaaagagaaattacactaaaaggcttcagagaaggtagttttaaagttttggtggcaaccaatgtggctgcccgtggtttggacattcctgaagttgacctggtgattcaaagttctcctcctcaggatgttgagtcctatatccatcgctctggacgcacaggtagagctggacggacagggatttgtatatgtttttatcaaccaagagaaagaggtcaactaagatatgtggaacaaaaagcaggaattacttttaaacgtgtaggtgttccttctacaatggatttagttaaatctaaaagcatggatgccatcaggtctctggcttccgtttcttacgctgctgttgattttttccgaccatcagctcagagactgatagaagagaaaggtgcagtggatgcattggctgcagctttagcccacatttctggtgcatcaagctttgaaccacgatctttgatcacctctgataaggggtttgtgaccatgactctggaaagcctagaggaaatacaggatgtcagctgtgcttggaaagaacttaacagaaagctgagtagtaatgcagtgtctcagattaccagaatgtgcctcctgaaaggaaatatgggtgtttgctttgatgttcctacaactgagtcagaaaggttacaggcagagtggcatgattccgactggatactctcagtgccagccaaattacctgaaattgaagaatattatgatggaaacacatcttctaattccagacagaggagtggctggtcaagtggtcgatcaggccggtcaggccggtcaggtggtcgatctggcggccggtcaggtagacagagtcgacaaggaagtcgctcaggaagtcgacaagatggtagaagacgaagtgggaatagaaatcgatcaagaagtgggggccacaaacggagttttgactga

SEQ ID NO: 50 - DNA, 1998 bp, Homo sapiens
  source 1..1998: mol_type = genomic DNA
gcgctgttctacgtcgcgcggtacccgggccccgatgcggcagctgcggcggggccggagggcgcggaggccggggcgcacggcagggcccgcgcgctgctcgagcggctgcagagccgggcccgcgaacggcagcagcagcgggagcccgcgcagaccgaggcggctgcatcgaccgagccggcgaccaggaggcgacggcggccccggcggcggcggcgggtgaacgacgcggagccggggagcccggaggcgccgcagggaaagcgacggaaggcggacggcgaggacgcgggcgcagaaagcaacgaggaggcgccaggggagcccagcgcagggagcagcgaggaggcgccaggggagcccagcgcagggagcagcgaggaggcgccgggggagcgcagcaccagcgccagcgccgaggcggccccagatggaccggccctggaggaggcggccggacccctggtccccggcctggtgctgggggggttcgggaagaggaaggcgccgaaggtccagcctttcctgccaaggtggctggctgagcctaactgtgtcagaaggaatgtcaccgaagacctggttcctatcgaggacatccctgacgtccatcctgacctgcagaagcagctgcgggcacacggcatctcgtcctactttccagtccaggcagctgtgattcctgccctcctggagagcgcagcctgtgggtttctggtgggcagaggtggctaccggcctagcgacctctgtgtttctgccccaacaggcagtgggaagacactggccttcgtcatccctgtggtgcaggccctgctttcgagagtggtctgccacatccgtgccctggttgtgctgcccaccaaggagctggcccagcaggtgagcaaagttttcaacatctacacagatgccacacctctgagagtctccctggttacgggacagaagtctctggccaaggagcaggagagcctcgtccagaaaacagctgatgggtaccgctgcttggctgacatcgtggtagccacccccggccgcctggtggaccacatcgaccagaccccaggattcagcctccagcagctccgcttcctgattatcgacgaggctgaccggatgattgacagcatgcatcagtcctggctgccgcgggtggtggcggccgccttccagagcgaggaccccgcggacccctgtgccctgctccagcgaaggcaggcccaggctgtgacagccgccagcacctgctgtccccagatgcccctgcagaagctgctcttctcagctactctgacccagaaccctgaaaagctgcagcagctgggcctccaccagccccggcttttctccacagggctagcacacaggggcctggaagatacagatggggacggggattcggggaagtatgcctttcctgttgggctcacgcaccactacgtgccctgcagcctcagctctaagccgctggtcgtcctgcacctggtcctggagatgggcttctcgagggttctctgcttcactaactcccgagagaactcccacaggctcttcctgctggtgcaagcttttgggggtgtggacgtggctgagttctcctcgcgctacgggcctggccagaggaggatgatcctgaagcagtttgaacaggggaagatccagctgctcatcagcacggacgccaccgcgcgaggcatcgacgtgcagggtgtggagctggtggtgaactacgacgccccccagtacctgagaacctacgtgcaccgggttgggaggacagctcgcgctgggaaaactggacaggccttcacactgctcctgaaagtgcaggagaggagattcctccgaatgctaactgaagctggggcacctgagttgcagcggcacgagctctccagcaagctgctgcagccgctggttcctcggtacgaggaggccctgtcccagctggaggagtctgtcaaggaagagcgcaagcagagggcggcctag

SEQ ID NO: 51 - DNA, 1797 bp, Homo sapiens
  source 1..1797: mol_type = genomic DNA
gacgtccacgatctctttcgccggctcggcgcgggggccaaattcgacacgagacgcttctcggcagacgcagctcgattccagataggaaaaaggaaatatgactttgattcttcggaggtgcttcagggactggacttttttggaaacaagaagtctgtcccaggtgtgtgtggagcatcacaaacacatcagaagccccaaaatggagagaaaaaagaagagagcctaactgaaaggaagagggagcagagcaagaaaaaaaggaagacgatgacttcagaaattgcttcccaagaagaaggtgctactatacagtggatgtcatctgtagaagcaaagattgaagacaaaaaagttcagagagaaagtaaactaacttccggaaagttggagaatctcagaaaagaaaagataaacttcttgcggaataaacacaaaattcacgtccaaggaaccgatcttcctgacccaattgctacatttcagcaacttgaccaggaatataaaatcaattctcgactacttcagaacattctagatgcaggtttccaaatgcctacgccaatccaaatgcaagccatcccagttatgctgcatggtcgggaacttctggcttctgctccaactggatctggaaaaacattagcttttagcattcctattttaatgcagctgaaacaacccgcaaataaaggcttcagagccctgattatatcaccaacacgagaacttgccagccagattcacagagagttaataaaaatttctgagggaacaggattcaggatacacatgatccacaaagcagcagtggcagccaagaaatttggacctaaatcatctaaaaagtttgatattcttgtgactactccaaatcgactaatctatttattaaagcaagatccccccggaatcgacctagcaagtgttgagtggcttgtagtagacgaatcagataaactgtttgaagatggcaaaactgggttcagagaccagctggcttccattttcctggcctgcacatcccacaaggtccgaagagctatgttcagtgcaacttttgcatatgatgttgaacagtggtgcaaactcaacctggacaatgtcatcagtgtgtccattggagcaaggaattctgcagtagaaactgtagaacaagagcttctctttgttggatctgagaccggaaaacttctggccatgagagaacttgttaaaaagggtttcaatccacctgttcttgtttttgttcagtccattgaaagggctaaagaactttttcatgagctcatatatgaaggtattaatgtggatgttattcatgcagagagaacacaacaacagagagataacacagtccacagtttcagagcaggaaaaatctgggttctgatttgtacagccttgctagcaagagggattgattttaaaggtgtgaacttggtgatcaactatgactttccaactagctcagtggaatatatccacaggataggtcgaactggaagagcagggaataagggaaaagcaattacatttttcactgaggatgataagccattattaagaagcgttgctaatgttatacagcaggctgggtgtcctgtaccagaatacataaaaggttttcagaaactactaagcaaacaaaagaaaaagatgattaagaaaccattggaaagggagagcattagtacaactccaaaatgtttcttagaaaaagctaaggataaacagaaaaaggtcactggtcagaacagcaagaagaaagtagctcttgaagacaaaagttaa

SEQ ID NO: 52 - DNA, 1893 bp, Homo sapiens
  source 1..1893: mol_type = genomic DNA
tcccactgggccccagagtggaagagggcggaggctaatccaagagaccttggggccagctgggatgtcaggggcagcagaggcagtggctggagtggccccttcggccatcagggaccgagagcagcaggctcccgtgaaccaccactctgctttaaaataaagaacaatatggttggtgtggtcattggttacagtggatcaaaaataaaagatctacaacattcgacaaacactaaaatacagatcataaacggggaatctgaagcaaaagtcagaatttttggcaatagggaaatgaaagcaaaggccaaagcggctatagaaacacttattagaaaacaagaaagctacaactcagaatccagtgtggataatgctgcatcccaaacccctattggaagaaatctaggcagaaatgacattgttggagaagctgagccattgtcaaattgggatcgcattagggcagcagtcgtggagtgcgaaaagagaaaatgggcagatctaccaccagttaagaaaaacttttacatagaatccaaagcaacaagctgcatgtctgaaatgcaggtgattaactggagaaaggaaaatttcaacataacgtgtgatgacttgaaaagtggtgaaaagcgtctcattccaaaaccaacttgcaggtttaaagacgcttttcagcaataccctgatcttctgaaaagcataataagggtagggattgtaaagccaacgccaattcagtcacaggcatggccaattattctacaaggaatagatcttatagtagttgcacaaaccggaacagggaaaacattgtcctatctaatgcctgggtttattcatcttgattctcaaccaatatctagagagcaaaggaatgggcctgggatgctagtccttacacccactagagagttggctcttcacgtggaagctgaatgttcaaagtattcatataaaggtctcaaaagcatttgcatatatggtggtagaaacagaaatggacaaatagaagacattagcaaaggtgtagatatcattattgcaactcctgggaggctgaatgacctacaaatgaataactctgtcaacctaagaagcataacctacttggttatagatgaggcagataaaatgctggatatggaatttgaaccccagataaggaagattttattagatgtgcgcccagaccgacagactgttatgacaagtgcaacttggccagatactgtacgtcaactagcactttcttatttgaaagatcctatgattgtttatgttggtaatctgaatctagtggctgtaaatacagtgaagcaaaatataattgttaccacagaaaaagaaaaacgagctctcacccaagaattcgtagagaacatgtcacccaacgacaaagtcatcatgtttgtcagccaaaaacatattgctgatgacttgtcaagcgacttcaatatccaaggcatatctgcagaatcattacatggcaacagtgaacagagtgatcaagagcgagcagtagaggactttaaaagcggaaacataaagatactgattacaactgatatagtatcccgaggtcttgatcttaatgatgtcacacatgtatataattatgatttcccaaggaatattgacgtatatgtacacagagtagggtacattggacggacaggaaagactggcacatcagttaccctcatcactcagagagattcgaaaatggccggtgaattgattaaaattctggacagagcaaatcagagtgttccggaagatcttgtagtaatggctgagcaatacaagttaaatcaacaaaagaggcacagagaaacacgatcaagaaaacctggacaaagacgcaaggagttttattttttaagttga

SEQ ID NO: 53 - DNA, 2643 bp, Homo sapiens
  source 1..2643: mol_type = genomic DNA
gcggccgacaagggcccggcggctggacctcggtcgcgagctgccatggcccagtggaggaagaagaaagggctccggaagcgccgaggcgcggcctcccaggcccgcggcagcgactcggaggacggcgagtttgagatccaggcggaagatgacgcccgggcccggaagctgggacctggaagacccctgcccaccttccccacctcggaatgcacctcggatgtggagccggacacccgggagatggtgcgtgcccagaacaagaagaagaagaagtctggaggcttccagtccatgggcctgagctacccggtgttcaaaggcatcatgaagaaggggtacaaggtgccaacacccatccagaggaagaccatcccggtgatcttggatggcaaggacgtggtggccatggcccggacgggcagtggcaagacagcctgcttcctcctcccaatgttcgagcggctcaagacccacagtgcccagaccggggcccgcgccctcatcctctcgccgacccgagagctggccctgcagaccctgaagttcactaaggagctaggcaagttcactggcctcaagactgccctgatcctgggtggagacaggatggaagaccagtttgcagccctgcacgaaaatcccgacataattattgccacgcccggacggttggtgcatgtggctgtggaaatgagcctgaagctgcagagtgtggaatacgtggtgttcgatgaagctgaccggctttttgaaatgggtttcgcagagcagctgcaggagatcatcgcccgcctccccgggggccaccagacggtgctgttctccgccacgctgcccaaactgctggtggaatttgcccgggctggcctcacggagcccgtgctcatccggcttgacgtggataccaagctcaacgagcagctgaagacctccttcttcctcgtgcgggaggacaccaaggctgccgtgctgctccacctgctgcacaacgtggtgcggccccaggaccagaccgtggtgtttgtggccacgaagcaccacgccgagtacctcactgagctgctgacgacccagcgggtgagctgcgcccacatctacagtgccctagacccgacagcccgcaagatcaatctcgccaaattcacgcttggcaagtgctccactctcattgtgactgacctggccgcccgaggcctggacatcccgctgctggacaatgtcatcaactacagcttccccgccaagggcaaactcttcctgcaccgcgtgggccgtgtggctcgggctggccgaagtggcacagcctactccttggtggcccctgatgaaatcccctacctgctggatctgcacctgttcctgggccgctccctcaccctcgcccgacccctcaaggagccctcaggtgtggccggtgtggatggcatgctgggtcgggtgccacagagtgtggtggacgaggaggacagtggtctgcagagcaccctggaggcatcgctggagctacggggcctggcccgcgttgctgataacgcccagcagcagtatgtgcgctcacgcccggcgccctcgcctgagtccatcaagagggccaaggagatggaccttgtggggctgggcctgcaccccctcttcagctcgcgttttgaggaggaggagctgcagcggctgaggctggtggacagcataaagaactaccgctcccgggcgactatctttgagatcaacgcctccagccgagacctgtgcagccaggtgatgcgcgccaagcggcagaaggaccgcaaggccatcgcccgcttccagcagggacagcaggggcggcaggagcagcaggagggcccagtgggcccagccccgagccgcccagcactgcaggagaagcagcctgagaaggaggaggaggaggaggcgggagagagtgtggaggacattttctcagaggtcgtgggccggaagcggcagcggtcaggacccaacaggggagccaagaggcggagggaggaggcccggcagcgggaccaggaattctacatcccctaccggcccaaggactttgacagcgagcggggcctgagcatcagcggggaagggggagcctttgagcagcaggcagctggcgctgtcctggacttgatgggggatgaagcccagaacctgacgaggggccggcagcagctcaagtgggaccgtaagaagaagcggtttgtgggacagtcaggacaggaagacaagaagaagattaagacagagagcggccgctacatcagcagctcctacaagcgagacctctatcagaagtggaaacagaaacagaaaattgatgatcgtgactcggacgaagaaggggcatctgaccggcgaggcccagagcgaagaggtgggaagcgagaccgtggccaaggtgcatcccggccccacgccccaggcacccctgcaggccgagtccgcccggaactcaagaccaagcagcagatcctgaagcagcggcgccgggcccagaagctgcacttcctgcagcgtggtggcctcaagcagctctctgcccgcaaccgccgccgcgtccaggagctgcagcagggcgccttcggccggggtgcccgctccaagaagggcaagatgcggaagaggatgtga

SEQ ID NO: 54 - DNA, 1800 bp, Homo sapiens
  source 1..1800: mol_type = genomic DNA
gagcatgtgacagagggctcctgggagtcgctgcctgtgccgctgcacccgcaggtgctgggcgcgctgcgggagctgggcttcccgtacatgacgccggtgcagtccgcaaccatccctctgttcatgcgaaacaaagatgtcgctgcagaagcggtcacaggtagtggcaaaacactcgcttttgtcatccccatcctggaaattcttctgagaagagaagagaagttaaaaaagagtcaggttggagccataatcatcacccccactcgagagctggccattcaaatagacgaggtcctgtcgcatttcacgaagcacttccccgagttcagccagattctttggatcggaggcaggaatcctggagaagatgttgagaggtttaagcaacaaggtgggaacatcattgtggccactccaggccgcttggaggacatgttccggaggaaggccgaaggcttggatctggccagctgtgtgcgatccctggatgtcctggtgttggatgaggcagacagacttctggacatggggtttgaggcaagcatcaacaccattctggagtttttgccaaagcagaggagaacaggccttttctctgccactcagacgcaggaagtggagaacctggtgagagcgggcctccggaaccctgtccgggtctcagtgaaggagaagggcgtggcagccagcagtgcccagaagaccccctcccgcctggaaaactactacatggtatgcaaggcagatgagaaatttaatcagctggtccattttcttcgcaatcataagcaggagaaacacctggtcttcttcagcacctgtgcctgtgtggaatactatgggaaggctctggaagtgctggtgaagggcgtgaagattatgtgcattcacggaaagatgaaatataaacgcaataagatcttcatggagttccgcaaattgcaaagtgggattttagtgtgcactgatgtgatggcccggggaattgatattcctgaagtcaactgggttttgcagtatgaccctcccagcaatgcaagtgccttcgtgcatcgctgcggtcgcacagctcgcattggccacgggggcagcgctctggtgttcctcctgcccatggaagagtcatacatcaatttccttgcaattaaccaaaaatgccccctgcaggagatgaagccccagagaaacacagcggaccttctgccaaaactcaagtccatggccctggctgacagagctgtgtttgaaaagggcatgaaagcttttgtgtcatatgtccaagcttatgcaaagcatgaatgcaacctgattttcagattaaaggatcttgattttgccagccttgctcgaggttttgccctgctgaggatgcccaagatgccagaattgagaggaaagcagtttccagattttgtgcccgtggacgttaataccgacacgattccatttaaagataaaatcagagaaaagcagaggcagaaactcctggagcaacaaagaagagagaaaacagaaaatgaagggagaagaaaattcataaaaaataaagcttggtcaaagcagaaggccaaaaaagaaaagaagaaaaaaatgaatgagaaaaggaaaagggaagagggttctgatattgaagatgaggacatggaagaacttcttaatgacacaagactcttgaaaaaacttaagaaaggcaaaataactgaagaagaatttgagaagggcttgttgacaactggcaaaagaacaatcaagacagtggatttagggatctcagatttggaagatgactgctga

SEQ ID NO: 55 - DNA, 1641 bp, Homo sapiens
  source 1..1641: mol_type = genomic DNA
gaggactctgaagcactgggcttcgaacacatgggcctcgatccccggctccttcaggctgtcaccgatctgggctggtcgcgacctacgctgatccaggagaaggccatcccactggccctagaagggaaggacctcctggctcgggcccgcacgggctccgggaagacggccgcttatgctattccgatgctgcagctgttgctccataggaaggcgacaggtccggtggtagaacaggcagtgagaggccttgttcttgttcctaccaaggagctggcacggcaagcacagtccatgattcagcagctggctacctactgtgctcgggatgtccgagtggccaatgtctcagctgctgaagactcagtctctcagagagctgtgctgatggagaagccagatgtggtagtagggaccccatctcgcatattaagccacttgcagcaagacagcctgaaacttcgtgactccctggagcttttggtggtggacgaagctgaccttcttttttcctttggctttgaagaagagctcaagagtctcctctgtcacttgccccggatttaccaggcttttctcatgtcagctacttttaacgaggacgtacaagcactcaaggagctgatattacataacccggttacccttaagttacaggagtcccagctgcctgggccagaccagttacagcagtttcaggtggtctgtgagactgaggaagacaaattcctcctgctgtatgccctgctcaagctgtcattgattcggggcaagtctctgctctttgtcaacactctagaacggagttaccggctacgcctgttcttggaacagttcagcatccccacctgtgtgctcaatggagagcttccactgcgctccaggtgccacatcatctcacagttcaaccaaggcttctacgactgtgtcatagcaactgatgctgaagtcctgggggccccagtcaagggcaagcgtcggggccgagggcccaaaggggacaaggcctctgatccggaagcaggtgtggcccggggcatagacttccaccatgtgtctgctgtgctcaactttgatcttcccccaacccctgaggcctacatccatcgagctggcaggacagcacgcgctaacaacccaggcatagtcttaacctttgtgcttcccacggagcagttccacttaggcaagattgaggagcttctcagtggagagaacaggggccccattctgctcccctaccagttccggatggaggagatcgagggcttccgctatcgctgcagggatgccatgcgctcagtgactaagcaggccattcgggaggcaagattgaaggagatcaaggaagagcttctgcattctgagaagcttaagacatactttgaagacaaccctagggacctccagctgctgcggcatgacctacctttgcaccccgcagtggtgaagccccacctgggccatgttcctgactacctggttcctcctgctctccgtggcctggtgcgccctcacaagaagcggaagaagctgtcttcctcttgtaggaaggccaagagagcaaagtcccagaacccactgcgcagcttcaagcacaaaggaaagaaattcagacccacagccaagccctcctga

SEQ ID NO: 56 - DNA, 2640 bp, Homo sapiens
  source 1..2640: mol_type = genomic DNA
accaccgagcagcgacgcagcctgcaagccttccaggattatatccggaagaccctggaccctacctacatcctgagctacatggccccctggtttagggagggttattctggactttatgaagccattgaaagttgggatttcaaaaaaattgaaaagttggaggagtatagattacttttaaaacgtttacaaccagaatttaaaaccagaattatcccaaccgatatcatttctgatctgtctgaatgtttaattaatcaggaatgtgaagaaattctacagatttgctctactaaggggatgatggcaggtgcagagaaattggtggaatgccttctcagatcagacaaggaaaactggcccaaaactttgaaacttgctttggagaaagaaaggaacaagttcagtgaactgtggattgtagagaaaggtataaaagatgttgaaacagaagatcttgaggataagatggaaacttctgacatacagattttctaccaagaagatccagaatgccagaatcttagtgagaattcatgtccaccttcagaagtgtctgatacaaacttgtacagcccatttaaaccaagaaattaccaattagagcttgctttgcctgctatgaaaggaaaaaacacaataatatgtgctcctacaggttgtggaaaaacctttgtttcactgcttatatgtgaacatcatcttaaaaaattcccacaaggacaaaaggggaaagttgtcttttttgcgaatcagatcccagtgtatgaacagcagaaatctgtattctcaaaatactttgaaagacatgggtatagagttacaggcatttctggagcaacagctgagaatgtcccagtggaacagattgttgagaacaatgacatcatcattttaactccacagattcttgtgaacaaccttaaaaagggaacgattccatcactatccatctttactttgatgatatttgatgaatgccacaacactagtaaacaacacccgtacaatatgatcatgtttaattatctagatcagaaacttggaggatcttcaggcccactgccccaggtcattgggctgactgcctcggttggtgttggggatgccaaaaacacagatgaagccttggattatatctgcaagctgtgtgcttctcttgatgcgtcagtgatagcaacagtcaaacacaatctggaggaactggagcaagttgtttataagccccagaagtttttcaggaaagtggaatcacggattagcgacaaatttaaatacatcatagctcagctgatgagggacacagagagtctggcaaagagaatctgcaaagacctcgaaaacttatctcaaattcaaaatagggaatttggaacacagaaatatgaacaatggattgttacagttcagaaagcatgcatggtgttccagatgccagacaaagatgaagagagcaggatttgtaaagccctgtttttatacacttcacatttgcggaaatataatgatgccctcattatcagtgagcatgcacgaatgaaagatgctctggattacttgaaagacttcttcagcaatgtccgagcagcaggattcgatgagattgagcaagatcttactcagagatttgaagaaaagctgcaggaactagaaagtgtttccagggatcccagcaatgagaatcctaaacttgaagacctctgcttcatcttacaagaagagtaccacttaaacccagagacaataacaattctctttgtgaaaaccagagcacttgtggacgctttaaaaaattggattgaaggaaatcctaaactcagttttctaaaacctggcatattgactggacgtggcaaaacaaatcagaacacaggaatgaccctcccggcacagaagtgtatattggatgcattcaaagccagtggagatcacaatattctgattgccacctcagttgctgatgaaggcattgacattgcacagtgcaatcttgtcatcctttatgagtatgtgggcaatgtcatcaaaatgatccaaaccagaggcagaggaagagcaagaggtagcaagtgcttccttctgactagtaatgctggtgtaattgaaaaagaacaaataaacatgtacaaagaaaaaatgatgaatgactctattttacgccttcagacatgggacgaagcagtatttagggaaaagattctgcatatacagactcatgaaaaattcatcagagatagtcaagaaaaaccaaaacctgtacctgataaggaaaataaaaaactgctctgcagaaagtgcaaagccttggcatgttacacagctgacgtaagagtgatagaggaatgccattacactgtgcttggagatgcttttaaggaatgctttgtgagtagaccacatcccaagccaaagcagttttcaagttttgaaaaaagagcaaagatattctgtgcccgacagaactgcagccatgactggggaatccatgtgaagtacaagacatttgagattccagttataaaaattgaaagttttgtggtggaggatattgcaactggagttcagacactgtactcgaagtggaaggactttcattttgagaagataccatttgatccagcagaaatgtccaaatga

SEQ ID NO: 57 - DNA, 1857 bp, Homo sapiens
  source 1..1857: mol_type = genomic DNA
tttgttccaagatctctaaaaatcaagaggaatgctaatgatgatggcaaaagttgtgtggctaagataattaaaccagacccagaagaccttcagttggacaaaagcagagatgttcccgttgatgctgtagctacagaagcagccacaatagacaggcacatcagcgaatcatgccctttccccagcccaggtggccagttggcagaggttcattcagtaagtcccgagcagggtgcgaaggacagccatccttctgaagagcccgttaagtcattttccaaaacacagcgctgggcagaaccaggggaacccatctgtgttgtctgtggtcgttatggagagtatatctgtgataagacagatgaagatgtgtgtagtttggagtgtaaagcgaaacatcttctacaagttaaggaaaaggaagagaaatcaaaactcagcaatccacagaaggctgattctgagccagagtctccactgaatgcttcctatgtctacaaagagcacccctttattttgaaccttcaggaagaccagattgaaaatcttaaacagcagctgggaattttagttcaagggcaagaagtcaccaggcccattattgactttgaacattgtagtctccctgaggtcttaaatcacaacttgaagaaatcaggctatgaggtgccaactcccattcaaatgcagatgattcctgtgggacttctgggaagagacattctggccagtgcagatactggctcaggaaaaacagctgcttttcttcttcctgttatcatgcgagctttattcgagagcaaaactccatctgcgctcattcttacaccaaccagagagttagccattcagatagagagacaagctaaagaattgatgagtggcctgccacgcatgaaaactgtgcttcttgtagggggcttacccttacccccacagctttatcgtctgcaacaacatgttaaggttatcatagcaacccctgggcgacttctggatataataaagcagagctctgtagaactctgtggtgtaaagattgtggtagtagatgaagctgataccatgttaaagatgggttttcaacaacaagtgcttgacattttggaaaacattcctaatgattgtcagaccattttggtttcagccacaattccaactagcatagaacagctagcaagccagcttctgcataatcctgtgagaattatcactggagaaaagaacctaccttgtgccaatgtacgtcagattattttgtgggtagaagacccagccaaaaagaaaaaattatttgaaattttaaatgataagaaactctttaagcctccagtgttagtatttgtggactgcaaactaggagcagatcttttgagtgaagccgttcagaaaatcacagggctgaaaagcatatctatacattcagagaagtcgcaaatagaaaggaaaaacatattgaagggattacttgaaggagactatgaagttgtagtgagcacaggagtcttgggacgaggcctagacttgatcagtgtcaggctggttgtcaattttgatatgccttcaagtatggatgagtatgtccatcagattggaagagtaggaagattaggtcaaaatggaacagcgattactttcatcaataataattcaaaaagactcttctgggatattgcaaaacgagtaaagcccacaggatccattcttccccctcagttattaaattccccataccttcatgaccagaagagaaaggaacaacagaaagataaacagacacagaatgatctggttacaggagctaatcttatggatattatcagaaaacatgataaaagtaattctcagaaatga

SEQ ID NO: 58 - DNA, 2209 bp, synthetic construct
  source 1..2209: mol_type = other DNA
ggcctaactggccggtacctgagtctaaatgagtcttcggacctcgcgggggccgcttaagcggtggttagggtttgtctgacgcggggggagggggaaggaacgaaacactctcattcggaggcggctcggggtttggtcttggtggccacgggcacgcagaagagcgccgcgatcctcttaagcacccccccgccctccgtggaggcgggggtttggtcggcgggtggtaactggcgggccgctgactcgggcgggtcgcgcgccccagagtgtgaccttttcggtctgctcgcagacccccgggcggcgccgccgcggcggcgacgggctcgctgggtcctaggctccatggggaccgtatacgtggacaggctctggagcatccgcacgactgcggtgatattaccggagaccttctgcgggacgagccgggtcacgcggctgacgcggagcgtccgttgggcgacaaacaccaggacggggcacaggtacactatcttgtcacccggaggcgcgagggactgcaggagcttcagggagtggcgcagctgcttcatccccgtggcccgttgctcgcgtttgctggcggtgtccccggaagaaatatatttgcatgtctttagttctatgatgacacaaaccccgcccagcgtcttgtcattggcgaagtcgaacacgcagatgcagtcggggcggcgcggtcccaggtccacttcgcatattaaggtgacgcgtgtggcctcgaacaccgagcgaccctgcagcgacccgcttaaaagcttggcaatccggtactgttggtaaagccaccatggtgaccggctaccggctgttcgaggagattctcgggagttccggtggtggcgggagcggaggtggaggcatggcgtcgctcaccgtgaaggcctaccttctgggcaaggaggacgcggcgcgcgagattcgccgcttcagcttctgctgcagccccgagcctgaggcggaagccgaggctgcggcgggtccgggaccctgcgagcggctgctgagccgggtggccgccctgttccccgcgctgcggcctggcggcttccaggcgcactaccgcgatgaggacggggacttggttgccttttccagtgacgaggaattgacaatggccatgtcctacgtgaaggatgacatcttccgaatctacattaaagagaaaaaagagtgccggcgggaccaccgcccaccgtgtgctcaggaggcgccccgcaacatggtgcaccccaatgtgatctgcgatggctgcaatgggcctgtggtaggaacccgctacaagtgcagcgtctgcccagactacgacttgtgtagcgtctgcgagggaaagggcttgcaccgggggcacaccaagctcgcattccccagccccttcgggcacctgtctgagggcttctcgcacagccgctggctccggaaggtgaaacacggacacttcgggtggccaggatgggaaatgggtccaccaggaaactggagcccacgtcctcctcgtgcaggggaggcccgccctggccccacggcagaatcagcttctggtccatcggaggatccgagtgtgaatttcctgaagaacgttggggagagtgtggcagctgcccttagccctctgggcattgaagttgatatcgatgtggagcacggagggaaaagaagccgcctgacccccgtctctccagagagttccagcacagaggagaagagcagctcacagccaagcagctgctgctctgaccccagcaagccgggtgggaatgttgagggcgccacgcagtctctggcggagcagatgaggaagatcgccttggagtccgaggggcgccctgaggaacagatggagtcggataactgttcaggaggagatgatgactggacccatctgtcttcaaaagaagtggacccgtctacaggtgaactccagtccctacagatgccagaatccgaagggccaagctctctggacccctcccaggagggacccacagggctgaaggaagctgccttgtacccacatctcccgccagaggctgacccgcggctgattgagtccctctcccagatgctgtccatgggcttctctgatgaaggcggctggctcaccaggctcctgcagaccaagaactatgacatcggagcggctctggacaccatccagtattcaaagcatcccccgccgttgtga

SEQ ID NO: 59 - DNA, 3550 bp, synthetic construct
  source 1..3550: mol_type = other DNA
ggcctaactggccggtacctgagtctaaatgagtcttcggacctcgcgggggccgcttaagcggtggttagggtttgtctgacgcggggggagggggaaggaacgaaacactctcattcggaggcggctcggggtttggtcttggtggccacgggcacgcagaagagcgccgcgatcctcttaagcacccccccgccctccgtggaggcgggggtttggtcggcgggtggtaactggcgggccgctgactcgggcgggtcgcgcgccccagagtgtgaccttttcggtctgctcgcagacccccgggcggcgccgccgcggcggcgacgggctcgctgggtcctaggctccatggggaccgtatacgtggacaggctctggagcatccgcacgactgcggtgatattaccggagaccttctgcgggacgagccgggtcacgcggctgacgcggagcgtccgttgggcgacaaacaccaggacggggcacaggtacactatcttgtcacccggaggcgcgagggactgcaggagcttcagggagtggcgcagctgcttcatccccgtggcccgttgctcgcgtttgctggcggtgtccccggaagaaatatatttgcatgtctttagttctatgatgacacaaaccccgcccagcgtcttgtcattggcgaagtcgaacacgcagatgcagtcggggcggcgcggtcccaggtccacttcgcatattaaggtgacgcgtgtggcctcgaacaccgagcgaccctgcagcgacccgcttaaaagcttggcaatccggtactgttggtaaagccaccatggtcttcacactcgaagatttcgttggggactgggaacagacagccgcctacaacctggaccaagtccttgaacagggaggtgtgtccagtttgctgcagaatctcgccgtgtccgtaactccgatccaaaggattgtccggagcggtgaaaatgccctgaagatcgacatccatgtcatcatcccgtatgaaggtctgagcgccgaccaaatggcccagatcgaagaggtgtttaaggtggtgtaccctgtggatgatcatcactttaaggtgatcctgccctatggcacactggtaatcgacggggttacgccgaacatgctgaactatttcggacggccgtatgaaggcatcgccgtgttcgacggcaaaaagatcactgtaacagggaccctgtggaacggcaacaaaattatcgacgagcgcctgatcacccccgacggctccatgctgttccgagtaaccatcaacagtgggagttccggtggtggcgggagcggaggtggaggcatggcggccttctccgagatgggtgtaatgcctgagattgcacaagctgtggaagagatggattggctcctcccaactgatatccaggctgaatctatcccattgatcttaggaggaggtgatgtacttatggctgcagaaacaggaagtggcaaaactggtgcttttagtattccagttatccagatagtttatgaaactctgaaagaccaacaggaaggcaaaaaaggaaaaacaacaattaaaactggtgcttcagtgctgaacaaatggcagatgaacccatatgacagaggatctgcttttgcaattgggtcagatggtctttgttgtcaaagcagagaagtaaaggaatggcatgggtgtagagctactaaaggattaatgaaagggaaacactactatgaagtatcctgtcatgaccaagggttatgcagggtcgggtggtctaccatgcaggcctctttggacctaggtactgacaagtttggatttggctttggtggaacaggaaagaaatcccataacaaacaatttgataattatggagaggaattcactatgcatgataccattggatgttacctggatatagataagggacatgtcaagttctccaaaaatggaaaagatcttggtctggcatttgaaataccaccacatatgaaaaaccaagccctctttcctgcctgtgttttgaagaatgctgaactgaaatttaacttcggtgaagaggaatttaagtttccaccaaaagatggctttgttgctctttccaaggcaccggatggttacattgtcaaatcacagcactcaggtaatgcacaggtgacacaaacaaagtttctccccaatgctccgaaagctctcattgttgaaccttcccgggagttagctgaacaaactttgaacaacatcaagcagtttaagaaatacattgataatcctaaattaagggagcttctgataattggaggtgttgcagcccgggatcagctctctgttttggaaaatggagtagatatagttgtaggtactccgggaagactagatgacttggtgtcaactggaaagctgaacttatctcaagttagattcctggtcctggatgaagctgatgggcttctttctcaaggttattctgattttataaataggatgcacaatcagattcctcaggttacctctgatggaaaaagacttcaggtgattgtttgctctgccactttgcattctttcgatgtaaagaaactgtccgagaagataatgcattttcctacatgggttgacttaaaaggagaagactctgttccagatactgtacaccatgttgttgtcccagtaaatcccaaaactgacagactctgggaaaggcttggaaagagccacattagaactgatgatgtacatgcaaaagataacacaagacctggtgctaatagtccagagatgtggtctgaagctattaaaatcctgaaaggggagtatgctgtccgggcaatcaaggaacataagatggatcaagcaattatcttctgtagaaccaaaattgactgtgataacttggagcagtactttatacaacaaggaggaggacctgataaaaaaggacaccagttctcatgtgtttgtcttcatggtgacagaaagcctcatgagagaaagcaaaacttggaaagatttaagaaaggagatgtaagattcttgatttgcacagatgtagctgctagaggaattgatatccacggtgttccttatgttataaatgtcactctgcccgatgaaaagcaaaactacgtacatcgaattggcagagtaggaagagctgaaaggatgggtctggcaatttccctggtggcaacagaaaaagaaaaggtttggtaccatgtatgtagcagccgtggaaaagggtgttataacacaagactcaaggaagatggaggctgtaccatatggtacaacgagatgcagttactatctgagatagaagaacacctgaactgtaccatttctcaggttgagccggatataaaggtaccagtggatgaatttgatgggaaagttacctacggtcagaaaagggctgctggtggtggaagctataaaggccatgtggatattttggcacctactgttcaagagttggctgcccttgaaaaggaggcgcagacatctttcctgcatcttggctaccttcctaaccagctgttcagaaccttctga

SEQ ID NO: 60 - DNA, 2548 bp, synthetic construct
  source 1..2548: mol_type = other DNA
ggcctaactggccggtacctgagtctaaatgagtcttcggacctcgcgggggccgcttaagcggtggttagggtttgtctgacgcggggggagggggaaggaacgaaacactctcattcggaggcggctcggggtttggtcttggtggccacgggcacgcagaagagcgccgcgatcctcttaagcacccccccgccctccgtggaggcgggggtttggtcggcgggtggtaactggcgggccgctgactcgggcgggtcgcgcgccccagagtgtgaccttttcggtctgctcgcagacccccgggcggcgccgccgcggcggcgacgggctcgctgggtcctaggctccatggggaccgtatacgtggacaggctctggagcatccgcacgactgcggtgatattaccggagaccttctgcgggacgagccgggtcacgcggctgacgcggagcgtccgttgggcgacaaacaccaggacggggcacaggtacactatcttgtcacccggaggcgcgagggactgcaggagcttcagggagtggcgcagctgcttcatccccgtggcccgttgctcgcgtttgctggcggtgtccccggaagaaatatatttgcatgtctttagttctatgatgacacaaaccccgcccagcgtcttgtcattggcgaagtcgaacacgcagatgcagtcggggcggcgcggtcccaggtccacttcgcatattaaggtgacgcgtgtggcctcgaacaccgagcgaccctgcagcgacccgcttaaaagcttggcaatccggtactgttggtaaagccaccatggtcttcacactcgaagatttcgttggggactgggaacagacagccgcctacaacctggaccaagtccttgaacagggaggtgtgtccagtttgctgcagaatctcgccgtgtccgtaactccgatccaaaggattgtccggagcggtgaaaatgccctgaagatcgacatccatgtcatcatcccgtatgaaggtctgagcgccgaccaaatggcccagatcgaagaggtgtttaaggtggtgtaccctgtggatgatcatcactttaaggtgatcctgccctatggcacactggtaatcgacggggttacgccgaacatgctgaactatttcggacggccgtatgaaggcatcgccgtgttcgacggcaaaaagatcactgtaacagggaccctgtggaacggcaacaaaattatcgacgagcgcctgatcacccccgacggctccatgctgttccgagtaaccatcaacagtgggagttccggtggtggcgggagcggaggtggaggcatgtctgcgagccaggattcccgatccagagacaatggccccgatgggatggagcccgaaggcgtcatcgagagtaactggaatgagattgttgacagctttgatgacatgaacctctcggagtcccttctccgtggcatctacgcgtatggttttgagaagccctctgccatccagcagcgagccattctaccttgtatcaagggttatgatgtgattgctcaagcccaatctgggactgggaaaacggccacatttgccatatcgattctgcagcagattgaattagatctaaaagccacccaggccttggtcctagcacccactcgagaattggctcagcagatacagaaggtggtcatggcactaggagactacatgggcgcctcctgtcacgcctgtatcgggggcaccaacgtgcgtgctgaggtgcagaaactgcagatggaagctccccacatcatcgtgggtacccctggccgtgtgtttgatatgcttaaccggagatacctgtcccccaaatacatcaagatgtttgtactggatgaagctgacgaaatgttaagccgtggattcaaggaccagatctatgacatattccaaaagctcaacagcaacacccaggtagttttgctgtcagccacaatgccttctgatgtgcttgaggtgaccaagaagttcatgagggaccccattcggattcttgtcaagaaggaagagttgaccctggagggtatccgccagttctacatcaacgtggaacgagaggagtggaagctggacacactatgtgacttgtatgaaaccctgaccatcacccaggcagtcatcttcatcaacacccggaggaaggtggactggctcaccgagaagatgcatgctcgagatttcactgtatccgccatgcatggagatatggaccaaaaggaacgagacgtgattatgagggagtttcgttctggctctagcagagttttgattaccactgacctgctggccagaggcattgatgtgcagcaggtttctttagtcatcaactatgaccttcccaccaacagggaaaactatatccacagaatcggtcgaggtggacggtttggccgtaaaggtgtggctattaacatggtgacagaagaagacaagaggactcttcgagacattgagaccttctacaacacctccattgaggaaatgcccctcaatgttgctgacctcatctga

SEQ ID NO: 61 - DNA, 3502 bp, synthetic construct
  source 1..3502: mol_type = other DNA
ggcctaactggccggtacctgagtctaaatgagtcttcggacctcgcgggggccgcttaagcggtggttagggtttgtctgacgcggggggagggggaaggaacgaaacactctcattcggaggcggctcggggtttggtcttggtggccacgggcacgcagaagagcgccgcgatcctcttaagcacccccccgccctccgtggaggcgggggtttggtcggcgggtggtaactggcgggccgctgactcgggcgggtcgcgcgccccagagtgtgaccttttcggtctgctcgcagacccccgggcggcgccgccgcggcggcgacgggctcgctgggtcctaggctccatggggaccgtatacgtggacaggctctggagcatccgcacgactgcggtgatattaccggagaccttctgcgggacgagccgggtcacgcggctgacgcggagcgtccgttgggcgacaaacaccaggacggggcacaggtacactatcttgtcacccggaggcgcgagggactgcaggagcttcagggagtggcgcagctgcttcatccccgtggcccgttgctcgcgtttgctggcggtgtccccggaagaaatatatttgcatgtctttagttctatgatgacacaaaccccgcccagcgtcttgtcattggcgaagtcgaacacgcagatgcagtcggggcggcgcggtcccaggtccacttcgcatattaaggtgacgcgtgtggcctcgaacaccgagcgaccctgcagcgacccgcttaaaagcttggcaatccggtactgttggtaaagccaccatggtcttcacactcgaagatttcgttggggactgggaacagacagccgcctacaacctggaccaagtccttgaacagggaggtgtgtccagtttgctgcagaatctcgccgtgtccgtaactccgatccaaaggattgtccggagcggtgaaaatgccctgaagatcgacatccatgtcatcatcccgtatgaaggtctgagcgccgaccaaatggcccagatcgaagaggtgtttaaggtggtgtaccctgtggatgatcatcactttaaggtgatcctgccctatggcacactggtaatcgacggggttacgccgaacatgctgaactatttcggacggccgtatgaaggcatcgccgtgttcgacggcaaaaagatcactgtaacagggaccctgtggaacggcaacaaaattatcgacgagcgcctgatcacccccgacggctccatgctgttccgagtaaccatcaacagtgggagttccggtggtggcgggagcggaggtggaggcatgggagatgaagattgggaagcagaaatcaaccctcatatgtcttcctatgttcccatatttgagaaggataggtattctggagaaaatggagacaattttaacaggactccagcttcatcatcagaaatggatgatggaccttctcgaagagatcatttcatgaaaagtggatttgcctctgggcggaattttggaaacagagatgctggtgagtgtaataagcgagataatacatccacaatgggtggttttggagttggaaagagttttggaaacagaggtttttcaaacagcaggtttgaagatggtgatagctctggtttctggagagagtctagtaatgactgcgaagataatccaacacggaacagagggttttccaagagaggcggctatcgagatggaaataattcagaagcttcagggccatacagaagaggtggaagaggtagtttccgaggttgccgtggaggatttggtctaggaagtccaaataatgacttagacccagacgaatgtatgcagcgcactggtggcctttttggttctagaagaccagtattaagtggcacaggtaatggtgatacttctcaaagcagaagtggcagtggaagtgaacgaggtggttacaaaggtttaaatgaagaagtaataacaggctctggaaagaattcttggaagtcagaagcagaaggaggagaaagtagtgatactcaaggaccaaaagtgacctacataccccctcctccacctgaggatgaggactccatctttgcacattatcagacaggcataaacttcgacaaatacgacactattcttgtggaagtgtctggacatgatgcaccaccagcaattctgacttttgaagaagctaatctctgtcagacactgaataacaacattgctaaagctggttatactaagcttactcctgtgcaaaaatacagtattcctatcatacttgcaggacgagatttgatggcttgcgctcaaacagggtctgggaagactgcggcttttctcctaccaattttggctcatatgatgcatgatggaataactgccagtcgttttaaagagttgcaggaaccagagtgtattattgtagcaccaactcgagaattggtcaaccagatttatttggaagccagaaaattttcttttgggacttgtgtaagagctgttgttatatatgggggaacccagctgggacattcaattcgacaaatagtacaaggctgtaatatattatgtgctactcctggaagactgatggatatcataggcaaagaaaagattggtctcaaacagatcaaatacttagttttggatgaagctgatcgcatgttggatatgggttttggtccagaaatgaagaagttaatttcttgcccaggaatgccatcaaaggaacagcgccaaacccttatgttcagtgcaacttttccagaggaaattcaaaggttggctgcagagtttttaaagtcaaattatctgtttgttgctgttggacaagtgggtggagcatgtagagatgttcagcagaccgttctccaagttggccagttctcaaaaagagaaaagctcgttgaaattctgcgaaacataggggatgaaagaactatggtctttgttgaaactaagaaaaaagcagattttattgcaacttttctttgtcaagaaaaaatatcaactacaagtattcatggtgatcgggaacagagagagcgggagcaagctcttggagattttcgctttggaaagtgcccagttcttgttgctacttcagtagctgccagagggctggatattgaaaatgtgcaacatgttatcaattttgatcttccttctaccattgatgaatatgttcatcgaattgggcgtactggtcgttgtgggaatactggcagagcaatttccttttttgatcttgaatcggataaccatttagcacagcctctagtaaaagtattgacagatgctcaacaggatgttcctgcatggttggaagaaattgcctttagtacatacattcctggcttcagtggtagtacaagaggaaacgtgtttgcatcagttgataccagaaagggcaagagcactttgaacacagctgggttttcttcttcacaagctcccaatccagtagatgatgagtcatgggattaa

SEQ ID NO: 62 - DNA, 3172 bp, synthetic construct
  source 1..3172: mol_type = other DNA
ggcctaactggccggtacctgagtctaaatgagtcttcggacctcgcgggggccgcttaagcggtggttagggtttgtctgacgcggggggagggggaaggaacgaaacactctcattcggaggcggctcggggtttggtcttggtggccacgggcacgcagaagagcgccgcgatcctcttaagcacccccccgccctccgtggaggcgggggtttggtcggcgggtggtaactggcgggccgctgactcgggcgggtcgcgcgccccagagtgtgaccttttcggtctgctcgcagacccccgggcggcgccgccgcggcggcgacgggctcgctgggtcctaggctccatggggaccgtatacgtggacaggctctggagcatccgcacgactgcggtgatattaccggagaccttctgcgggacgagccgggtcacgcggctgacgcggagcgtccgttgggcgacaaacaccaggacggggcacaggtacactatcttgtcacccggaggcgcgagggactgcaggagcttcagggagtggcgcagctgcttcatccccgtggcccgttgctcgcgtttgctggcggtgtccccggaagaaatatatttgcatgtctttagttctatgatgacacaaaccccgcccagcgtcttgtcattggcgaagtcgaacacgcagatgcagtcggggcggcgcggtcccaggtccacttcgcatattaaggtgacgcgtgtggcctcgaacaccgagcgaccctgcagcgacccgcttaaaagcttggcaatccggtactgttggtaaagccaccatggtcttcacactcgaagatttcgttggggactgggaacagacagccgcctacaacctggaccaagtccttgaacagggaggtgtgtccagtttgctgcagaatctcgccgtgtccgtaactccgatccaaaggattgtccggagcggtgaaaatgccctgaagatcgacatccatgtcatcatcccgtatgaaggtctgagcgccgaccaaatggcccagatcgaagaggtgtttaaggtggtgtaccctgtggatgatcatcactttaaggtgatcctgccctatggcacactggtaatcgacggggttacgccgaacatgctgaactatttcggacggccgtatgaaggcatcgccgtgttcgacggcaaaaagatcactgtaacagggaccctgtggaacggcaacaaaattatcgacgagcgcctgatcacccccgacggctccatgctgttccgagtaaccatcaacagtgggagttccggtggtggcgggagcggaggtggaggcatgtcgggttattcgagtgaccgagaccgcggccgggaccgagggtttggtgcacctcgatttggaggaagtagggcagggcccttatctggaaagaagtttggaaaccctggggagaaattagttaaaaagaagtggaatcttgatgagctgcctaaatttgagaagaatttttatcaagagcaccctgatttggctaggcgcacagcacaagaggtggaaacatacagaagaagcaaggaaattacagttagaggtcacaactgcccgaagccagttctaaatttttatgaagccaatttccctgcaaatgtcatggatgttattgcaagacagaatttcactgaacccactgctattcaagctcagggatggccagttgctctaagtggattggatatggttggagtggcacagactggatctgggaaaacattgtcttatttgcttcctgccattgtccacatcaatcatcagccattcctagagagaggcgatgggcctatttgtttggtgctggcaccaactcgggaactggcccaacaggtgcagcaagtagctgctgaatattgtagagcatgtcgcttgaagtctacttgtatctacggtggtgctcctaagggaccacaaatacgtgatttggagagaggtgtggaaatctgtattgcaacacctggaagactgattgactttttagagtgtggaaaaaccaatctgagaagaacaacctaccttgtccttgatgaagcagatagaatgcttgatatgggctttgaaccccaaataaggaagattgtggatcaaataagacctgataggcaaactctaatgtggagtgcgacttggccaaaagaagtaagacagcttgctgaagatttcctgaaagactatattcatataaacattggtgcacttgaactgagtgcaaaccacaacattcttcagattgtggatgtgtgtcatgacgtagaaaaggatgaaaaacttattcgtctaatggaagagatcatgagtgagaaggagaataaaaccattgtttttgtggaaaccaaaagaagatgtgatgagcttaccagaaaaatgaggagagatgggtggcctgccatgggtatccatggtgacaagagtcaacaagagcgtgactgggttctaaatgaattcaaacatggaaaagctcctattctgattgctacagatgtggcctccagagggctagatgtggaagatgtgaaatttgtcatcaattatgactaccctaactcctcagaggattatattcatcgaattggaagaactgctcgcagtaccaaaacaggcacagcatacactttctttacacctaataacataaagcaagtgagcgaccttatctctgtgcttcgtgaagctaatcaagcaattaatcccaagttgcttcagttggtcgaagacagaggttcaggtcgttccaggggtagaggaggcatgaaggatgaccgtcgggacagatactctgcgggcaaaaggggtggatttaatacctttagagacagggaaaattatgacagaggttactctagcctgcttaaaagagattttggggcaaaaactcagaatggtgtttacagtgctgcaaattacaccaatgggagctttggaagtaattttgtgtctgctggtatacagaccagttttaggactggtaatccaacagggacttaccagaatggttatgatagcactcagcaatacggaagtaatgttccaaatatgcacaatggtatgaaccaacaggcatatgcatatcctgctactgcagctgcacctatgattggttatccaatgccaacaggatattcccaataa

SEQ ID NO: 63 - DNA, 2779 bp, synthetic construct
  source 1..2779: mol_type = other DNA
ggcctaactggccggtacctgagtctaaatgagtcttcggacctcgcgggggccgcttaagcggtggttagggtttgtctgacgcggggggagggggaaggaacgaaacactctcattcggaggcggctcggggtttggtcttggtggccacgggcacgcagaagagcgccgcgatcctcttaagcacccccccgccctccgtggaggcgggggtttggtcggcgggtggtaactggcgggccgctgactcgggcgggtcgcgcgccccagagtgtgaccttttcggtctgctcgcagacccccgggcggcgccgccgcggcggcgacgggctcgctgggtcctaggctccatggggaccgtatacgtggacaggctctggagcatccgcacgactgcggtgatattaccggagaccttctgcgggacgagccgggtcacgcggctgacgcggagcgtccgttgggcgacaaacaccaggacggggcacaggtacactatcttgtcacccggaggcgcgagggactgcaggagcttcagggagtggcgcagctgcttcatccccgtggcccgttgctcgcgtttgctggcggtgtccccggaagaaatatatttgcatgtctttagttctatgatgacacaaaccccgcccagcgtcttgtcattggcgaagtcgaacacgcagatgcagtcggggcggcgcggtcccaggtccacttcgcatattaaggtgacgcgtgtggcctcgaacaccgagcgaccctgcagcgacccgcttaaaagcttggcaatccggtactgttggtaaagccaccatggtcttcacactcgaagatttcgttggggactgggaacagacagccgcctacaacctggaccaagtccttgaacagggaggtgtgtccagtttgctgcagaatctcgccgtgtccgtaactccgatccaaaggattgtccggagcggtgaaaatgccctgaagatcgacatccatgtcatcatcccgtatgaaggtctgagcgccgaccaaatggcccagatcgaagaggtgtttaaggtggtgtaccctgtggatgatcatcactttaaggtgatcctgccctatggcacactggtaatcgacggggttacgccgaacatgctgaactatttcggacggccgtatgaaggcatcgccgtgttcgacggcaaaaagatcactgtaacagggaccctgtggaacggcaacaaaattatcgacgagcgcctgatcacccccgacggctccatgctgttccgagtaaccatcaacagtgggagttccggtggtggcgggagcggaggtggaggcatgagcacggccagaacagagaaccctgttataatgggtctgtccagtcaaaatggtcagctgagaggccctgtgaaacccactggtggccctggaggagggggcacacagacacagcaacagatgaaccagctgaaaaacaccaacacaatcaataatggcactcagcagcaagcacagagtatgaccaccactattaaacctggtgatgactggaaaaagactttaaaactccctccaaaggatctaagaatcaaaacttcggatgtgacctccacaaaaggaaatgagtttgaagattactgtttgaaacgggagttactgatgggaatttttgaaatgggctgggaaaagccatctcctattcaggaggagagcattcccattgctttatctggtagggatatcttagctagagcaaaaaatggaacaggcaagagcggtgcctacctcattcccttacttgaacggctagacctgaagaaggacaatatacaagcaatggtgattgttcccactagagaacttgctctacaggtcagtcaaatttgcatccaggtcagcaaacacatgggaggggccaaagtgatggcaaccacaggaggaaccaatttacgagatgacataatgaggcttgatgatacagtgcacgtggtgattgctacccctgggagaatcctggatcttattaagaaaggagtagcaaaggttgatcatgtccagatgatagtattggatgaggcagataagttgctgtcacaggattttgtgcagataatggaggatattattctcacgctacctaaaaacaggcagattttactatattccgctactttccctcttagtgtacagaagttcatgaattcccatttgcagaaaccctatgagattaacctgatggaggaactaactctgaagggagtaacccagtactacgcatatgtaactgagcgccaaaaagtacactgcctcaacacacttttctccaggcttcagataaaccagtcgatcattttctgtaactcctctcagcgagttgaattgctagccaagaagatttctcaactgggttattcttgcttctatattcatgctaaaatgaggcaggaacatcgaaatcgtgtatttcatgatttccgaaatggcttatgccgcaatcttgtttgcactgatctgtttacccgaggtattgatatacaagctgtgaatgtggtaataaactttgatttcccaaagctggcagagacctatctccatcgtattggaagatcaggtcgctttggtcatcttggcttagccatcaacttgatcacatatgatgatcgcttcaacctgaaaagtattgaggagcagctgggaacagaaattaaacctattccgagcaacattgataagagcctgtatgtggcagaataccacagcgagcctgtagaagatgagaaaccttaa

SEQ ID NO: 64 - DNA, 3955 bp, synthetic construct
  source 1..3955: mol_type = other DNA
ggcctaactggccggtacctgagtctaaatgagtcttcggacctcgcgggggccgcttaagcggtggttagggtttgtctgacgcggggggagggggaaggaacgaaacactctcattcggaggcggctcggggtttggtcttggtggccacgggcacgcagaagagcgccgcgatcctcttaagcacccccccgccctccgtggaggcgggggtttggtcggcgggtggtaactggcgggccgctgactcgggcgggtcgcgcgccccagagtgtgaccttttcggtctgctcgcagacccccgggcggcgccgccgcggcggcgacgggctcgctgggtcctaggctccatggggaccgtatacgtggacaggctctggagcatccgcacgactgcggtgatattaccggagaccttctgcgggacgagccgggtcacgcggctgacgcggagcgtccgttgggcgacaaacaccaggacggggcacaggtacactatcttgtcacccggaggcgcgagggactgcaggagcttcagggagtggcgcagctgcttcatccccgtggcccgttgctcgcgtttgctggcggtgtccccggaagaaatatatttgcatgtctttagttctatgatgacacaaaccccgcccagcgtcttgtcattggcgaagtcgaacacgcagatgcagtcggggcggcgcggtcccaggtccacttcgcatattaaggtgacgcgtgtggcctcgaacaccgagcgaccctgcagcgacccgcttaaaagcttggcaatccggtactgttggtaaagccaccatggtcttcacactcgaagatttcgttggggactgggaacagacagccgcctacaacctggaccaagtccttgaacagggaggtgtgtccagtttgctgcagaatctcgccgtgtccgtaactccgatccaaaggattgtccggagcggtgaaaatgccctgaagatcgacatccatgtcatcatcccgtatgaaggtctgagcgccgaccaaatggcccagatcgaagaggtgtttaaggtggtgtaccctgtggatgatcatcactttaaggtgatcctgccctatggcacactggtaatcgacggggttacgccgaacatgctgaactatttcggacggccgtatgaaggcatcgccgtgttcgacggcaaaaagatcactgtaacagggaccctgtggaacggcaacaaaattatcgacgagcgcctgatcacccccgacggctccatgctgttccgagtaaccatcaacagtgggagttccggtggtggcgggagcggaggtggaggcatgggcaaaacggccaactctccgggttcgggagcccgacccgacccggtgcggagcttcaatcgctggaagaaaaaacacagccataggcagaacaaaaagaagcagttgaggaagcaactgaagaaacccgaatggcaggtcgagcgcgagagtatcagccgcctcatgcagaactatgaaaagataaatgtaaatgaaatcacaagattttcagattttcccttgtccaaaaaaacattgaaaggtttgcaagaagctcagtaccgtttggtgactgagatacagaagcagaccattggattggctttgcaaggtaaagatgtacttggagcggccaaaactggatctggcaagactctggcttttcttgttccagtgctggaagccttatatcgtctgcaatggacttcaacagatgggctgggggttctcataatatcacctacgagagaactggcctatcagacctttgaggttctccgaaaagtaggaaagaatcatgacttctcagctggtctcatcattggtggaaaggatctaaaacacgaagctgagaggatcaacaacataaatatactcgtgtgcacaccaggtcggcttcttcaacacatggatgaaacagtatcttttcatgctaccgacctccaaatgttagttcttgatgaagcagatagaatcttggatatgggctttgctgataccatgaatgctgttattgaaaatctccccaagaaacgtcagactttacttttctcagcaacacaaactaaatctgtaaaggaccttgcacgcttgagtttgaaaaaccctgagtatgtctgggttcatgaaaaagcaaaatatagcacccctgccactttggaacagaactacatagtctgtgagctgcagcaaaaaataagtgtgctgtattcctttttgagaagccatctgaagaagaagagcattgtatttttttccagttgcaaagaggtccagtatctgtaccgagtgttttgccggctacgtcctggtgtttctatccttgcactccatggtcgacagcagcaaatgagaagaatggaagtctataatgagtttgtccgtaagagagctgcagtactctttgctactgatattgcagccaggggtctggatttcccggccgtgaattgggttcttcagtttgattgtcctgaggatgccaacacatatattcacagagcaggtagaactgccaggtacaaagaggatggtgaagctttgctaattttgctaccctcagaaaaagctatggtgcagcagcttcttcagaagaaagtacctgtgaaggaaatcaaaatcaatccagaaaaacttatagatgtccagaaaaaattggaatctattttagctcaagatcaagatttaaaagaaagagctcaaaggtgtttcgtctcctatgtacgatctgtatatctgatgaaggataaagaagtatttgatgtgagcaagttacctatacctgaatatgccctgtctcttggtcttgctgtggcaccacgcgtaagatttcttcagaaaatgcagaaacaacccaccaaagaattggtaaggagccaagccgataaagtaattgagccaagggctccctccctcaccaatgacgaagtggaagaatttagagcctacttcaatgagaaaatgtccatccttcaaaaaggtggaaaaagactcgaagggacagagcacagacaggataatgatactggtaatgaagaacaggaagaagaagaagacgatgaagaagaaatggaagagaaactggcaaaagcaaaaggatctcaagccccatctcttcctaacaccagtgaggcacagaagatcaaggaagttcctacacagttcttggacagagatgaggaggaagaagatgctgatttcttgaaggtgaagcggcataatgtgtttggattggaccttaaagacgagaaaacattacagaagaaagaaccttctaaatccagcatcaagaaaaaaatgaccaaagttgcagaagcaaaaaaagtaatgaagagaaattttaaagtgaataagaagataacatttactgatgaaggggagttggttcagcagtggccacaaatgcagaaatctgccatcaaggatgctgaggaagatgatgacacaggtggtatcaacttacataaagcaaaggaaagacttcaggaagaggacaaatttgacaaagaagaatataggaaaaaaattaaggcaaagcatcgggagaaaagactgaaagaaagggaagccagaagagaagccaacaagagacaagcaaaggccaaagatgaagaggaagcctttctggattggagtgatgatgatgatgatgatgatgatggatttgatccaagcacactcccagatccagataaatacagaagctctgaagattcagatagtgaagatatggaaaataaaataagtgataccaagaagaagcaggggatgaagaagaggagcaacagtgaagtggaagacgtgggaccaacaagtcataacagaaagaaggccaggtgggacactttagagcctttggataccggcctgtctttagcagaggatgaagagctggtgttacatctgctaagaagtcaaagctaa

SEQ ID NO: 65 - DNA, 4040 bp, synthetic construct
  source 1..4040: mol_type = other DNA
ggcctaactggccggtacctgagtctaaatgagtcttcggacctcgcgggggccgcttaagcggtggttagggtttgtctgacgcggggggagggggaaggaacgaaacactctcattcggaggcggctcggggtttggtcttggtggccacgggcacgcagaagagcgccgcgatcctcttaagcacccccccgccctccgtggaggcgggggtttggtcggcgggtggtaactggcgggccgctgactcgggcgggtcgcgcgccccagagtgtgaccttttcggtctgctcgcagacccccgggcggcgccgccgcggcggcgacgggctcgctgggtcctaggctccatggggaccgtatacgtggacaggctctggagcatccgcacgactgcggtgatattaccggagaccttctgcgggacgagccgggtcacgcggctgacgcggagcgtccgttgggcgacaaacaccaggacggggcacaggtacactatcttgtcacccggaggcgcgagggactgcaggagcttcagggagtggcgcagctgcttcatccccgtggcccgttgctcgcgtttgctggcggtgtccccggaagaaatatatttgcatgtctttagttctatgatgacacaaaccccgcccagcgtcttgtcattggcgaagtcgaacacgcagatgcagtcggggcggcgcggtcccaggtccacttcgcatattaaggtgacgcgtgtggcctcgaacaccgagcgaccctgcagcgacccgcttaaaagcttggcaatccggtactgttggtaaagccaccatggtcttcacactcgaagatttcgttggggactgggaacagacagccgcctacaacctggaccaagtccttgaacagggaggtgtgtccagtttgctgcagaatctcgccgtgtccgtaactccgatccaaaggattgtccggagcggtgaaaatgccctgaagatcgacatccatgtcatcatcccgtatgaaggtctgagcgccgaccaaatggcccagatcgaagaggtgtttaaggtggtgtaccctgtggatgatcatcactttaaggtgatcctgccctatggcacactggtaatcgacggggttacgccgaacatgctgaactatttcggacggccgtatgaaggcatcgccgtgttcgacggcaaaaagatcactgtaacagggaccctgtggaacggcaacaaaattatcgacgagcgcctgatcacccccgacggctccatgctgttccgagtaaccatcaacagtgggagttccggtggtggcgggagcggaggtggaggcatggctaatgaaacacagaaggttggtgccatccattttccttttcccttcacaccctattccatccaggaagacttcatggcagagctgtaccgggttttggaggctggcaagattgggatatttgagagtccaactggcactgggaagtccttaagtcttatttgtggggccctctcttggctccgtgactttgaacagaagaagcgtgaagaagaggcacgactccttgaaactggaactggccccttacatgatgagaaagatgaatccctgtgtctgtcttcttcctgcgaaggggctgcaggcaccccgaggcctgctggagaaccggcctgggttactcagtttgtgcagaagaaagaagagagggacctggtggaccgactaaaggcggagcaggccaggaggaagcagcgagaagaacgcctgcagcagctgcagcacagggtgcagctcaagtatgcagccaagcgcctgaggcaggaagaagaagaaagagagaatctcctccgcctcagcagggagatgctagagacaggcccggaggctgagcggctggagcagctggagtctggggaggaggagctggtcctcgccgaatacgagagtgatgaggagaaaaaggtggcgagcagagtggatgaggatgaggatgacctggaggaagaacacataactaagatttattactgtagtcggacacactcccagctggcccagtttgtgcatgaggtgaagaagagcccctttggcaaggatgttcggctggtctcccttggctcccggcagaacctttgtgtaaatgaagacgtgaaaagcctaggttctgtgcagcttatcaacgaccgctgtgtggacatgcagagaagcaggcacgagaagaagaaaggagctgaggaggagaagccaaagaggaggaggcaggagaagcaggcagcctgccccttctacaaccacgagcagatgggccttctccgggatgaggccctggcagaggtgaaggacatggagcagctgctggcccttgggaaggaggcccgggcctgtccctattacgggagccgccttgccatccctgcagcccagctggtggtgctgccctatcagatgctgctgcatgcggccactcggcaggccgcgggcatccggctgcaggaccaggtggtgatcatcgacgaggcgcacaacctgatcgacaccatcacgggcatgcacagcgtggaggtcagcggctcccagctctgccaggcccattcccagctgctgcagtacgtggagcgatacgggaagcgtttgaaggccaagaacctgatgtacctgaagcagatcctgtatttgctggagaaattcgtggctgtgctaggggggaacattaagcaaaatcccaatacacagagtctgtcacagacagggacggagctgaagaccatcaacgactttctcttccagagccagatcgacaacatcaacctgttcaaggtgcagcgatactgtgagaagagcatgatcagcagaaagctctttggattcactgaacggtacggagcagtgttctcatcccgggagcagcccaaactggctgggtttcagcaattcctgcagagcctgcagcccaggacgactgaagctcttgcagcccctgcagacgagagtcaggccagcaccctgcgaccagcttctccactgatgcacatccaaggcttcctggcagctctcactacggccaaccaggacggcagggtcatcctgagccgccaaggcagcctcagtcagagcaccctgaagtttttgctcctgaatccagctgtgcactttgcccaagtggtgaaggaatgccgggcagtggtcattgcggggggtaccatgcagccggtgtctgacttccggcagcagctgctggcctgtgccggggtggaagctgagcgcgtggtggagttttcctgtggtcacgtgatccctccagacaacatcctgcccctcgtcatctgcagcgggatctccaaccagccgctggaattcacgttccagaaaagagagctgcctcagatgatggacgaggtgggtcgcattctctgtaacctgtgcggtgtggttcctggaggggtggtctgtttcttcccctcctacgagtacctgcgccaggtccatgcccactgggagaagggtggcctgctgggccgtctggctgccaggaagaagatattccaggaacctaagagcgcacaccaggtggagcaggtgctgctggcatattccaggtgcatccaggcctgtggccaggagagaggccaggtgacaggggccctgctcctctctgtggttggaggaaagatgagtgaagggatcaacttctctgacaacctaggccggtgtgtggtgatggtgggcatgcccttccccaacatcaggtctgcagagctgcaggagaagatggcctacttggatcaaaccctcagcccccggccaggcacccccagggaaggctctggtggagaacctgtgcatgaaggccgtcaaccagtccataggcagggccatcaggcaccagaaggattttgccagcgtagtgctcctggaccagcgatatgcccggccccctgtcctggccaagctgccggcctggatccgagcccgtgtggaggtcaaagctacctttggccccgccattgctgctgtgcagaagtttcaccgggagaagtcggcctcttcc

SEQ ID NO: 66 - DNA, 3517 bp, synthetic construct
  source 1..3517: mol_type = other DNA
ggcctaactggccggtacctgagtctaaatgagtcttcggacctcgcgggggccgcttaagcggtggttagggtttgtctgacgcggggggagggggaaggaacgaaacactctcattcggaggcggctcggggtttggtcttggtggccacgggcacgcagaagagcgccgcgatcctcttaagcacccccccgccctccgtggaggcgggggtttggtcggcgggtggtaactggcgggccgctgactcgggcgggtcgcgcgccccagagtgtgaccttttcggtctgctcgcagacccccgggcggcgccgccgcggcggcgacgggctcgctgggtcctaggctccatggggaccgtatacgtggacaggctctggagcatccgcacgactgcggtgatattaccggagaccttctgcgggacgagccgggtcacgcggctgacgcggagcgtccgttgggcgacaaacaccaggacggggcacaggtacactatcttgtcacccggaggcgcgagggactgcaggagcttcagggagtggcgcagctgcttcatccccgtggcccgttgctcgcgtttgctggcggtgtccccggaagaaatatatttgcatgtctttagttctatgatgacacaaaccccgcccagcgtcttgtcattggcgaagtcgaacacgcagatgcagtcggggcggcgcggtcccaggtccacttcgcatattaaggtgacgcgtgtggcctcgaacaccgagcgaccctgcagcgacccgcttaaaagcttggcaatccggtactgttggtaaagccaccatggtcttcacactcgaagatttcgttggggactgggaacagacagccgcctacaacctggaccaagtccttgaacagggaggtgtgtccagtttgctgcagaatctcgccgtgtccgtaactccgatccaaaggattgtccggagcggtgaaaatgccctgaagatcgacatccatgtcatcatcccgtatgaaggtctgagcgccgaccaaatggcccagatcgaagaggtgtttaaggtggtgtaccctgtggatgatcatcactttaaggtgatcctgccctatggcacactggtaatcgacggggttacgccgaacatgctgaactatttcggacggccgtatgaaggcatcgccgtgttcgacggcaaaaagatcactgtaacagggaccctgtggaacggcaacaaaattatcgacgagcgcctgatcacccccgacggctccatgctgttccgagtaaccatcaacagtgggagttccggtggtggcgggagcggaggtggaggcatgcccaccggctttgtagccccgattctctgtgttttgctcccgtctccgacgagagaggcggcgacggtggcgtctgcgacgggagacagcgcgtcggagcgagagagcgctgcgcctgccgccgccccaacagcggaggcgccgccgccatcggtcgtcaccagaccggagccgcaggccctcccgagcccggccatccgtgccccgctcccagatctctatccttttgggaccatgcgcggaggaggctttggggaccgggaccgggatcgtgaccgtggaggatttggagcaagaggtggtggtggccttcccccgaagaaatttggtaatcctggggagcgtttgcgtaaaaaaaagtgggatttgagtgagctccccaagtttgagaaaaatttttatgtggaacatccggaagtagcaaggctgacaccatatgaggttgatgagctacgccgaaagaaggagattacagtgagggggggagatgtttgtcctaaacccgtgtttgccttccatcatgctaacttcccacaatatgtaatggatgtgttgatggatcagcactttacagaaccaactccaattcagtgccagggatttccgttggctcttagtggccgggatatggtgggcattgctcagactggctctgggaagacgttggcgtatctcctgcctgcaattgttcatattaaccaccagccatacttggaaaggggagatggcccaatctgtctagttctggctcctaccagagagcttgcccagcaagtacagcaggtggccgatgactatggcaaatgttctagattgaagagtacttgtatttatggaggtgctcctaaaggtccccagattcgagacttggaaagaggtgttgagatctgcatagccactcctggacgtctgatagatttcctggagtcaggaaagacaaatcttcgccgatgtacttaccttgtattggacgaagctgacagaatgcttgatatggggtttgaaccccagatccgtaaaattgttgaccaaatcaggcctgataggcagacactgatgtggagtgcaacctggccaaaagaagtaagacagcttgcagaggatttccttcgtgattacacccagatcaacgtaggcaatctggagttgagtgccaaccacaacatcctccagatagtggatgtctgcatggaaagtgaaaaagaccacaagttgatccaactaatggaagaaataatggctgaaaaggaaaacaaaacaataatatttgtggagacaaagagacgctgtgatgatctgactcgaaggatgcgcagagatggttggccagctatgtgtatccatggagacaagagtcaaccagaaagagattgggtacttaatgagttccgttctggaaaggcacccatccttattgctacagatgtagcctcccgtgggctagatgtggaagatgtcaagtttgtgatcaactatgactatccaaacagctcagaggattatgtgcaccgtattggccgaacagcccgtagcaccaacaagggtaccgcctataccttcttcaccccagggaacctaaaacaggccagagagcttatcaaagtgctggaagaggccaatcaggctatcaatccaaaactgatgcagcttgtggaccacagaggaggcggcggaggcgggggtggtcgttctcgttaccggaccacttcttcagccaacaatcccaatctgatgtatcaggatgagtgtgaccgaaggcttcgaggagtcaaggatggtggccggagagactctgcaagctatcgggatcgtagtgaaaccgatagagctggttatgctaatggcagtggctatggaagtccaaattctgcctttggagcacaagcaggccaatacacctatggtcaaggcacctatggggcagctgcttatggcaccagtagctatacagctcaagaatatggtgctggcacttatggagctagtagcaccacctcaactgggagaagttcacagagctctagccagcagtttagtgggataggccggtctgggcagcagccacagccactgatgtcacaacagtttgcacagcctccgggagctaccaatatgataggttacatggggcagactgcctaccaataccctcctcctcctccccctcctcctccttcacgtaaatga

SEQ ID NO: 67 - DNA, 3340 bp, synthetic construct
  source 1..3340: mol_type = other DNA
ggcctaactggccggtacctgagtctaaatgagtcttcggacctcgcgggggccgcttaagcggtggttagggtttgtctgacgcggggggagggggaaggaacgaaacactctcattcggaggcggctcggggtttggtcttggtggccacgggcacgcagaagagcgccgcgatcctcttaagcacccccccgccctccgtggaggcgggggtttggtcggcgggtggtaactggcgggccgctgactcgggcgggtcgcgcgccccagagtgtgaccttttcggtctgctcgcagacccccgggcggcgccgccgcggcggcgacgggctcgctgggtcctaggctccatggggaccgtatacgtggacaggctctggagcatccgcacgactgcggtgatattaccggagaccttctgcgggacgagccgggtcacgcggctgacgcggagcgtccgttgggcgacaaacaccaggacggggcacaggtacactatcttgtcacccggaggcgcgagggactgcaggagcttcagggagtggcgcagctgcttcatccccgtggcccgttgctcgcgtttgctggcggtgtccccggaagaaatatatttgcatgtctttagttctatgatgacacaaaccccgcccagcgtcttgtcattggcgaagtcgaacacgcagatgcagtcggggcggcgcggtcccaggtccacttcgcatattaaggtgacgcgtgtggcctcgaacaccgagcgaccctgcagcgacccgcttaaaagcttggcaatccggtactgttggtaaagccaccatggtcttcacactcgaagatttcgttggggactgggaacagacagccgcctacaacctggaccaagtccttgaacagggaggtgtgtccagtttgctgcagaatctcgccgtgtccgtaactccgatccaaaggattgtccggagcggtgaaaatgccctgaagatcgacatccatgtcatcatcccgtatgaaggtctgagcgccgaccaaatggcccagatcgaagaggtgtttaaggtggtgtaccctgtggatgatcatcactttaaggtgatcctgccctatggcacactggtaatcgacggggttacgccgaacatgctgaactatttcggacggccgtatgaaggcatcgccgtgttcgacggcaaaaagatcactgtaacagggaccctgtggaacggcaacaaaattatcgacgagcgcctgatcacccccgacggctccatgctgttccgagtaaccatcaacagtgggagttccggtggtggcgggagcggaggtggaggcatgtcacacctgccgatgaaactcctgcgtaagaagatcgagaagcggaacctcaaattgcggcagcggaacctaaagtttcagggggcctcaaatctgaccctatcggaaactcaaaatggagatgtatctgaagaaacaatgggaagtagaaaggttaaaaaatcaaaacaaaagcccatgaatgtgggcttatcagaaactcaaaatggaggcatgtctcaagaagcagtgggaaatataaaagttacaaagtctccccagaaatccactgtattaaccaatggagaagcagcaatgcagtcttccaattcagaatcaaaaaagaaaaagaagaaaaagagaaaaatggtgaatgatgctgagcctgatacgaaaaaagcaaaaactgaaaacaaagggaaatctgaagaagaaagtgccgagactactaaagaaacagaaaataatgtggagaagccagataatgatgaagatgagagtgaggtgcccagtctgcccctgggactgacaggagcttttgaggatacttcgtttgcttctctatgtaatcttgtcaatgaaaacactctgaaggcaataaaagaaatgggttttacaaacatgactgaaattcagcataaaagtatcagaccacttctggaaggcagggatcttctagcagctgcaaaaacaggcagtggtaaaaccctggcttttctcatccctgcagttgaactcattgttaagttaaggttcatgcccaggaatggaacaggagtccttattctctcacctactagagaactagccatgcaaacctttggtgttcttaaggagctgatgactcaccacgtgcatacctatggcttgataatgggtggcagtaacagatctgctgaagcacagaaacttggtaatgggatcaacatcattgtggccacaccaggccgtctgctggaccatatgcagaataccccaggatttatgtataaaaacctgcagtgtctggttattgatgaagctgatcgtatcttggatgtggggtttgaagaggaattaaagcaaattattaaacttttgccaacacgtagacagactatgctcttttctgccacccaaactcgaaaagttgaagacctggcaaggatttctctgaaaaaggagccattgtatgttggcgttgatgatgataaagcgaatgcaacagtggatggtcttgaacagggatatgttgtttgtccttctgaaaagagattccttctgctctttacattccttaagaagaaccgaaagaagaagcttatggtcttcttttcatcttgtatgtctgtgaaataccactatgagttgctgaactacattgatttgcccgtcttggccattcatggaaagcaaaagcaaaataagcgtacaaccacattcttccagttctgcaatgcagattcgggaacactattgtgtacggatgtggcagcgagaggactagacattcctgaagtcgactggattgttcagtatgaccctccggatgaccctaaggaatatattcatcgtgtgggtagaacagccagaggcctaaatgggagagggcatgccttgctcattttgcgcccagaagaattgggttttcttcgctacttgaaacaatccaaggttccattaagtgaatttgacttttcctggtctaaaatttctgacattcagtctcagcttgagaaattgattgaaaagaattactttcttcataagtcagcccaggaagcatataagtcatacatacgagcctatgattcccattctctgaaacagatctttaatgttaataacctaaatttgcctcaggttgctctgtcatttggtttcaaggtgcctcccttcgttgatctgaacgtcaacagtaatgaaggcaagcagaaaaagcgaggaggtggtggtggatttggctaccagaaaaccaagaaagttgagaaatccaaaatctttaaacacattagcaagaaatcatctgacagcaggcagttctctcactga

SEQ ID NO: 68 - DNA, 2767 bp, Homo sapiens
  source 1..2767: mol_type = genomic DNA
ggcctaactggccggtacctgagtctaaatgagtcttcggacctcgcgggggccgcttaagcggtggttagggtttgtctgacgcggggggagggggaaggaacgaaacactctcattcggaggcggctcggggtttggtcttggtggccacgggcacgcagaagagcgccgcgatcctcttaagcacccccccgccctccgtggaggcgggggtttggtcggcgggtggtaactggcgggccgctgactcgggcgggtcgcgcgccccagagtgtgaccttttcggtctgctcgcagacccccgggcggcgccgccgcggcggcgacgggctcgctgggtcctaggctccatggggaccgtatacgtggacaggctctggagcatccgcacgactgcggtgatattaccggagaccttctgcgggacgagccgggtcacgcggctgacgcggagcgtccgttgggcgacaaacaccaggacggggcacaggtacactatcttgtcacccggaggcgcgagggactgcaggagcttcagggagtggcgcagctgcttcatccccgtggcccgttgctcgcgtttgctggcggtgtccccggaagaaatatatttgcatgtctttagttctatgatgacacaaaccccgcccagcgtcttgtcattggcgaagtcgaacacgcagatgcagtcggggcggcgcggtcccaggtccacttcgcatattaaggtgacgcgtgtggcctcgaacaccgagcgaccctgcagcgacccgcttaaaagcttggcaatccggtactgttggtaaagccaccatggtcttcacactcgaagatttcgttggggactgggaacagacagccgcctacaacctggaccaagtccttgaacagggaggtgtgtccagtttgctgcagaatctcgccgtgtccgtaactccgatccaaaggattgtccggagcggtgaaaatgccctgaagatcgacatccatgtcatcatcccgtatgaaggtctgagcgccgaccaaatggcccagatcgaagaggtgtttaaggtggtgtaccctgtggatgatcatcactttaaggtgatcctgccctatggcacactggtaatcgacggggttacgccgaacatgctgaactatttcggacggccgtatgaaggcatcgccgtgttcgacggcaaaaagatcactgtaacagggaccctgtggaacggcaacaaaattatcgacgagcgcctgatcacccccgacggctccatgctgttccgagtaaccatcaacagtgggagttccggtggtggcgggagcggaggtggaggcatggccactgactcatgggccctggcggtggacgagcaggaagctgcggctgagtcgttgagcaacttgcatcttaaggaagagaaaatcaaaccagataccaatggtgctgttgtcaagaccaatgccaatgcagagaagacagatgaagaagagaaagaggacagagctgcccagtccttactcaacaagctgatcagaagcaaccttgttgataacacaaaccaagtggaagtcctgcaacgggatccaaactcccctctgtactcggtgaagtcgtttgaagagcttcggctgaaaccacagcttctccagggagtctatgccatgggcttcaatcgaccctccaagatacaagagaacgcattacccatgatgcttgctgaacccccacagaatctgattgcccagtctcagtctggcactggtaaaacagctgcctttgtcttagccatgctcagccgagtggagccatcagacagatacccccagtgtctgtgcctctccccaacatatgagctggcgcttcaaacaggaaaagtgattgagcagatgggcaaattttacccagaactgaagcttgcctatgccgttcgaggcaataaattggaaagaggccagaagatcagtgagcagattgtcattggcacccctgggaccgtgctggactggtgctccaagctcaagttcattgatcccaagaaaatcaaggtgtttgttctggatgaggctgatgtcatgatagccactcagggccaccaagatcagagcatccgcatccagaggatgctgcccaggaactgccagatgctgcttttctccgccacctttgaagactctgtgtggaagtttgcccagaaagtggtcccagacccaaatgttatcaaactgaagcgtgaggaagagaccctggataccatcaagcagtactatgtcctgtgcagcagcagagacgagaagttccaggccttgtgtaacctctacggggccatcaccattgctcaagccatgatcttctgccatactcgcaaaacagctagttggctggcagcagagctctcaaaagaaggccaccaggtggctctgctgagtggggagatgatggtggagcagagggctgcggtgattgagcgcttccgagagggcaaagagaaggttttggtgaccaccaacgtgtgtgcccgcggcattgatgttgaacaagtgtctgtcgtcatcaactttgatcttcccgtggacaaggacgggaatcctgacaatgagacctacctgcaccggatcgggcgcacgggccgctttggcaagaggggcctggcagtgaacatggtggacagcaagcacagcatgaacatcctgaacagaatccaggagcattttaataagaagatagaaagattggacacagatgatttggacgagattgagaaaatagccaactga

SEQ ID NO: 69 - DNA, 3802 bp, synthetic construct
  source 1..3802: mol_type = other DNA
ggcctaactggccggtacctgagtctaaatgagtcttcggacctcgcgggggccgcttaagcggtggttagggtttgtctgacgcggggggagggggaaggaacgaaacactctcattcggaggcggctcggggtttggtcttggtggccacgggcacgcagaagagcgccgcgatcctcttaagcacccccccgccctccgtggaggcgggggtttggtcggcgggtggtaactggcgggccgctgactcgggcgggtcgcgcgccccagagtgtgaccttttcggtctgctcgcagacccccgggcggcgccgccgcggcggcgacgggctcgctgggtcctaggctccatggggaccgtatacgtggacaggctctggagcatccgcacgactgcggtgatattaccggagaccttctgcgggacgagccgggtcacgcggctgacgcggagcgtccgttgggcgacaaacaccaggacggggcacaggtacactatcttgtcacccggaggcgcgagggactgcaggagcttcagggagtggcgcagctgcttcatccccgtggcccgttgctcgcgtttgctggcggtgtccccggaagaaatatatttgcatgtctttagttctatgatgacacaaaccccgcccagcgtcttgtcattggcgaagtcgaacacgcagatgcagtcggggcggcgcggtcccaggtccacttcgcatattaaggtgacgcgtgtggcctcgaacaccgagcgaccctgcagcgacccgcttaaaagcttggcaatccggtactgttggtaaagccaccatggtcttcacactcgaagatttcgttggggactgggaacagacagccgcctacaacctggaccaagtccttgaacagggaggtgtgtccagtttgctgcagaatctcgccgtgtccgtaactccgatccaaaggattgtccggagcggtgaaaatgccctgaagatcgacatccatgtcatcatcccgtatgaaggtctgagcgccgaccaaatggcccagatcgaagaggtgtttaaggtggtgtaccctgtggatgatcatcactttaaggtgatcctgccctatggcacactggtaatcgacggggttacgccgaacatgctgaactatttcggacggccgtatgaaggcatcgccgtgttcgacggcaaaaagatcactgtaacagggaccctgtggaacggcaacaaaattatcgacgagcgcctgatcacccccgacggctccatgctgttccgagtaaccatcaacagtgggagttccggtggtggcgggagcggaggtggaggcatggcggcggcatttgaagcctcgggagccttagcagcagtggcgactgctatgccggctgagcatgtggccgtgcaggtcccggccccagagccaacacccgggcctgtgaggatcctgcggaccgctcaggatctcagcagcccgcggacccgcacgggggatgtgctgttggcggagccggccgacttcgagtcactgctgctttcgcggccggtgctggaggggctgcgggcggccggcttcgagaggccctcgccggtgcagctcaaggccatcccgttggggcgctgcgggctcgatttaattgttcaagctaaatctggcaccgggaaaacctgtgtgttctccaccatagctttggactctcttgttcttgaaaacttaagtacccagattttgatcttggctcctacaagagaaattgctgtacagatacattctgttattacagccattggaataaaaatggaaggcttagagtgtcatgtctttattggagggaccccattatcacaagacaaaaccagacttaaaaagtgtcatattgctgttggatctcctggcagaattaagcaactcatagaacttgactacttgaacccaggcagtatacgcctctttattcttgatgaagcagataagcttttagaagaaggcagcttccaggagcaaataaattggatttattcttccttgcctgccagtaaacagatgctggcagtatcagctacttatcccgaatttttggctaatgctttgacaaagtacatgagagatcccacttttgtaagactgaattccagtgatccaagtctcataggtttgaagcagtattacaaagttgtcaattcataccctttggcacataaggtttttgaggaaaagactcagcatttacaggaactgttcagcagaattccatttaatcaagctttagtcttttctaatttgcacagcagagcacaacatttggctgatatcctttcttctaaaggctttcctgctgagtgcatttcaggcaatatgaatcagaatcagcgtcttgatgctatggctaaactgaagcactttcattgcagagtcctcatttccacagatttgacttctcgtgggattgatgctgagaaggtgaatctggttgtaaatctggatgtaccattggattgggagacatacatgcatcggattgggagagctggccgttttggtacattggggctgacagtgacctactgttgccggggagaggaagaaaatatgatgatgagaattgcccagaaatgtaatatcaaccttctccctttaccagatcccattccttctggtctgatggaagaatgtgtggattgggatgtggaagttaaagctgctgtgcatacatatggtatagcaagtgtacctaaccaacccttaaaaaagcaaattcagaaaatagagagaacccttcaaattcagaaagctcatggtgaccacatggcttcctctagaaataattctgtatctggactatcagtcaaatcaaaaaataataccaaacaaaagcttcctgtgaaaagccactcagaatgtggaatcatagaaaaagcaacgtcaccaaaagaactgggctgtgacaggcaatccgaagagcaaatgaagaattctgttcagactcccgttgaaaactccaccaacagtcagcaccaggtcaaagaagctttacctgtgtcactcccccagattccttgtctgtcttcctttaaaatccatcagccatacacgttgacttttgctgaattggtagaggattatgaacattatattaaagaggggttagagaaacctgtggaaatcatcaggcactacacaggccctggggatcagactgtgaatcctcaaaatggttttgtgagaaataaagttattgaacagagagtccctgtgttggcaagtagtagccaatctggagactctgagagtgacagtgattcttacagctcaagaacctcttcccagagcaaaggaaataagtcatacttggaaggctcttctgataatcagctgaaagactctgaatctacgcctgtggatgatcgtatttctttggaacaaccaccaaatggaagtgacacccccaatccagagaaatatcaagaatcacctggaatccagatgaagacaagacttaaagagggggctagccagagagctaagcagagccggagaaacctacccaggcggtcttccttcagattgcagactgaagcccaggaagatgattggtatgactgtcatagggaaatacgtctgagtttttctgatacctatcaggattatgaggagtactggagagcttactacagggcatggcaagaatattatgctgccgcttctcattcatattattggaatgctcagagacatccaagttggatggcagcttatcacatgaataccatttatctacaagaaatgatgcatagtaaccagtga

SEQ ID NO: 70 - DNA, 3679 bp, synthetic construct
  source 1..3679: mol_type = other DNA
ggcctaactggccggtacctgagtctaaatgagtcttcggacctcgcgggggccgcttaagcggtggttagggtttgtctgacgcggggggagggggaaggaacgaaacactctcattcggaggcggctcggggtttggtcttggtggccacgggcacgcagaagagcgccgcgatcctcttaagcacccccccgccctccgtggaggcgggggtttggtcggcgggtggtaactggcgggccgctgactcgggcgggtcgcgcgccccagagtgtgaccttttcggtctgctcgcagacccccgggcggcgccgccgcggcggcgacgggctcgctgggtcctaggctccatggggaccgtatacgtggacaggctctggagcatccgcacgactgcggtgatattaccggagaccttctgcgggacgagccgggtcacgcggctgacgcggagcgtccgttgggcgacaaacaccaggacggggcacaggtacactatcttgtcacccggaggcgcgagggactgcaggagcttcagggagtggcgcagctgcttcatccccgtggcccgttgctcgcgtttgctggcggtgtccccggaagaaatatatttgcatgtctttagttctatgatgacacaaaccccgcccagcgtcttgtcattggcgaagtcgaacacgcagatgcagtcggggcggcgcggtcccaggtccacttcgcatattaaggtgacgcgtgtggcctcgaacaccgagcgaccctgcagcgacccgcttaaaagcttggcaatccggtactgttggtaaagccaccatggtcttcacactcgaagatttcgttggggactgggaacagacagccgcctacaacctggaccaagtccttgaacagggaggtgtgtccagtttgctgcagaatctcgccgtgtccgtaactccgatccaaaggattgtccggagcggtgaaaatgccctgaagatcgacatccatgtcatcatcccgtatgaaggtctgagcgccgaccaaatggcccagatcgaagaggtgtttaaggtggtgtaccctgtggatgatcatcactttaaggtgatcctgccctatggcacactggtaatcgacggggttacgccgaacatgctgaactatttcggacggccgtatgaaggcatcgccgtgttcgacggcaaaaagatcactgtaacagggaccctgtggaacggcaacaaaattatcgacgagcgcctgatcacccccgacggctccatgctgttccgagtaaccatcaacagtgggagttccggtggtggcgggagcggaggtggaggcatgccgggaaaactccgtagtgacgctggtttggaatcagacaccgcaatgaaaaaaggggagacactgcgaaagcaaaccgaggagaaagagaaaaaagagaagccaaaatctgataagactgaagagatagcagaagaggaagaaactgttttccccaaagctaaacaagttaaaaagaaagcagagccttctgaagttgacatgaattctcctaaatccaaaaaggcaaaaaagaaagaggagccatctcaaaatgacatttctcctaaaaccaaaagtttgagaaagaaaaaggagcccattgaaaagaaagtggtttcttctaaaaccaaaaaagtgacaaaaaatgaggagccttctgaggaagaaatagatgctcctaagcccaagaagatgaagaaagaaaaggaaatgaatggagaaactagagagaaaagccccaaactgaagaatggatttcctcatcctgaaccggactgtaaccccagtgaagctgccagtgaagaaagtaacagtgagatagagcaggaaatacctgtggaacaaaaagaaggcgctttctctaattttcccatatctgaagaaactattaaacttctcaaaggccgaggagtgaccttcctatttcctatacaagcaaagacattccatcatgtttacagcgggaaggacttaattgcacaggcacggacaggaactgggaagacattctcctttgccatccctttgattgagaaacttcatggggaactgcaagacaggaagagaggccgtgcccctcaggtactggttcttgcacctacaagagagttggcaaatcaagtaagcaaagacttcagtgacatcacaaaaaagctgtcagtggcttgtttttatggtggaactccctatggaggtcaatttgaacgcatgaggaatgggattgatatcctggttggaacaccaggtcgtatcaaagaccacatacagaatggcaaactagatctcaccaaacttaagcatgttgtcctggatgaagtggaccagatgttggatatgggatttgctgatcaagtggaagagattttaagtgtggcatacaagaaagattctgaagacaatccccaaacattgcttttttctgcaacttgccctcattgggtatttaatgttgccaagaaatacatgaaatctacatatgaacaggtggacctgattggtaaaaagactcagaaaacggcaataactgtggagcatctggctattaagtgccactggactcagagggcagcagttattggggatgtcatccgagtatatagtggtcatcaaggacgcactatcatcttttgtgaaaccaagaaagaagcccaggagctgtcccagaattcagctataaagcaggatgctcagtccttgcatggagacattccacagaagcaaagggaaatcaccctgaaaggttttagaaatggtagttttggagttttggtggcaaccaatgttgctgcacgtgggttagacatccctgaggttgatttggttatacaaagctctccaccaaaggatgtagagtcctacattcatcgatccgggcggacaggcagagctggaaggacgggggtgtgcatctgcttttatcagcacaaggaagaatatcagttagtacaagtggagcaaaaagcgggaattaagttcaaacgaataggtgttccttctgcaacagaaataataaaagcttccagcaaagatgccatcaggcttttggattccgtgcctcccactgccattagtcacttcaaacaatcagctgagaagctgatagaggagaagggagctgtggaagctctggcagcagcactggcccatatttcaggtgccacgtccgtagaccagcgctccttgatcaactcaaatgtgggttttgtgaccatgatcttgcagtgctcaattgaaatgccaaatattagttatgcttggaaagaacttaaagagcagctgggcgaggagattgattccaaagtgaagggaatggtttttctcaaaggaaagctgggtgtttgctttgatgtacctaccgcatcagtaacagaaatacaggagaaatggcatgattcacgacgctggcagctctctgtggccacagagcaaccagaactggaaggaccacgggaaggatatggaggcttcaggggacagcgggaaggcagtcgaggcttcaggggacagcgggacggaaacagaagattcagaggacagcgggaaggcagtagaggcccgagaggacagcgatcaggaggtggcaacaaaagtaacagatcccaaaacaaaggccagaagcggagtttcagtaaagcatttggtcaataa

SEQ ID NO: 71 - DNA, 3790 bp, synthetic construct
  source 1..3790: mol_type = other DNA
ggcctaactggccggtacctgagtctaaatgagtcttcggacctcgcgggggccgcttaagcggtggttagggtttgtctgacgcggggggagggggaaggaacgaaacactctcattcggaggcggctcggggtttggtcttggtggccacgggcacgcagaagagcgccgcgatcctcttaagcacccccccgccctccgtggaggcgggggtttggtcggcgggtggtaactggcgggccgctgactcgggcgggtcgcgcgccccagagtgtgaccttttcggtctgctcgcagacccccgggcggcgccgccgcggcggcgacgggctcgctgggtcctaggctccatggggaccgtatacgtggacaggctctggagcatccgcacgactgcggtgatattaccggagaccttctgcgggacgagccgggtcacgcggctgacgcggagcgtccgttgggcgacaaacaccaggacggggcacaggtacactatcttgtcacccggaggcgcgagggactgcaggagcttcagggagtggcgcagctgcttcatccccgtggcccgttgctcgcgtttgctggcggtgtccccggaagaaatatatttgcatgtctttagttctatgatgacacaaaccccgcccagcgtcttgtcattggcgaagtcgaacacgcagatgcagtcggggcggcgcggtcccaggtccacttcgcatattaaggtgacgcgtgtggcctcgaacaccgagcgaccctgcagcgacccgcttaaaagcttggcaatccggtactgttggtaaagccaccatggtcttcacactcgaagatttcgttggggactgggaacagacagccgcctacaacctggaccaagtccttgaacagggaggtgtgtccagtttgctgcagaatctcgccgtgtccgtaactccgatccaaaggattgtccggagcggtgaaaatgccctgaagatcgacatccatgtcatcatcccgtatgaaggtctgagcgccgaccaaatggcccagatcgaagaggtgtttaaggtggtgtaccctgtggatgatcatcactttaaggtgatcctgccctatggcacactggtaatcgacggggttacgccgaacatgctgaactatttcggacggccgtatgaaggcatcgccgtgttcgacggcaaaaagatcactgtaacagggaccctgtggaacggcaacaaaattatcgacgagcgcctgatcacccccgacggctccatgctgttccgagtaaccatcaacagtgggagttccggtggtggcgggagcggaggtggaggcatggcaggagagctggctgacaaaaaggaccgtgatgcatcaccttccaaggaggaaaggaagcgatcacggactcctgacagagagcgggatagagaccgggaccggaagtcttccccatctaaagatagaaagcggcatcgttcaagggatagacgtcgaggaggcagccgttctcgctctcgttcccgttccaaatctgcagaaagagaacgacggcacaaagaacgagaacgagataaggagcgggatcggaataagaaggaccgagatcgagacaaggatgggcacagacgggacaaggaccgtaaacgatccagcttatctcctggtcgaggaaaagactttaaatctcggaaggacagagactctaagaaggatgaagaggatgaacatggtgataagaagcctaaggcccagccattatccctggaggagcttctggccaagaaaaaggctgaggaagaagctgaggctaagcccaagttcctctctaaagcagaacgagaggctgaagctctaaagcgacggcagcaggaggtggaagagcggcagaggatgcttgaagaagagaggaagaaaaggaaacagttccaagacttgggcaggaagatgttggaagatcctcaggaacgggaacgtcgggaacgcagggagaggatggaacgggagaccaatggaaatgaggatgaggaagggcggcagaagatccgggaagagaaggataagagcaaggaactgcatgccattaaggagcgttacctgggtggcatcaaaaagcggcgccgaacgagacatctcaatgaccggaaatttgtttttgagtgggatgcatctgaggacacatccattgactacaaccccctgtacaaagaacggcaccaggtgcagttgttagggcgaggcttcattgcaggcattgacctcaagcagcagaagcgagagcagtcacgtttctatggagacctaatggagaagaggcgaaccctggaagaaaaggagcaggaggaggcaagactccgcaaacttcgtaagaaggaagccaagcagcgctgggatgatcgtcattggtctcagaaaaagttagatgagatgacggacagggactggcggatcttccgtgaggactacagcatcaccaccaaaggtggcaagatccccaatcccatccgatcctggaaagactcttctctgcccccacacatcttggaggtcattgataagtgtggctacaaggaaccaacacctatacagcgtcaggcaattcccattgggctacagaatcgtgacatcattggtgtggctgagactggcagtggcaagacagcagccttcctcatccctctgctggtctggatcaccacacttcccaaaattgacaggatcgaagagtcagaccaaggcccttatgccatcatcctggctcccacccgtgagttggctcaacagattgaggaagagaccatcaagtttgggaaaccgctaggtatccgcactgtggctgtcattggtggcatctccagagaagaccagggcttcaggctgcgcatgggttgtgagattgtgattgctacccctgggcgtttgattgatgtgctggagaaccgctacctggtgctgagccgctgtacctatgtggttctggatgaggcagataggatgattgacatgggctttgagccagatgtccagaagatcctggagcacatgcctgtcagcaaccagaagccagacacggatgaggctgaggaccctgagaagatgctggccaactttgagtcgggaaaacataagtaccgccaaacagtcatgttcacggccaccatgcccccagcggtggagcgtctggccaggagctatcttcggcgacctgctgtggtgtacattggctccgcaggcaagccccatgagcgtgtggaacagaaggtcttcctcatgtcagagtcagaaaagaggaaaaagctgctggcaatcttggagcaaggctttgacccacccatcattatttttgtcaaccagaagaagggctgcgacgtgttggccaaatccctggagaagatggggtacaatgcttgcacactgcacggtggaaaaggccaggagcagcgagagtttgcgttgtccaacctcaaggctggggccaaggatattttggtggctacagatgtggctggtcgtggtattgacatccaagatgtgtctatggttgtcaactatgatatggccaaaaatattgaagattacatccaccgcattggccgcacgggacgagcaggcaagagtggggtggccatcaccttcctcacaaaagaggactctgctgtgttctacgagctgaagcaagctatcctggaaagcccagtgtcttcctgtccccccgaactagccaaccacccagatgcccagcataagccaggcaccatcctcaccaagaagcgccgggaagagaccatctttgcctga

SEQ ID NO: 72 - DNA, 3907 bp, synthetic construct
  source 1..3907: mol_type = other DNA
ggcctaactggccggtacctgagtctaaatgagtcttcggacctcgcgggggccgcttaagcggtggttagggtttgtctgacgcggggggagggggaaggaacgaaacactctcattcggaggcggctcggggtttggtcttggtggccacgggcacgcagaagagcgccgcgatcctcttaagcacccccccgccctccgtggaggcgggggtttggtcggcgggtggtaactggcgggccgctgactcgggcgggtcgcgcgccccagagtgtgaccttttcggtctgctcgcagacccccgggcggcgccgccgcggcggcgacgggctcgctgggtcctaggctccatggggaccgtatacgtggacaggctctggagcatccgcacgactgcggtgatattaccggagaccttctgcgggacgagccgggtcacgcggctgacgcggagcgtccgttgggcgacaaacaccaggacggggcacaggtacactatcttgtcacccggaggcgcgagggactgcaggagcttcagggagtggcgcagctgcttcatccccgtggcccgttgctcgcgtttgctggcggtgtccccggaagaaatatatttgcatgtctttagttctatgatgacacaaaccccgcccagcgtcttgtcattggcgaagtcgaacacgcagatgcagtcggggcggcgcggtcccaggtccacttcgcatattaaggtgacgcgtgtggcctcgaacaccgagcgaccctgcagcgacccgcttaaaagcttggcaatccggtactgttggtaaagccaccatggtcttcacactcgaagatttcgttggggactgggaacagacagccgcctacaacctggaccaagtccttgaacagggaggtgtgtccagtttgctgcagaatctcgccgtgtccgtaactccgatccaaaggattgtccggagcggtgaaaatgccctgaagatcgacatccatgtcatcatcccgtatgaaggtctgagcgccgaccaaatggcccagatcgaagaggtgtttaaggtggtgtaccctgtggatgatcatcactttaaggtgatcctgccctatggcacactggtaatcgacggggttacgccgaacatgctgaactatttcggacggccgtatgaaggcatcgccgtgttcgacggcaaaaagatcactgtaacagggaccctgtggaacggcaacaaaattatcgacgagcgcctgatcacccccgacggctccatgctgttccgagtaaccatcaacagtgggagttccggtggtggcgggagcggaggtggaggcatgaagttgaaggacacaaaatcaaggccaaagcagtcaagctgtggcaaatttcagacaaagggaatcaaagttgtgggaaaatggaaggaagtgaagattgacccaaatatgtttgcagatggacagatggatgacttggtgtgctttgaggaattgacagattaccagttggtctcccctgccaagaatccctccagtctcttctcaaaggaagcacccaagagaaaggcacaagctgtttcagaagaagaggaggaggaggagggaaagtctagctcaccaaagaaaaagatcaagttgaagaaaagtaaaaatgtagcaactgaaggaaccagtacccagaaagaatttgaagtgaaagatcctgagctggaggcccagggagatgacatggtttgtgatgatccggaggctggggagatgacatcagaaaacctggtccaaactgctccaaaaaagaagaaaaataaagggaaaaaagggttggagccttctcagagcactgctgccaaggtgcccaaaaaagcgaagacatggattcctgaagttcatgatcagaaagcagatgtgtcagcttggaaggacctgtttgttcccaggccggttctccgagcactcagctttctaggcttctctgcacccacaccaatccaagccctgaccttggcacctgccatccgtgacaaactggacatccttggggctgctgagacaggaagtgggaaaactcttgcctttgccatcccaatgattcatgcggtgttgcagtggcagaagaggaatgctgcccctcctccaagtaacaccgaagcaccacctggagagaccagaactgaggccggagctgagactagatcaccaggcaaggctgaagctgagtctgatgcattgcctgacgatactgtaattgagagtgaagcactgcccagtgatattgcagccgaggccagagccaagactggaggcactgtctcagaccaggcgttgctctttggtgacgatgatgctggtgaagggccttcttccctgatcagggagaaacctgttcccaaacagaatgagaatgaggaggaaaatcttgataaagagcagactggaaatctaaaacaggagttggatgacaaaagcgccacctgtaaggcatatccaaagcgtcctctgcttggactggttctgactcccactcgagagctggccgtccaggtcaaacagcacattgatgctgtggccaggtttacaggaattaaaactgctattttggttggtggaatgtccacgcagaaacagcagaggatgctgaaccgtcgtcctgagattgtggttgctactccaggccggctgtgggaattaattaaagaaaagcattatcatttgaggaaccttcggcagctcaggtgcctggtagtggatgaggctgaccggatggttgagaaaggccattttgctgagctctcacagctgctagagatgctcaatgactcccaatacaacccaaagagacaaacgcttgttttttctgccacactcaccctggtgcatcaggctcctgctcgaatccttcataagaagcacaccaagaaaatggataaaacagccaaacttgacctccttatgcagaaaattggcatgaggggcaagcccaaggtcattgacctcacaaggaatgaggccacggtggagacgctaacagagaccaagatccattgtgagactgatgagaaagacttctacttgtactacttcctgatgcagtatccaggccgcagcttagtgtttgccaacagtatctcctgcatcaaacgcctctctgggctcctcaaagtccttgatatcatgcccttgaccctgcatgcctgtatgcaccagaagcagaggctcagaaacctggagcagtttgcccgtctggaagactgtgttctcttggcaacagatgtggcagctcggggtctggatattcctaaagtccagcatgtcatccattaccaggtcccacgtacctcggagatttatgtccaccgaagtggtcgaactgctcgagctaccaatgaaggcctcagtctgatgctcattgggcctgaggatgtgatcaactttaagaagatttacaaaacgctcaagaaagatgaggatatcccactgttccccgtgcagacaaaatacatggatgtggtcaaggagcgaatccgtttagctcgacagattgagaaatctgagtatcggaacttccaggcttgcctgcacaactcttggattgagcaggcagcagctgccctggagattgagctggaagaagacatgtataagggaggaaaagctgaccagcaagaagaacgtcggagacaaaagcagatgaaggttctgaagaaggagctgcgccacctgctgtcccagccactgtttacggagagccagaaaaccaagtatcccactcagtctggcaagccgcccctgcttgtgtctgccccaagtaagagcgagtctgctttgagctgtctctccaagcagaagaagaagaagacaaagaagccgaaggagccacagccggaacagccacagccaagtacaagtgcaaattaa

SEQ ID NO: 73 - DNA, 2779 bp, synthetic construct
  source 1..2779: mol_type = other DNA
ggcctaactggccggtacctgagtctaaatgagtcttcggacctcgcgggggccgcttaagcggtggttagggtttgtctgacgcggggggagggggaaggaacgaaacactctcattcggaggcggctcggggtttggtcttggtggccacgggcacgcagaagagcgccgcgatcctcttaagcacccccccgccctccgtggaggcgggggtttggtcggcgggtggtaactggcgggccgctgactcgggcgggtcgcgcgccccagagtgtgaccttttcggtctgctcgcagacccccgggcggcgccgccgcggcggcgacgggctcgctgggtcctaggctccatggggaccgtatacgtggacaggctctggagcatccgcacgactgcggtgatattaccggagaccttctgcgggacgagccgggtcacgcggctgacgcggagcgtccgttgggcgacaaacaccaggacggggcacaggtacactatcttgtcacccggaggcgcgagggactgcaggagcttcagggagtggcgcagctgcttcatccccgtggcccgttgctcgcgtttgctggcggtgtccccggaagaaatatatttgcatgtctttagttctatgatgacacaaaccccgcccagcgtcttgtcattggcgaagtcgaacacgcagatgcagtcggggcggcgcggtcccaggtccacttcgcatattaaggtgacgcgtgtggcctcgaacaccgagcgaccctgcagcgacccgcttaaaagcttggcaatccggtactgttggtaaagccaccatggtcttcacactcgaagatttcgttggggactgggaacagacagccgcctacaacctggaccaagtccttgaacagggaggtgtgtccagtttgctgcagaatctcgccgtgtccgtaactccgatccaaaggattgtccggagcggtgaaaatgccctgaagatcgacatccatgtcatcatcccgtatgaaggtctgagcgccgaccaaatggcccagatcgaagaggtgtttaaggtggtgtaccctgtggatgatcatcactttaaggtgatcctgccctatggcacactggtaatcgacggggttacgccgaacatgctgaactatttcggacggccgtatgaaggcatcgccgtgttcgacggcaaaaagatcactgtaacagggaccctgtggaacggcaacaaaattatcgacgagcgcctgatcacccccgacggctccatgctgttccgagtaaccatcaacagtgggagttccggtggtggcgggagcggaggtggaggcatggcgtcgttactgtggggaggcgacgcaggggcggcggagagcgagcggctgaacagccacttttcaaacctcagccaaccccggaagaacctttggggtattaagagtactgcagtccgaaacatagatggttctattaataacatcaatgaagatgatgaagaagatgtagtggatttggcagctaattcactcttaaacaagttaatccatcaatccttagtagaatccagtcaccgtgtggaagttttacagaaggatcccagctctccactttactcagtaaagacatttgaagagctgcggctaaaggaagagttactaaaaggaatctatgcaatgggatttaataggccatctaaaatccaagagatggctctccctatgatgctggcacatccaccccagaacctcatagcacagagccagtctggaacaggaaagacagcggcatttgtgttggcaatgttaagcagagttaatgccttggaattgttcccacagtgcctctgcctagctcctacttatgaattggctctgcaaactggccgtgtggttgagcagatgggaaaattctgtgtggatgttcaagtgatgtatgccattcgagggaatcgaattcccagaggcaccgacatcactaaacagattataattggcactcctgggactgtcctagattggtgttttaaactaaaattgattgatttgactaagattcgtgtgtttgtcctggatgaagcagatgtgatgattgacactcaaggattctcagatcatagtattcgtattcaaagagctctaccctccgaatgccaaatgctcctcttttcagcaacctttgaggactctgtgtggcactttgctgagcgaatcatccctgaccctaatgttatcaagttacgcaaagaggagctcacactgaacaacatccggcaatattacgtgctgtgtgagcacaggaaagacaaataccaagctctgtgcaacatttatggcagcatcaccattggtcaggccatcatcttctgccagactcgtcgaaacgctaagtggttgaccgtggagatgatacaggatggccaccaggtgtctttgttaagcggggagctgaccgtggagcagcgagcttccatcattcagaggtttcgggatgggaaagagaaggttctcataacaactaatgtttgtgcccgagggattgatgtgaagcaggtcacaattgttgtgaactttgatctccctgtaaaacaaggagaggagccggactatgagacctacctccaccgcatagggcggacggggcgctttgggaaaaaaggccttgccttcaacatgattgaagtagatgagctgccctcgctcatgaaaatccaggaccactttaacagcagtattaagcaactcaacgctgaagacatggatgaaattgaaaagattgactattga

SEQ ID NO: 74 - DNA, 3625 bp, synthetic construct
  source 1..3625: mol_type = other DNA
ggcctaactggccggtacctgagtctaaatgagtcttcggacctcgcgggggccgcttaagcggtggttagggtttgtctgacgcggggggagggggaaggaacgaaacactctcattcggaggcggctcggggtttggtcttggtggccacgggcacgcagaagagcgccgcgatcctcttaagcacccccccgccctccgtggaggcgggggtttggtcggcgggtggtaactggcgggccgctgactcgggcgggtcgcgcgccccagagtgtgaccttttcggtctgctcgcagacccccgggcggcgccgccgcggcggcgacgggctcgctgggtcctaggctccatggggaccgtatacgtggacaggctctggagcatccgcacgactgcggtgatattaccggagaccttctgcgggacgagccgggtcacgcggctgacgcggagcgtccgttgggcgacaaacaccaggacggggcacaggtacactatcttgtcacccggaggcgcgagggactgcaggagcttcagggagtggcgcagctgcttcatccccgtggcccgttgctcgcgtttgctggcggtgtccccggaagaaatatatttgcatgtctttagttctatgatgacacaaaccccgcccagcgtcttgtcattggcgaagtcgaacacgcagatgcagtcggggcggcgcggtcccaggtccacttcgcatattaaggtgacgcgtgtggcctcgaacaccgagcgaccctgcagcgacccgcttaaaagcttggcaatccggtactgttggtaaagccaccatggtcttcacactcgaagatttcgttggggactgggaacagacagccgcctacaacctggaccaagtccttgaacagggaggtgtgtccagtttgctgcagaatctcgccgtgtccgtaactccgatccaaaggattgtccggagcggtgaaaatgccctgaagatcgacatccatgtcatcatcccgtatgaaggtctgagcgccgaccaaatggcccagatcgaagaggtgtttaaggtggtgtaccctgtggatgatcatcactttaaggtgatcctgccctatggcacactggtaatcgacggggttacgccgaacatgctgaactatttcggacggccgtatgaaggcatcgccgtgttcgacggcaaaaagatcactgtaacagggaccctgtggaacggcaacaaaattatcgacgagcgcctgatcacccccgacggctccatgctgttccgagtaaccatcaacagtgggagttccggtggtggcgggagcggaggtggaggcatgcttgcggacctcggcttaatcggaaccataggcgaggatgacgaggtgccggtggagcccgagtctgactccggggacgaggaagaggaggggcccattgtgctgggcagacgacaaaaagctttggggaagaaccgcagtgctgatttcaaccctgatttcgttttcactgagaaggaggggacgtacgatggcagctgggccctggctgatgtcatgagccaactcaagaagaagagggcagccactacattagatgagaagattgagaaagttcgaaagaaaaggaaaacagaggataaagaagccaagtctgggaagttggaaaaggagaaagaagcaaaggaaggctctgaaccaaaggagcaggaagaccttcaagagaatgatgaggaaggctcagaagatgaagcctcggagactgactactcatcagctgatgagaacatcctcaccaaagcagatacactcaaagtaaaggatcggaagaagaagaagaagaaaggacaggaagcaggaggattttttgaagatgcatctcagtacgatgaaaacctctcgttccaggacatgaacctttcccgccctcttctgaaggccattacagccatgggcttcaagcagcccaccccgatccagaaggcgtgcatacctgtgggtctattggggaaggacatctgtgcctgtgcagccactgggacaggtaaaactgccgcctttgccctgcctgttttggagcgtctgatttataaaccccgccaggctccagtcacccgcgtgctggtgctagtgcccacccgagagctgggcatccaggtgcactctgtcaccagacagctggcccagttctgcaacatcaccacctgcctggctgtgggcggcttggatgtgaagtctcaggaagcagctcttcgggcagcgcctgacatcctcatcgccaccccaggccggctcatcgatcacctccacaactgcccttccttccacctgagcagcatcgaggtgctcatcctggacgaggctgacaggatgctggatgagtactttgaggagcagatgaaggagatcatccgaatgtgttcccaccaccgccagaccatgctcttctcggccaccatgacagacgaggtgaaagatctggcttctgtctccttgaagaatcctgtccggatatttgtgaacagcaacacagatgtggctcccttcctgcggcaggagttcatccggatccggcctaatcgtgaaggagaccgggaagccatcgtggcagctttgttgacgaggaccttcactgaccatgtgatgctgttcacgcaaaccaagaagcaggcccaccgcatgcacatcctcctggggctcatggggctgcaggtgggtgagctccatggcaacttgtcacagacgcagcggctggaggccctccggcgttttaaggatgaacagattgacatcctcgtggccactgatgtggcagcccgtggacttgacattgagggggtcaaaacggtaatcaacttcacaatgcctaataccatcaaacattatgtccaccgggtggggcgaacagcacgtgctggcagggctgggcgctcagtctctctggtgggagaagatgagcggaagatgctgaaggagattgtaaaagctgccaaggcccctgtgaaggccaggatacttccccaagatgtcatcctcaaattccgggacaagattgagaaaatggagaaagatgtgtatgcagttctgcagctagaggcggaggaaaaagagatgcagcagtcagaagcccagatcaatacagcaaagcggctcctggagaaggggaaggaggcagtggtccaagagcccgagaggagctggttccagaccaaagaagagaggaagaaggagaaaattgccaaagctctgcaggaatttgacttggccttaagaggaaagaagaaaaggaagaagtttatgaaggatgccaaaaaaaagggggagatgacagcagaggaaaggtctcagtttgaaatcctcaaggcgcagatgtttgctgaacggctagcgaagaggaatcgcagagccaagcgggcccgagcaatgcccgaggaggagccagtgagaggtcctgccaagaagcaaaagcaggggaagaaatctgtatttgatgaagaactcaccaacacaagcaagaaggccctgaaacagtatcgagctggcccttcctttgaagaaaggaaacagttgggcttgccccaccagagacgaggaggaaactttaaatctaaatccagatacaagaggaggaagtag

SEQ ID NO: 75 - DNA, 2950 bp, synthetic construct
  source 1..2950: mol_type = other DNA
ggcctaactggccggtacctgagtctaaatgagtcttcggacctcgcgggggccgcttaagcggtggttagggtttgtctgacgcggggggagggggaaggaacgaaacactctcattcggaggcggctcggggtttggtcttggtggccacgggcacgcagaagagcgccgcgatcctcttaagcacccccccgccctccgtggaggcgggggtttggtcggcgggtggtaactggcgggccgctgactcgggcgggtcgcgcgccccagagtgtgaccttttcggtctgctcgcagacccccgggcggcgccgccgcggcggcgacgggctcgctgggtcctaggctccatggggaccgtatacgtggacaggctctggagcatccgcacgactgcggtgatattaccggagaccttctgcgggacgagccgggtcacgcggctgacgcggagcgtccgttgggcgacaaacaccaggacggggcacaggtacactatcttgtcacccggaggcgcgagggactgcaggagcttcagggagtggcgcagctgcttcatccccgtggcccgttgctcgcgtttgctggcggtgtccccggaagaaatatatttgcatgtctttagttctatgatgacacaaaccccgcccagcgtcttgtcattggcgaagtcgaacacgcagatgcagtcggggcggcgcggtcccaggtccacttcgcatattaaggtgacgcgtgtggcctcgaacaccgagcgaccctgcagcgacccgcttaaaagcttggcaatccggtactgttggtaaagccaccatggtcttcacactcgaagatttcgttggggactgggaacagacagccgcctacaacctggaccaagtccttgaacagggaggtgtgtccagtttgctgcagaatctcgccgtgtccgtaactccgatccaaaggattgtccggagcggtgaaaatgccctgaagatcgacatccatgtcatcatcccgtatgaaggtctgagcgccgaccaaatggcccagatcgaagaggtgtttaaggtggtgtaccctgtggatgatcatcactttaaggtgatcctgccctatggcacactggtaatcgacggggttacgccgaacatgctgaactatttcggacggccgtatgaaggcatcgccgtgttcgacggcaaaaagatcactgtaacagggaccctgtggaacggcaacaaaattatcgacgagcgcctgatcacccccgacggctccatgctgttccgagtaaccatcaacagtgggagttccggtggtggcgggagcggaggtggaggcatggctctaacgcggccggtgcggctcttttccctcgtgactcggttgctcctggcgccgcgacggggcctcacggtccgcagtcccgacgaacccctgccggtggtgcgcatcccagtggctctacagcggcagttggaacagcggcagagcaggcggcggaacctcccgaggccggtgctggttcgacccggaccgctgctggtttcggcgcggcggccggagttgaaccagccggcgcgcctcacactgggccgttgggagcgcgcgccgctagcctctcaaggctggaagagtcgacgcgcgcgtcgggaccacttctccatcgagcgcgcgcaacaggaggcgccagcggtgcgaaagctctcgtctaagggcagctttgctgacctgggcctggagccccgtgtgctgcacgcactacaggaggctgcgcctgaagtcgttcagcccacaaccgtgcagtctagcaccatcccctcactacttcgcggccgccatgtcgtttgcgccgcagaaaccggcagtggcaagactctcagctacctcctgccgctgcttcaacggctcttgggccagccaagcctggactcccttcctatccccgcgccccgaggcctggtccttgttccttcccgagaattggcccaacaggtgcgggctgtggcccaacccttgggccgctccttgggcctgctggtgcgggacctggagggaggccacggcatgcgtaggatcaggctgcagctgtccagacagccttcagcagatgtgcttgtggccactccaggggctctgtggaaggccctgaaaagtcgactgatcagtctggagcaactctccttcttggtgttggatgaggcagacacactgctggatgaaagcttcctggaactggtggactacatcttagagaagagccacatagcagaaggcccagctgacttggaagaccccttcaatcccaaagctcagttagtgctggtaggagccacatttcccgaaggtgtaggccagttgctgaataaagtcgccagcccagatgctgtcaccaccatcaccagctccaagctccactgtatcatgcctcatgtgaaacagacatttctgagactgaagggagcagataaggtggccgagctggtgcacatcctcaagcatcgtgacagagcagaaaggactggtccctcaggaactgttctggtgttctgtaatagctccagcactgtgaactggctgggatatattctggatgaccacaaaatccaacacctaaggttgcaggggcaaatgccagccttgatgagggtaggaatcttccagtccttccagaagagctcccgagacatacttctctgcacagacatagcctctcggggcctggacagcactggtgtggagctggttgtcaattatgatttccccccaacgctgcaagattacatccacagagcagggagagtgggccgtgtggggagcgaggtgccaggcaccgtcatcagttttgtgacccatccctgggatgtgagcctggttcagaagattgagctggcggctcgccgaaggagaagtcttccaggactagcatcctcggtgaaagagcctttgccccaagcaacctga

SEQ ID NO: 76 - DNA, 3568 bp, synthetic construct
  source 1..3568: mol_type = other DNA
ggcctaactggccggtacctgagtctaaatgagtcttcggacctcgcgggggccgcttaagcggtggttagggtttgtctgacgcggggggagggggaaggaacgaaacactctcattcggaggcggctcggggtttggtcttggtggccacgggcacgcagaagagcgccgcgatcctcttaagcacccccccgccctccgtggaggcgggggtttggtcggcgggtggtaactggcgggccgctgactcgggcgggtcgcgcgccccagagtgtgaccttttcggtctgctcgcagacccccgggcggcgccgccgcggcggcgacgggctcgctgggtcctaggctccatggggaccgtatacgtggacaggctctggagcatccgcacgactgcggtgatattaccggagaccttctgcgggacgagccgggtcacgcggctgacgcggagcgtccgttgggcgacaaacaccaggacggggcacaggtacactatcttgtcacccggaggcgcgagggactgcaggagcttcagggagtggcgcagctgcttcatccccgtggcccgttgctcgcgtttgctggcggtgtccccggaagaaatatatttgcatgtctttagttctatgatgacacaaaccccgcccagcgtcttgtcattggcgaagtcgaacacgcagatgcagtcggggcggcgcggtcccaggtccacttcgcatattaaggtgacgcgtgtggcctcgaacaccgagcgaccctgcagcgacccgcttaaaagcttggcaatccggtactgttggtaaagccaccatggtcttcacactcgaagatttcgttggggactgggaacagacagccgcctacaacctggaccaagtccttgaacagggaggtgtgtccagtttgctgcagaatctcgccgtgtccgtaactccgatccaaaggattgtccggagcggtgaaaatgccctgaagatcgacatccatgtcatcatcccgtatgaaggtctgagcgccgaccaaatggcccagatcgaagaggtgtttaaggtggtgtaccctgtggatgatcatcactttaaggtgatcctgccctatggcacactggtaatcgacggggttacgccgaacatgctgaactatttcggacggccgtatgaaggcatcgccgtgttcgacggcaaaaagatcactgtaacagggaccctgtggaacggcaacaaaattatcgacgagcgcctgatcacccccgacggctccatgctgttccgagtaaccatcaacagtgggagttccggtggtggcgggagcggaggtggaggcatggcagccgccgacggttcgctcttcgacaaccccaggacgttctccagacgtcccccagcccaggcgagtcggcaagcaaaggctacgaaaagaaaataccaagcgtccagtgaggctcccccagcgaaacggaggaacgaaacttcatttctcccagccaagaaaactagtgttaaagaaactcagaggacttttaaggggaacgcacaaaaaatgttttctccaaagaagcattcggttagcacaagtgatagaaaccaggaggagagacagtgcattaagacttcatcactgtttaaaaacaaccctgacattccagaactccacagacctgtggtaaagcaggtgcaagaaaaagtgtttacttcagctgcttttcatgagctgggcctccacccacatttaatttccacaataaatacggtcttaaaaatgtctagtatgaccagtgttcagaagcaaagtattcctgtgttgctggaaggcagagatgctctcgtgagatcccagacgggctcaggtaaaactcttgcctattgcatccctgtggtccagtcccttcaagcaatggagtcaaaaatacagcgcagtgatggcccctatgccctggtgctcgtgccaacgagagagctagctctacaaagctttgacactgtccagaaactgcttaagcctttcacctggattgtgcctggagtgttaatgggaggagagaagagaaaatcagaaaaggccagactccgcaaaggaataaatatccttatctcaactcctggacgcctggtggatcatataaaatccacaaagaacattcattttagtcggctgcggtggttggtgtttgatgaagcagacagaatcttggatttgggttttgaaaaggacatcacagtgatacttaatgctgtaaatgctgaatgccaaaaacgacagaatgtcttgctatcagcgacactcacagaaggtgtaacgcggctagctgatatcagtttgcatgatccagtcagtatttctgtcctggacaagagccatgaccagttgaacccaaaggacaaagcggtccaggaggtctgtcctccaccagctggcgacaagctggacagctttgcaataccagagagtctcaagcagcatgtgactgtggttcccagcaaactgaggcttgtctgcctagcggccttcatccttcagaaatgcaagtttgaggaagaccagaagatggttgtctttttctcaagttgcgagctggtggagttccactacagcctcttcctacagaccctgctgagcagctcaggggcgccggcatcagggcagttgccatctgcctccatgcgattaaaattcctacggctgcatggcggcatggagcaggaggaaagaacagcagtgtttcaggaattttcacattccagaagaggcgtccttctttgcacggatgttgcagctcggggcttagatctccctcaagtcacgtggattgttcagtacaacgctccatcttcacctgcagaatacatccaccggattggaagaaccgcccggattggctgccatgggagcagcctgctcattttggctccttcggaggcagaatatgtcaactcgttggcttctcacaaaatcaacgtttctgagattaagatggaagatattttgtgtgttctgacaagagatgattgttttaaagggaaacgatggggagcccagaaatcccatgctgttggcccccaggaaatccgagagcgagccacagtcttgcagacggtatttgaagattacgtgcactccagtgagaggagggtctcctgggcaaagaaagctctgcagtccttcatccaagcctacgccacctaccccagggagctgaagcacatcttccacgtccgatccctccaccttgggcatgtggcgaagagcttcggactaagagatgcccccaggaatcttagtgccttgactagaaagaagaggaaagcacacgtgaaaaggcctgaccttcataagaagacccagagtaaacacagcctcgctgaaatcctacgttcggaatactcaagcggcatggaggccgacatcgccaaggtcaaaaagcaaaacgcacctggagagcctggtggccggcccctgcagcacagtctgcagccgacaccctgctttggccgtgggaaaacattaaaatggagaaaaacccaaaaaggtgtacagcgggacagcaagacttcccagaaagtttaa

SEQ ID NO: 77 - DNA, 2614 bp, synthetic construct
  source 1..2614: mol_type = other DNA
ggcctaactggccggtacctgagtctaaatgagtcttcggacctcgcgggggccgcttaagcggtggttagggtttgtctgacgcggggggagggggaaggaacgaaacactctcattcggaggcggctcggggtttggtcttggtggccacgggcacgcagaagagcgccgcgatcctcttaagcacccccccgccctccgtggaggcgggggtttggtcggcgggtggtaactggcgggccgctgactcgggcgggtcgcgcgccccagagtgtgaccttttcggtctgctcgcagacccccgggcggcgccgccgcggcggcgacgggctcgctgggtcctaggctccatggggaccgtatacgtggacaggctctggagcatccgcacgactgcggtgatattaccggagaccttctgcgggacgagccgggtcacgcggctgacgcggagcgtccgttgggcgacaaacaccaggacggggcacaggtacactatcttgtcacccggaggcgcgagggactgcaggagcttcagggagtggcgcagctgcttcatccccgtggcccgttgctcgcgtttgctggcggtgtccccggaagaaatatatttgcatgtctttagttctatgatgacacaaaccccgcccagcgtcttgtcattggcgaagtcgaacacgcagatgcagtcggggcggcgcggtcccaggtccacttcgcatattaaggtgacgcgtgtggcctcgaacaccgagcgaccctgcagcgacccgcttaaaagcttggcaatccggtactgttggtaaagccaccatggtcttcacactcgaagatttcgttggggactgggaacagacagccgcctacaacctggaccaagtccttgaacagggaggtgtgtccagtttgctgcagaatctcgccgtgtccgtaactccgatccaaaggattgtccggagcggtgaaaatgccctgaagatcgacatccatgtcatcatcccgtatgaaggtctgagcgccgaccaaatggcccagatcgaagaggtgtttaaggtggtgtaccctgtggatgatcatcactttaaggtgatcctgccctatggcacactggtaatcgacggggttacgccgaacatgctgaactatttcggacggccgtatgaaggcatcgccgtgttcgacggcaaaaagatcactgtaacagggaccctgtggaacggcaacaaaattatcgacgagcgcctgatcacccccgacggctccatgctgttccgagtaaccatcaacagtgggagttccggtggtggcgggagcggaggtggaggcatggcagagaacgatgtggacaatgagctcttggactatgaagatgatgaggtggagacagcagctgggggagatggggctgaggcccctgccaagaaggatgtcaagggctcctatgtctccatccacagctctggctttcgtgacttcctgctcaagccagagttgctccgggccattgtcgactgtggctttgagcatccgtcagaagtccagcatgagtgcatccctcaggccattctgggaatggatgtcctgtgccaggccaagtcgggcatgggaaagacagcagtgtttgtcttggccacactgcaacagctggagccagttactgggcaggtgtctgtactggtgatgtgtcacactcgggagttggcttttcagatcagcaaggaatatgagcgcttctctaaatacatgcccaatgtcaaggttgctgttttttttggtggtctgtctatcaagaaggatgaagaggtgctgaagaagaactgcccgcatatcgtcgtggggactccaggccgtatcctagccctggctcgaaataagagcctcaacctcaaacacattaaacactttattttggatgaatgtgataagatgcttgaacagctcgacatgcgtcgggatgtccaggaaatttttcgcatgaccccccacgagaagcaggtcatgatgttcagtgctaccttgagcaaagagatccgtccagtctgccgcaagttcatgcaagatccaatggagatcttcgtggatgatgagacgaagttgacgctgcatgggttgcagcagtactacgtgaaactgaaggacaacgagaagaaccggaagctctttgaccttctggatgtccttgagttcaaccaggtggtgatctttgtgaagtctgtgcagcggtgcattgccttggcccagctactagtggagcagaacttcccagccattgccatccaccgtgggatgccccaggaggagaggctttctcggtatcagcagtttaaagattttcaacgacgaattcttgtggctaccaacctatttggccgaggcatggacatcgagcgggtgaacattgcttttaattatgacatgcctgaggattctgacacctacctgcatcgggtggccagagcaggccggtttggcaccaagggcttggctatcacatttgtgtccgatgagaatgatgccaagatcctcaatgatgtgcaggatcgctttgaggtcaatattagtgagctgcctgatgagatagacatctcctcctacattgaacagacacggtag

SEQ ID NO: 78 - DNA, 3196 bp, synthetic construct
  source 1..3196: mol_type = other DNA
ggcctaactggccggtacctgagtctaaatgagtcttcggacctcgcgggggccgcttaagcggtggttagggtttgtctgacgcggggggagggggaaggaacgaaacactctcattcggaggcggctcggggtttggtcttggtggccacgggcacgcagaagagcgccgcgatcctcttaagcacccccccgccctccgtggaggcgggggtttggtcggcgggtggtaactggcgggccgctgactcgggcgggtcgcgcgccccagagtgtgaccttttcggtctgctcgcagacccccgggcggcgccgccgcggcggcgacgggctcgctgggtcctaggctccatggggaccgtatacgtggacaggctctggagcatccgcacgactgcggtgatattaccggagaccttctgcgggacgagccgggtcacgcggctgacgcggagcgtccgttgggcgacaaacaccaggacggggcacaggtacactatcttgtcacccggaggcgcgagggactgcaggagcttcagggagtggcgcagctgcttcatccccgtggcccgttgctcgcgtttgctggcggtgtccccggaagaaatatatttgcatgtctttagttctatgatgacacaaaccccgcccagcgtcttgtcattggcgaagtcgaacacgcagatgcagtcggggcggcgcggtcccaggtccacttcgcatattaaggtgacgcgtgtggcctcgaacaccgagcgaccctgcagcgacccgcttaaaagcttggcaatccggtactgttggtaaagccaccatggtcttcacactcgaagatttcgttggggactgggaacagacagccgcctacaacctggaccaagtccttgaacagggaggtgtgtccagtttgctgcagaatctcgccgtgtccgtaactccgatccaaaggattgtccggagcggtgaaaatgccctgaagatcgacatccatgtcatcatcccgtatgaaggtctgagcgccgaccaaatggcccagatcgaagaggtgtttaaggtggtgtaccctgtggatgatcatcactttaaggtgatcctgccctatggcacactggtaatcgacggggttacgccgaacatgctgaactatttcggacggccgtatgaaggcatcgccgtgttcgacggcaaaaagatcactgtaacagggaccctgtggaacggcaacaaaattatcgacgagcgcctgatcacccccgacggctccatgctgttccgagtaaccatcaacagtgggagttccggtggtggcgggagcggaggtggaggcatggaggagtcggaacccgaacggaagcgggctcgcaccgacgaggtgcctgccggaggaagccgctccgaggcggaagatgaggacgacgaggactacgtgccctatgtgccgttacggcagcgccggcagctactgctccagaagctgctgcagcgaagacgcaagggagctgcggaggaagagcagcaggacagcggtagtgaaccccggggagatgaggacgacatcccgctaggccctcagtccaacgtcagcctcctggatcagcaccagcaccttaaagagaaggctgaagcgcgcaaagagtctgccaaggagaagcagctgaaggaagaagagaagatcctggagagtgttgccgagggccgagcattgatgtcagtgaaggagatggctaagggcattacgtatgatgaccccatcaaaaccagctggactccaccccgttatgttctgagcatgtctgaagagcgacatgagcgcgtgcggaagaaataccacatcctggtggagggagacggtatcccaccacccatcaagagcttcaaggaaatgaagtttcctgcagccatcctgagaggcctgaagaagaaaggcattcaccacccaacacccattcagatccagggcatccccaccattctatctggccgtgacatgataggcatcgctttcacgggttcaggcaagacactggtgttcacgttgcccgtcatcatgttctgcctggaacaagagaagaggttacccttctcaaagcgcgaggggccctatggactcatcatctgcccctcgcgggagctggcccggcagacccatggcatcctggagtactactgccgcctgctgcaggaggacagctcaccactcctgcgctgcgccctctgcattgggggcatgtccgtgaaagagcagatggagaccatccgacacggtgtacacatgatggtggccaccccggggcgcctcatggatttgctgcagaagaagatggtcagcctagacatctgtcgctacctggccctggacgaggctgaccgcatgatcgacatgggcttcgagggtgacatccgtaccatcttctcctacttcaagggccagcgacagaccctgctcttcagtgccaccatgccgaagaagattcagaactttgctaagagtgcccttgtaaagcctgtgaccatcaatgtggggcgcgctggggctgccagcctggatgtcatccaggaggtagaatatgtgaaggaggaggccaagatggtgtacctgctcgagtgcctgcagaagacacccccgcctgtactcatctttgcagagaagaaggcagacgtggacgccatccacgagtacctgctgctcaagggggttgaggccgtagccatccatgggggcaaagaccaggaggaacggactaaggccatcgaggcattccgggagggcaagaaggatgtcctagtagccacagacgttgcctccaagggcctggacttccctgccatccagcacgtcatcaattatgacatgccagaggagattgagaactatgtacaccggattggccgcaccgggcgctcgggaaacacaggcatcgccactaccttcatcaacaaagcgtgtgatgagtcagtgctgatggacctcaaagcgctgctgctagaagccaagcagaaggtgccgcccgtgctgcaggtgctgcattgcggggatgagtccatgctggacattggaggagagcgcggctgtgccttctgcgggggcctgggtcatcggatcactgactgccccaaactcgaggctatgcagaccaagcaggtcagcaacatcggtcgcaaggactacctggcccacagctccatggacttctga

SEQ ID NO: 79 - DNA, 4144 bp, synthetic construct
  source 1..4144: mol_type = other DNA
ggcctaactggccggtacctgagtctaaatgagtcttcggacctcgcgggggccgcttaagcggtggttagggtttgtctgacgcggggggagggggaaggaacgaaacactctcattcggaggcggctcggggtttggtcttggtggccacgggcacgcagaagagcgccgcgatcctcttaagcacccccccgccctccgtggaggcgggggtttggtcggcgggtggtaactggcgggccgctgactcgggcgggtcgcgcgccccagagtgtgaccttttcggtctgctcgcagacccccgggcggcgccgccgcggcggcgacgggctcgctgggtcctaggctccatggggaccgtatacgtggacaggctctggagcatccgcacgactgcggtgatattaccggagaccttctgcgggacgagccgggtcacgcggctgacgcggagcgtccgttgggcgacaaacaccaggacggggcacaggtacactatcttgtcacccggaggcgcgagggactgcaggagcttcagggagtggcgcagctgcttcatccccgtggcccgttgctcgcgtttgctggcggtgtccccggaagaaatatatttgcatgtctttagttctatgatgacacaaaccccgcccagcgtcttgtcattggcgaagtcgaacacgcagatgcagtcggggcggcgcggtcccaggtccacttcgcatattaaggtgacgcgtgtggcctcgaacaccgagcgaccctgcagcgacccgcttaaaagcttggcaatccggtactgttggtaaagccaccatggtcttcacactcgaagatttcgttggggactgggaacagacagccgcctacaacctggaccaagtccttgaacagggaggtgtgtccagtttgctgcagaatctcgccgtgtccgtaactccgatccaaaggattgtccggagcggtgaaaatgccctgaagatcgacatccatgtcatcatcccgtatgaaggtctgagcgccgaccaaatggcccagatcgaagaggtgtttaaggtggtgtaccctgtggatgatcatcactttaaggtgatcctgccctatggcacactggtaatcgacggggttacgccgaacatgctgaactatttcggacggccgtatgaaggcatcgccgtgttcgacggcaaaaagatcactgtaacagggaccctgtggaacggcaacaaaattatcgacgagcgcctgatcacccccgacggctccatgctgttccgagtaaccatcaacagtgggagttccggtggtggcgggagcggaggtggaggcatgaactggaataaaggtggtcctggcactaagcgaggatttggctttggaggttttgccatcagtgctgggaaaaaggaggaacccaaactcccacagcagtcccacagtgcctttggggcaaccagctcttcttctggatttggaaagtcagctccaccacagcttccttctttctacaaaattggatctaagcgggccaactttgatgaagaaaatgcctattttgaagatgaggaagaagattctagcaacgttgatttaccttacattcctgctgaaaactcaccaactcgccagcaattccattccaagccagtagattctgacagcgatgatgatcccttggaggcattcatggctgaagtggaggatcaggcagctagagacatgaagaggcttgaagaaaaggacaaggaaagaaaaaacgtaaagggtattcgagatgacattgaagaggaagatgaccaagaagcttattttcgatacatggcagaaaacccaactgctggtgtggttcaggaggaagaggaagacaatctagaatatgatagtgacggaaatccaattgcacctaccaaaaaaatcattgatcctcttccccccattgatcattcagagattgactatccaccatttgaaaaaaacttttacaatgagcatgaagagataaccaacctcactccacagcagttaatagatctccggcataagctcaatcttcgggtctctggtgctgcacctcctagaccaggaagtagctttgctcattttgggtttgacgaacaacttatgcaccagattcggaaatctgaatacacacagcccactccaatacagtgccagggtgtgcctgtggcattaagtggtagagacatgattggtattgccaaaacaggtagtgggaaaactgcagccttcatttggcccatgttgattcatataatggaccagaaggagttggaaccaggtgatggaccaattgcagtgattgtgtgtcctaccagggagctttgccagcagatccatgcagaatgtaagcggtttggaaaagcatataatcttcgatcagtggccgtatatggaggagggagtatgtgggagcaggccaaggcccttcaggagggggcagagattgttgtgtgtaccccaggtcgactgatagatcatgtgaaaaagaaagctaccaatcttcaaagagtctcttaccttgtgtttgatgaagcagatcgaatgtttgacatgggatttgagtaccaagttcgatccatagcaagtcatgttcgtcctgacaggcagactctcttatttagtgcaacttttcggaagaagattgaaaagttggccagagacatcctgatcgaccctattcgagtggtgcagggagatattggagaggcaaatgaagatgtgacacagattgtggagattctccattctggacctagtaaatggaactggcttacccggcgtctggtagaatttacctcttcagggagtgtcctcctctttgttactaaaaaagccaatgctgaagagctagcgaataaccttaaacaggagggtcataatcttgggctgctccatggggatatggatcagagtgagagaaacaaggtcatttcagactttaagaaaaaggacatcccagtcctggtggccacagatgttgcagcccgtggtctggacattccttcaattaagactgtcattaactatgatgtggcacgagacattgatacccacacgcataggattggccgcacaggaagagcgggtgagaaaggtgtggcctataccctactcactcccaaggacagcaattttgctggtgacctggtccggaacttggaaggagccaatcaacacgtttctaaggaactcctagatctggcaatgcagaatgcctggtttcggaaatctcgattcaaaggagggaaaggaaaaaagctgaacattggtggaggaggcctaggctacagggagcggcctggcctgggctctgagaacatggatcgaggaaataacaatgtaatgagcaattatgaggcctacaagccttccacaggagctatgggagatcgactaacggcaatgaaagcagctttccagtcacagtacaagagtcactttgttgcagccagtttaagtaatcagaaggctggaagttctgctgctggggcaagtgggtggactagtgcagggagcttgaattctgttccaactaactcagcacaacagggccataacagtcctgacagccccgtcaccagtgccgccaagggcatcccaggctttggcaatactggcaacatcagtggtgcccctgtgacctacccgtctgccggagcccaaggagtcaacaacacagcttcagggaataacagccgagaagggactgggggcagcaacgggaaaagagagagatatactgagaaccggggcagcagccgtcacagtcacggagagactggcaatcggcatagcgatagtccacgtcacggagatggtggtcgccatggagatggataccgccatccagaaagcagcagccgtcatactgatggccatcggcacggggagaacagacatggaggaagcgcaggccggcatggggagaaccggggtgcaaatgatggtcggaatggggaaagcaggaaagaagcttttaatcgtgagagcaagatggagcccaagatggaacccaaagtggacagcagcaagatggacaaggtggacagcaagacagataagacagctgacggctttgctgtcccagagccgcctaaacgcaagaaaagtcgatgggacagttag

SEQ ID NO: 80 - DNA, 3274 bp, synthetic construct
  source 1..3274: mol_type = other DNA
ggcctaactggccggtacctgagtctaaatgagtcttcggacctcgcgggggccgcttaagcggtggttagggtttgtctgacgcggggggagggggaaggaacgaaacactctcattcggaggcggctcggggtttggtcttggtggccacgggcacgcagaagagcgccgcgatcctcttaagcacccccccgccctccgtggaggcgggggtttggtcggcgggtggtaactggcgggccgctgactcgggcgggtcgcgcgccccagagtgtgaccttttcggtctgctcgcagacccccgggcggcgccgccgcggcggcgacgggctcgctgggtcctaggctccatggggaccgtatacgtggacaggctctggagcatccgcacgactgcggtgatattaccggagaccttctgcgggacgagccgggtcacgcggctgacgcggagcgtccgttgggcgacaaacaccaggacggggcacaggtacactatcttgtcacccggaggcgcgagggactgcaggagcttcagggagtggcgcagctgcttcatccccgtggcccgttgctcgcgtttgctggcggtgtccccggaagaaatatatttgcatgtctttagttctatgatgacacaaaccccgcccagcgtcttgtcattggcgaagtcgaacacgcagatgcagtcggggcggcgcggtcccaggtccacttcgcatattaaggtgacgcgtgtggcctcgaacaccgagcgaccctgcagcgacccgcttaaaagcttggcaatccggtactgttggtaaagccaccatggtcttcacactcgaagatttcgttggggactgggaacagacagccgcctacaacctggaccaagtccttgaacagggaggtgtgtccagtttgctgcagaatctcgccgtgtccgtaactccgatccaaaggattgtccggagcggtgaaaatgccctgaagatcgacatccatgtcatcatcccgtatgaaggtctgagcgccgaccaaatggcccagatcgaagaggtgtttaaggtggtgtaccctgtggatgatcatcactttaaggtgatcctgccctatggcacactggtaatcgacggggttacgccgaacatgctgaactatttcggacggccgtatgaaggcatcgccgtgttcgacggcaaaaagatcactgtaacagggaccctgtggaacggcaacaaaattatcgacgagcgcctgatcacccccgacggctccatgctgttccgagtaaccatcaacagtgggagttccggtggtggcgggagcggaggtggaggcatgtcccaccacggaggagctcccaaggcctctacgtgggtcgttgctagtcggcgaagctcgacagtgtcccgagcgccagagaggaggccggcggaggagttgaatcgaacaggtcctgagggatatagtgtcggcagaggtggtcgctggagaggcacctctaggcccccggaggccgtggccgctggtcacgaggaactgccgctgtgttttgctttgaagagccactttgttggcgcggtaatcggtcgtggtgggtcaaaaataaagaatatacaaagtacaacaaacaccacaatccaaataatacaagaacaaccagaatcattagtcaaaatttttggcagcaaggcaatgcaaacgaaagcaaaagcagtgatagacaattttgttaaaaagctagaagaaaattacaattcagaatgcggaattgatactgcattccaaccttctgttggaaaagatggaagcacagataacaatgttgttgcaggagatcggccattgatagattgggatcaaattagagaggaaggtttgaaatggcaaaaaacaaagtgggcagatttaccaccaattaagaaaaacttttataaagagtccactgccacaagtgccatgtcaaaagtagaagcagatagttggaggaaagaaaattttaatataacgtgggatgacttgaaggatggggagaaacgacctatccccaatcctacctgcacatttgatgacgcctttcaatgttatcctgaggttatggaaaacattaaaaaggcaggttttcaaaagccaacacctattcagtcacaggcatggcccattgtgttgcaaggaatagatcttataggagtagcccagactggaacaggaaagacattgtgttatttaatgcctggatttattcatctggtccttcaacccagccttaaaggtcaaaggaatagacccggcatgttagttctaactcccactcgggaattagcacttcaagtagaaggagaatgttgcaaatattcatataaagggcttcggagtgtttgtgtatatggtggtggaaatagagatgaacaaatagaagagcttaaaaaaggtgtagatatcataattgcaactcccggaagattgaatgatctgcaaatgagtaacttcgtcaatctgaagaatataacctacttggttttagatgaagcagacaagatgttggacatgggatttgaaccccagataatgaagattttgttagatgtgcgcccagataggcagacagttatgaccagtgctacatggcctcattcagttcatcgcctcgcacaatcttatttgaaagaaccaatgattgtctatgttggtacattggatctagttgctgtaagttcagtgaagcaaaatataattgtaaccaccgaggaagagaaatggagtcacatgcaaacttttctacagagtatgtcatccacagacaaagtcattgtcttcgtttctcgaaaagctgttgcggatcacttatcaagtgacctaatacttggaaatatatcagtagagtctctgcatggagatagagaacagagagatcgggagaaagcattagagaactttaaaacaggcaaagtgagaatactaattgcaactgatctagcctctagaggacttgatgtccatgacgttacacatgtctataattttgactttccacggaatattgaagaatacgtacaccgaatagggcgcacgggaagagcagggaggactggtgtttccattacaactttgactagaaatgattggagggttgcctctgaattgattaatattctggaaagagcaaatcagagtattccagaggagcttgtatcaatggctgagaggtttaaggcacatcaacagaaaagggaaatggaaagaaaaatggaaagacctcaaggaaggcccaagaagtttcattaa

SEQ ID NO: 81 - DNA, 4426 bp, synthetic construct
  source 1..4426: mol_type = other DNA
ggcctaactggccggtacctgagtctaaatgagtcttcggacctcgcgggggccgcttaagcggtggttagggtttgtctgacgcggggggagggggaaggaacgaaacactctcattcggaggcggctcggggtttggtcttggtggccacgggcacgcagaagagcgccgcgatcctcttaagcacccccccgccctccgtggaggcgggggtttggtcggcgggtggtaactggcgggccgctgactcgggcgggtcgcgcgccccagagtgtgaccttttcggtctgctcgcagacccccgggcggcgccgccgcggcggcgacgggctcgctgggtcctaggctccatggggaccgtatacgtggacaggctctggagcatccgcacgactgcggtgatattaccggagaccttctgcgggacgagccgggtcacgcggctgacgcggagcgtccgttgggcgacaaacaccaggacggggcacaggtacactatcttgtcacccggaggcgcgagggactgcaggagcttcagggagtggcgcagctgcttcatccccgtggcccgttgctcgcgtttgctggcggtgtccccggaagaaatatatttgcatgtctttagttctatgatgacacaaaccccgcccagcgtcttgtcattggcgaagtcgaacacgcagatgcagtcggggcggcgcggtcccaggtccacttcgcatattaaggtgacgcgtgtggcctcgaacaccgagcgaccctgcagcgacccgcttaaaagcttggcaatccggtactgttggtaaagccaccatggtcttcacactcgaagatttcgttggggactgggaacagacagccgcctacaacctggaccaagtccttgaacagggaggtgtgtccagtttgctgcagaatctcgccgtgtccgtaactccgatccaaaggattgtccggagcggtgaaaatgccctgaagatcgacatccatgtcatcatcccgtatgaaggtctgagcgccgaccaaatggcccagatcgaagaggtgtttaaggtggtgtaccctgtggatgatcatcactttaaggtgatcctgccctatggcacactggtaatcgacggggttacgccgaacatgctgaactatttcggacggccgtatgaaggcatcgccgtgttcgacggcaaaaagatcactgtaacagggaccctgtggaacggcaacaaaattatcgacgagcgcctgatcacccccgacggctccatgctgttccgagtaaccatcaacagtgggagttccggtggtggcgggagcggaggtggaggcatgggtcgggagtcacgccactatcgaaaacgatcggcatcccggggtcgctctggaagtcggtctagaagtcgctcaccctcagacaaaagaagtaaacgtggagatgacagacggtctagaagtagagatagagataggaggagagagaggtctcgtagcagggataaaagaagatctcggtcaagggacaggaagcgtctgagacgttccagaagtagagagagagacagaagccgagagcgaagaagatctcgaagtagagacaggagacgctcaaggagtagaagccggggccggcgatcccgatcctccagtcctggaaataaaagcaagaaaactgagaatagatctaggtccaaagagaaaactgatggtggggaaagttctaaagagaagaaaaaagacaaagatgacaaggaggatgaaaaagaaaaagatgctggcaactttgaccagaataagctggaagaagaaatgagaaagcgaaaagaaagagtagaaaaatggcgagaagagcaacgtaaaaaggctatggaaaacataggagaactgaaaaaggaaatcgaagagatgaaacaagggaaaaagtggagtttagaggacgatgatgatgacgaagatgatcctgcagaagctgaaaaggagggaaatgaaatggagggtgaggagttagatccattagatgcttacatggaagaagtgaaagaggaagtaaaaaaatttaacatgagaagtgtaaaaggtggtgggggaaatgaaaagaagtctgggccaacggtcacaaaagttgtcactgttgtgacaaccaaaaaagcagttgtggattctgataagaagaaaggtgagctgatggagaatgaccaggatgccatggagtattcttcagaggaggaagaagttgatcttcagacagcccttacagggtatcaaacaaaacagcgaaagcttctagaaccagttgatcatggaaaaattgagtatgagccatttaggaaaaacttctatgttgaagttccagaactagcaaaaatgtctcaagaagaggtaaatgtgtttcgattggaaatggagggcattacagttaaaggaaaaggttgccccaaaccaattaaatcctgggtccagtgtggaatttccatgaagatcttaaattccctcaagaagcatggctatgaaaagcccacgcccatccaaacccaagctattcctgctataatgtctggacgagatttgattggcattgccaaaacaggaagtggaaagaccattgcttttctgttgcccatgtttagacacatcatggatcagaggtcattagaggaaggagaggggccaatagctgtcatcatgactccaactcgagaactggctttacagattactaaagagtgtaagaagttttccaagactttgggacttagagtggtctgtgtttacggaggaacaggaatcagtgagcagattgctgagctgaaaagaggtgctgaaattattgtttgcacacctggtcgaatgattgacatgttagccgctaacagtggtcgggtcacaaatcttcgaagagtgacatatgttgttttagatgaagcagacagaatgtttgacatgggttttgaaccccaggtcatgcgcatcgtggataatgttcgtcctgatcgacagacggttatgttttcagctactttccccagagctatggaggctttggctcgcaggatcctcagtaaacctattgaagtacaagttggaggcaggagtgtggtttgctcagatgtggagcaacaagtgattgtgattgaagaagaaaagaaattcttgaagttacttgagcttctaggccattatcaagagtcaggatctgtcattatatttgtggataagcaggaacatgctgatggtcttcttaaggatttaatgagagcatcttatccttgcatgtctcttcatggaggcattgatcaatatgacagagatagcatcataaatgactttaagaatgggacctgcaaacttcttgtggctacctctgttgctgcccgaggtctagatgtgaaacatctgattcttgtagtaaattatagctgccccaaccattatgaggattatgtacacagagcagggcggactggaagagcaggaaacaagggttatgcttatacttttatcacagaggatcaagctcgctatgctggtgacataattaaagctcttgaattgtcagggactgcagtacctcctgatttagagaaactgtggagtgatttcaaagatcagcagaaagctgaggggaaaataattaaaaagagtagtgggttctctggtaagggattcaagtttgatgaaacagaacaagctttggctaatgagaggaagaagttacaaaaagcagctcttggtctacaagattcagatgatgaggatgctgcagttgatattgatgagcaaattgaaagcatgtttaattcaaagaagagagtaaaggatatggctgctcctggaacatcaagtgttcctgctccaactgcaggaaatgctgagaaattagaaattgctaagagattggctcttagaatcaatgcccagaagaatttgggcatcgagtctcaggtagatgtgatgcagcaggccaccaatgcaattcttaggggtggcaccattctggctcccactgtttctgcaaaaaccattgcagaacaacttgctgaaaagatcaatgccaagctcaattatgtgccgttagagaaacaagaagaagagagacaggatggtggacagaatgaatcttttaagagatatgaagaagaattagagatcaatgacttcccacagactgctaggtggaaagttacctctaaggaagctctgcagagaatcagtgaatactctgaagccgcaattacaatcagaggaacctacttccctcctggcaaagaacccaaggaaggcgagcggaagatttacttggcaattgaaagtgccaatgaactggctgtgcagaaagcaaaggcagaaatcaccaggctcataaaagaagagctgatccggctgcaaaattcataccaaccaacaaataaaggaagatacaaagtcttatag

SEQ ID NO: 82 - DNA, 2695 bp, synthetic construct
  source 1..2695: mol_type = other DNA
ggcctaactggccggtacctgagtctaaatgagtcttcggacctcgcgggggccgcttaagcggtggttagggtttgtctgacgcggggggagggggaaggaacgaaacactctcattcggaggcggctcggggtttggtcttggtggccacgggcacgcagaagagcgccgcgatcctcttaagcacccccccgccctccgtggaggcgggggtttggtcggcgggtggtaactggcgggccgctgactcgggcgggtcgcgcgccccagagtgtgaccttttcggtctgctcgcagacccccgggcggcgccgccgcggcggcgacgggctcgctgggtcctaggctccatggggaccgtatacgtggacaggctctggagcatccgcacgactgcggtgatattaccggagaccttctgcgggacgagccgggtcacgcggctgacgcggagcgtccgttgggcgacaaacaccaggacggggcacaggtacactatcttgtcacccggaggcgcgagggactgcaggagcttcagggagtggcgcagctgcttcatccccgtggcccgttgctcgcgtttgctggcggtgtccccggaagaaatatatttgcatgtctttagttctatgatgacacaaaccccgcccagcgtcttgtcattggcgaagtcgaacacgcagatgcagtcggggcggcgcggtcccaggtccacttcgcatattaaggtgacgcgtgtggcctcgaacaccgagcgaccctgcagcgacccgcttaaaagcttggcaatccggtactgttggtaaagccaccatggtcttcacactcgaagatttcgttggggactgggaacagacagccgcctacaacctggaccaagtccttgaacagggaggtgtgtccagtttgctgcagaatctcgccgtgtccgtaactccgatccaaaggattgtccggagcggtgaaaatgccctgaagatcgacatccatgtcatcatcccgtatgaaggtctgagcgccgaccaaatggcccagatcgaagaggtgtttaaggtggtgtaccctgtggatgatcatcactttaaggtgatcctgccctatggcacactggtaatcgacggggttacgccgaacatgctgaactatttcggacggccgtatgaaggcatcgccgtgttcgacggcaaaaagatcactgtaacagggaccctgtggaacggcaacaaaattatcgacgagcgcctgatcacccccgacggctccatgctgttccgagtaaccatcaacagtgggagttccggtggtggcgggagcggaggtggaggcatggcggcacccgaggaacacgattctccgaccgaagcgtcccagccgattgtggaagaggaggaaactaaaacatttaaagacctgggtgtgacagatgtgttgtgtgaagcttgtgaccagttgggatggacaaaacccaccaagatccagattgaagctattcctttggccttacaaggtcgtgatatcattgggcttgcagaaactggctctggaaagacaggcgcctttgctttgcccattctaaacgcactgctggagaccccgcagcgtttgtttgccctagttcttaccccgactcgggagctggcctttcagatctcagagcagtttgaagccctggggtcctctattggagtgcagagtgctgtgattgtaggtggaattgattcaatgtctcaatctttggcccttgcaaaaaaaccacatataataatagcaactcctggtcgactgattgaccacttggaaaatacgaaaggtttcaacttgagagctctcaaatacttggtcatggatgaagccgaccgaatactgaatatggattttgagacagaggttgacaagatcctcaaagtgattcctcgagatcggaaaacattcctcttctctgccaccatgaccaagaaggttcaaaaacttcagcgagcagctctgaagaatcctgtgaaatgtgccgtttcctctaaataccagacagttgaaaaattacagcaatattatatttttattccctctaaattcaaggatacctacctggtttatattctaaatgaattggctggaaactcctttatgatattctgcagcacctgtaataatacccagagaacagctttgctactgcgaaatcttggcttcactgccatccccctccatggacaaatgagtcagagtaagcgcctaggatcccttaataagtttaaggccaaggcccgttccattcttctagcaactgacgttgccagccgaggtttggacatacctcatgtagatgtggttgtcaactttgacattcctacccattccaaggattacatccatcgagtaggtcgaacagctagagctgggcgctccggaaaggctattacttttgtcacacagtatgatgtggaactcttccagcgcatagaacacttaattgggaagaaactaccaggttttccaacacaggatgatgaggttatgatgctgacagaacgcgtcgctgaagcccaaaggtttgcccgaatggagttaagggagcatggagaaaagaagaaacgctcgcgagaggatgctggagataatgatgacacagagggtgctattggtgtcaggaacaaggtggctggaggaaaaatgaagaagcggaaaggccgttaa

SEQ ID NO: 83 - DNA, 2563 bp, synthetic construct
  source 1..2563: mol_type = other DNA
ggcctaactggccggtacctgagtctaaatgagtcttcggacctcgcgggggccgcttaagcggtggttagggtttgtctgacgcggggggagggggaaggaacgaaacactctcattcggaggcggctcggggtttggtcttggtggccacgggcacgcagaagagcgccgcgatcctcttaagcacccccccgccctccgtggaggcgggggtttggtcggcgggtggtaactggcgggccgctgactcgggcgggtcgcgcgccccagagtgtgaccttttcggtctgctcgcagacccccgggcggcgccgccgcggcggcgacgggctcgctgggtcctaggctccatggggaccgtatacgtggacaggctctggagcatccgcacgactgcggtgatattaccggagaccttctgcgggacgagccgggtcacgcggctgacgcggagcgtccgttgggcgacaaacaccaggacggggcacaggtacactatcttgtcacccggaggcgcgagggactgcaggagcttcagggagtggcgcagctgcttcatccccgtggcccgttgctcgcgtttgctggcggtgtccccggaagaaatatatttgcatgtctttagttctatgatgacacaaaccccgcccagcgtcttgtcattggcgaagtcgaacacgcagatgcagtcggggcggcgcggtcccaggtccacttcgcatattaaggtgacgcgtgtggcctcgaacaccgagcgaccctgcagcgacccgcttaaaagcttggcaatccggtactgttggtaaagccaccatggtcttcacactcgaagatttcgttggggactgggaacagacagccgcctacaacctggaccaagtccttgaacagggaggtgtgtccagtttgctgcagaatctcgccgtgtccgtaactccgatccaaaggattgtccggagcggtgaaaatgccctgaagatcgacatccatgtcatcatcccgtatgaaggtctgagcgccgaccaaatggcccagatcgaagaggtgtttaaggtggtgtaccctgtggatgatcatcactttaaggtgatcctgccctatggcacactggtaatcgacggggttacgccgaacatgctgaactatttcggacggccgtatgaaggcatcgccgtgttcgacggcaaaaagatcactgtaacagggaccctgtggaacggcaacaaaattatcgacgagcgcctgatcacccccgacggctccatgctgttccgagtaaccatcaacagtgggagttccggtggtggcgggagcggaggtggaggcatggcgaccacggccacgatggcgacctcgggctcggcgcgaaagcggctgctcaaagaggaagacatgactaaagtggaattcgagaccagcgaggaggtggatgtgacccccacgttcgacaccatgggcctgcgggaggacctgctgcggggcatctacgcttacggttttgaaaaaccatcagcaatccagcaacgagcaatcaagcagatcatcaaagggagagatgtcatcgcacagtctcagtccggcacaggaaaaacagccaccttcagtatctcagtcctccagtgtttggatattcaggttcgtgaaactcaagctttgatcttggctcccacaagagagttggctgtgcagatccagaaggggctgcttgctctcggtgactacatgaatgtccagtgccatgcctgcattggaggcaccaatgttggcgaggacatcaggaagctggattacggacagcatgttgtcgcgggcactccagggcgtgtttttgatatgattcgtcgcagaagcctaaggacacgtgctatcaaaatgttggttttggatgaagctgatgaaatgttgaataaaggtttcaaagagcagatttacgatgtatacaggtacctgcctccagccacacaggtggttctcatcagtgccacgctgccacacgagattctggagatgaccaacaagttcatgaccgacccaatccgcatcttggtgaaacgtgatgaattgactctggaaggcatcaagcaatttttcgtggcagtggagagggaagagtggaaatttgacactctgtgtgacctctacgacacactgaccatcactcaggcggtcatcttctgcaacaccaaaagaaaggtggactggctgacggagaaaatgagggaagccaacttcactgtatcctcaatgcatggagacatgccccagaaagagcgggagtccatcatgaaggagttccggtcgggcgccagccgagtgcttatttctacagatgtctgggccagggggttggatgtccctcaggtgtccctcatcattaactatgatctccctaataacagagaattgtacatacacagaattgggagatcaggtcgatacggccggaagggtgtggccattaactttgtaaagaatgacgacatccgcatcctcagagatatcgagcagtactattccactcagattgatgagatgccgatgaacgttgctgatcttatctga

SEQ ID NO: 84 - DNA, 2779 bp, synthetic construct
  source 1..2779: mol_type = other DNA
ggcctaactggccggtacctgagtctaaatgagtcttcggacctcgcgggggccgcttaagcggtggttagggtttgtctgacgcggggggagggggaaggaacgaaacactctcattcggaggcggctcggggtttggtcttggtggccacgggcacgcagaagagcgccgcgatcctcttaagcacccccccgccctccgtggaggcgggggtttggtcggcgggtggtaactggcgggccgctgactcgggcgggtcgcgcgccccagagtgtgaccttttcggtctgctcgcagacccccgggcggcgccgccgcggcggcgacgggctcgctgggtcctaggctccatggggaccgtatacgtggacaggctctggagcatccgcacgactgcggtgatattaccggagaccttctgcgggacgagccgggtcacgcggctgacgcggagcgtccgttgggcgacaaacaccaggacggggcacaggtacactatcttgtcacccggaggcgcgagggactgcaggagcttcagggagtggcgcagctgcttcatccccgtggcccgttgctcgcgtttgctggcggtgtccccggaagaaatatatttgcatgtctttagttctatgatgacacaaaccccgcccagcgtcttgtcattggcgaagtcgaacacgcagatgcagtcggggcggcgcggtcccaggtccacttcgcatattaaggtgacgcgtgtggcctcgaacaccgagcgaccctgcagcgacccgcttaaaagcttggcaatccggtactgttggtaaagccaccatggtcttcacactcgaagatttcgttggggactgggaacagacagccgcctacaacctggaccaagtccttgaacagggaggtgtgtccagtttgctgcagaatctcgccgtgtccgtaactccgatccaaaggattgtccggagcggtgaaaatgccctgaagatcgacatccatgtcatcatcccgtatgaaggtctgagcgccgaccaaatggcccagatcgaagaggtgtttaaggtggtgtaccctgtggatgatcatcactttaaggtgatcctgccctatggcacactggtaatcgacggggttacgccgaacatgctgaactatttcggacggccgtatgaaggcatcgccgtgttcgacggcaaaaagatcactgtaacagggaccctgtggaacggcaacaaaattatcgacgagcgcctgatcacccccgacggctccatgctgttccgagtaaccatcaacagtgggagttccggtggtggcgggagcggaggtggaggcatggcaggcttcgcggagctcgggctgtcatcgtggctcgtggaacaatgtcggcagctgggtttgaagcagcccacgcccgtgcagctcggctgcatccccgccatcctggagggtcgagactgcttgggctgtgctaagacaggcagtgggaagacagcagcgtttgtccttcccatcttgcagaagctgtctgaggatccctatggcatcttctgcctcgtcctgacacccaccagggagctggcctaccagatcgcagagcagttccgggtcctggggaagcctctagggctgaaagactgcatcatcgtcggtggcatggacatggtggcccaggcgctggagctctctcggaaaccacacgtggtcatcgccacgccggggcgcctggcagatcacctgcgcagctccaacacttttagtataaagaagatccgcttcctggtgatggatgaggcagaccggctgctggaacagggctgcactgacttcaccgtggacctggaggccatcctggcggctgtgccggcccgcaggcagacactgctgttcagcgccacgctgaccgacacactccgggagctgcagggtctggccaccaaccagcccttcttctgggaagcacaggccccggtgagcaccgtggagcagctggaccagcgctacctgctggtgcctgagaaggtcaaggacgcctacctggtccacctgatccagcgcttccaggatgagcacgaggactggtccattatcatcttcaccaacacgtgcaagacctgccagattctgtgcatgatgctgcgcaaattcagcttccccaccgtggctctgcactccatgatgaagcagaaagaacgctttgccgccctagccaagttcaagtccagcatctaccggatcctgatcgcaacagacgtggcctcccggggcctggacatccctacggtacaggtggtcatcaaccacaacacccccgggctccccaagatctacatccaccgagtcggccggacggcccgtgcagggcggcagggtcaggccatcacgctggtgacacagtacgacatccacctggtgcacgccatcgaggagcagatcaagaagaagctggaggagttctccgtggaagaggccgaggtgctacagatcctcacacaggtcaacgtggtgcgaagagagtgtgagatcaaactggaggcggcccactttgacgaaaagaaggagatcaacaaacggaagcagctgatcctggaggggaaggaccctgacctggaggccaagcgcaaggctgagctggccaagatcaagcagaagaaccggcgcttcaaggagaaggtggaggagacgctgaagcgacagaaggctggcagggctggccacaaggggcgtccacccaggacaccgtctgggtcccactcaggcccagtcccctcccagggcctggtctga

SEQ ID NO: 85 - DNA, 3541 bp, synthetic construct
  source 1..3541: mol_type = other DNA
ggcctaactggccggtacctgagtctaaatgagtcttcggacctcgcgggggccgcttaagcggtggttagggtttgtctgacgcggggggagggggaaggaacgaaacactctcattcggaggcggctcggggtttggtcttggtggccacgggcacgcagaagagcgccgcgatcctcttaagcacccccccgccctccgtggaggcgggggtttggtcggcgggtggtaactggcgggccgctgactcgggcgggtcgcgcgccccagagtgtgaccttttcggtctgctcgcagacccccgggcggcgccgccgcggcggcgacgggctcgctgggtcctaggctccatggggaccgtatacgtggacaggctctggagcatccgcacgactgcggtgatattaccggagaccttctgcgggacgagccgggtcacgcggctgacgcggagcgtccgttgggcgacaaacaccaggacggggcacaggtacactatcttgtcacccggaggcgcgagggactgcaggagcttcagggagtggcgcagctgcttcatccccgtggcccgttgctcgcgtttgctggcggtgtccccggaagaaatatatttgcatgtctttagttctatgatgacacaaaccccgcccagcgtcttgtcattggcgaagtcgaacacgcagatgcagtcggggcggcgcggtcccaggtccacttcgcatattaaggtgacgcgtgtggcctcgaacaccgagcgaccctgcagcgacccgcttaaaagcttggcaatccggtactgttggtaaagccaccatggtcttcacactcgaagatttcgttggggactgggaacagacagccgcctacaacctggaccaagtccttgaacagggaggtgtgtccagtttgctgcagaatctcgccgtgtccgtaactccgatccaaaggattgtccggagcggtgaaaatgccctgaagatcgacatccatgtcatcatcccgtatgaaggtctgagcgccgaccaaatggcccagatcgaagaggtgtttaaggtggtgtaccctgtggatgatcatcactttaaggtgatcctgccctatggcacactggtaatcgacggggttacgccgaacatgctgaactatttcggacggccgtatgaaggcatcgccgtgttcgacggcaaaaagatcactgtaacagggaccctgtggaacggcaacaaaattatcgacgagcgcctgatcacccccgacggctccatgctgttccgagtaaccatcaacagtgggagttccggtggtggcgggagcggaggtggaggcatgcctgggaaactcctctggggggacattatggagctggaagcacccttggaggagtccgagagccagaagaaggagaggcaaaagagtgacagaaggaagtcaaggcaccattatgactcggatgagaaatcagaaacaagagaaaatggtgttacagatgacctggatgctcccaaggccaaaaaatctaaaatgaaagagaagctaaatggagacactgaagaaggatttaatagactttcagatgaattctccaaatctcataagtcaagaagaaaagatctaccaaatggagatatagatgaatatgaaaaaaaatcaaagcgagtatcatctttagatacttctactcataaatcaagtgataataaactagaggagaccttaacacgtgaacagaaagaaggagccttctccaattttcctatttctgaagagactataaagcttctgaaaggtcgaggggtaacatatctctttcctattcaagttaagacctttggtcctgtatatgaaggaaaagatttaatagctcaagcacggacaggaacaggaaagacattctcttttgccatccccttaattgaaagactccaaagaaatcaagaaacaattaaaaaaagccgctcaccaaaggtacttgttttggctccaacaagggaactggcaaaccaagtagccaaagacttcaaagatataactaggaaactcagcgtggcgtgtttttatggtggaacatcatatcaaagccaaattaatcatattcgaaatggtattgacatcttggttggaacacctggtcgtatcaaagaccatctgcagagtggccgattggatctttctaaactgcgacatgttgtgcttgatgaagtggatcagatgttagatttaggtttcgctgaacaagttgaagatattattcatgaatcctacaaaactgattctgaagacaatcctcagactttacttttttctgcaacttgcccacagtgggtatacaaagttgcaaaaaaatacatgaaatccagatatgaacaggttgaccttgttggaaaaatgactcaaaaggctgcaactactgtggaacatttggccatccagtgtcattggtctcagaggccagcagttattggagatgtccttcaagtctacagtgggtctgaagggagggctattattttctgtgagaccaagaagaatgtaactgaaatggccatgaatccacacataaaacagaatgcccagtgtttacatggggacattgcacagtcacaaagagaaattacactaaaaggcttcagagaaggtagttttaaagttttggtggcaaccaatgtggctgcccgtggtttggacattcctgaagttgacctggtgattcaaagttctcctcctcaggatgttgagtcctatatccatcgctctggacgcacaggtagagctggacggacagggatttgtatatgtttttatcaaccaagagaaagaggtcaactaagatatgtggaacaaaaagcaggaattacttttaaacgtgtaggtgttccttctacaatggatttagttaaatctaaaagcatggatgccatcaggtctctggcttccgtttcttacgctgctgttgattttttccgaccatcagctcagagactgatagaagagaaaggtgcagtggatgcattggctgcagctttagcccacatttctggtgcatcaagctttgaaccacgatctttgatcacctctgataaggggtttgtgaccatgactctggaaagcctagaggaaatacaggatgtcagctgtgcttggaaagaacttaacagaaagctgagtagtaatgcagtgtctcagattaccagaatgtgcctcctgaaaggaaatatgggtgtttgctttgatgttcctacaactgagtcagaaaggttacaggcagagtggcatgattccgactggatactctcagtgccagccaaattacctgaaattgaagaatattatgatggaaacacatcttctaattccagacagaggagtggctggtcaagtggtcgatcaggccggtcaggccggtcaggtggtcgatctggcggccggtcaggtagacagagtcgacaaggaagtcgctcaggaagtcgacaagatggtagaagacgaagtgggaatagaaatcgatcaagaagtgggggccacaaacggagttttgactga

SEQ ID NO: 86 - DNA, 3328 bp, synthetic construct
  source 1..3328: mol_type = other DNA
ggcctaactggccggtacctgagtctaaatgagtcttcggacctcgcgggggccgcttaagcggtggttagggtttgtctgacgcggggggagggggaaggaacgaaacactctcattcggaggcggctcggggtttggtcttggtggccacgggcacgcagaagagcgccgcgatcctcttaagcacccccccgccctccgtggaggcgggggtttggtcggcgggtggtaactggcgggccgctgactcgggcgggtcgcgcgccccagagtgtgaccttttcggtctgctcgcagacccccgggcggcgccgccgcggcggcgacgggctcgctgggtcctaggctccatggggaccgtatacgtggacaggctctggagcatccgcacgactgcggtgatattaccggagaccttctgcgggacgagccgggtcacgcggctgacgcggagcgtccgttgggcgacaaacaccaggacggggcacaggtacactatcttgtcacccggaggcgcgagggactgcaggagcttcagggagtggcgcagctgcttcatccccgtggcccgttgctcgcgtttgctggcggtgtccccggaagaaatatatttgcatgtctttagttctatgatgacacaaaccccgcccagcgtcttgtcattggcgaagtcgaacacgcagatgcagtcggggcggcgcggtcccaggtccacttcgcatattaaggtgacgcgtgtggcctcgaacaccgagcgaccctgcagcgacccgcttaaaagcttggcaatccggtactgttggtaaagccaccatggtcttcacactcgaagatttcgttggggactgggaacagacagccgcctacaacctggaccaagtccttgaacagggaggtgtgtccagtttgctgcagaatctcgccgtgtccgtaactccgatccaaaggattgtccggagcggtgaaaatgccctgaagatcgacatccatgtcatcatcccgtatgaaggtctgagcgccgaccaaatggcccagatcgaagaggtgtttaaggtggtgtaccctgtggatgatcatcactttaaggtgatcctgccctatggcacactggtaatcgacggggttacgccgaacatgctgaactatttcggacggccgtatgaaggcatcgccgtgttcgacggcaaaaagatcactgtaacagggaccctgtggaacggcaacaaaattatcgacgagcgcctgatcacccccgacggctccatgctgttccgagtaaccatcaacagtgggagttccggtggtggcgggagcggaggtggaggcatggcgctgttctacgtcgcgcggtacccgggccccgatgcggcagctgcggcggggccggagggcgcggaggccggggcgcacggcagggcccgcgcgctgctcgagcggctgcagagccgggcccgcgaacggcagcagcagcgggagcccgcgcagaccgaggcggctgcatcgaccgagccggcgaccaggaggcgacggcggccccggcggcggcggcgggtgaacgacgcggagccggggagcccggaggcgccgcagggaaagcgacggaaggcggacggcgaggacgcgggcgcagaaagcaacgaggaggcgccaggggagcccagcgcagggagcagcgaggaggcgccaggggagcccagcgcagggagcagcgaggaggcgccgggggagcgcagcaccagcgccagcgccgaggcggccccagatggaccggccctggaggaggcggccggacccctggtccccggcctggtgctgggggggttcgggaagaggaaggcgccgaaggtccagcctttcctgccaaggtggctggctgagcctaactgtgtcagaaggaatgtcaccgaagacctggttcctatcgaggacatccctgacgtccatcctgacctgcagaagcagctgcgggcacacggcatctcgtcctactttccagtccaggcagctgtgattcctgccctcctggagagcgcagcctgtgggtttctggtgggcagaggtggctaccggcctagcgacctctgtgtttctgccccaacaggcagtgggaagacactggccttcgtcatccctgtggtgcaggccctgctttcgagagtggtctgccacatccgtgccctggttgtgctgcccaccaaggagctggcccagcaggtgagcaaagttttcaacatctacacagatgccacacctctgagagtctccctggttacgggacagaagtctctggccaaggagcaggagagcctcgtccagaaaacagctgatgggtaccgctgcttggctgacatcgtggtagccacccccggccgcctggtggaccacatcgaccagaccccaggattcagcctccagcagctccgcttcctgattatcgacgaggctgaccggatgattgacagcatgcatcagtcctggctgccgcgggtggtggcggccgccttccagagcgaggaccccgcggacccctgtgccctgctccagcgaaggcaggcccaggctgtgacagccgccagcacctgctgtccccagatgcccctgcagaagctgctcttctcagctactctgacccagaaccctgaaaagctgcagcagctgggcctccaccagccccggcttttctccacagggctagcacacaggggcctggaagatacagatggggacggggattcggggaagtatgcctttcctgttgggctcacgcaccactacgtgccctgcagcctcagctctaagccgctggtcgtcctgcacctggtcctggagatgggcttctcgagggttctctgcttcactaactcccgagagaactcccacaggctcttcctgctggtgcaagcttttgggggtgtggacgtggctgagttctcctcgcgctacgggcctggccagaggaggatgatcctgaagcagtttgaacaggggaagatccagctgctcatcagcacggacgccaccgcgcgaggcatcgacgtgcagggtgtggagctggtggtgaactacgacgccccccagtacctgagaacctacgtgcaccgggttgggaggacagctcgcgctgggaaaactggacaggccttcacactgctcctgaaagtgcaggagaggagattcctccgaatgctaactgaagctggggcacctgagttgcagcggcacgagctctccagcaagctgctgcagccgctggttcctcggtacgaggaggccctgtcccagctggaggagtctgtcaaggaagagcgcaagcagagggcggcctag

SEQ ID NO: 87 - DNA, 3127 bp, synthetic construct
  source 1..3127: mol_type = other DNA
ggcctaactggccggtacctgagtctaaatgagtcttcggacctcgcgggggccgcttaagcggtggttagggtttgtctgacgcggggggagggggaaggaacgaaacactctcattcggaggcggctcggggtttggtcttggtggccacgggcacgcagaagagcgccgcgatcctcttaagcacccccccgccctccgtggaggcgggggtttggtcggcgggtggtaactggcgggccgctgactcgggcgggtcgcgcgccccagagtgtgaccttttcggtctgctcgcagacccccgggcggcgccgccgcggcggcgacgggctcgctgggtcctaggctccatggggaccgtatacgtggacaggctctggagcatccgcacgactgcggtgatattaccggagaccttctgcgggacgagccgggtcacgcggctgacgcggagcgtccgttgggcgacaaacaccaggacggggcacaggtacactatcttgtcacccggaggcgcgagggactgcaggagcttcagggagtggcgcagctgcttcatccccgtggcccgttgctcgcgtttgctggcggtgtccccggaagaaatatatttgcatgtctttagttctatgatgacacaaaccccgcccagcgtcttgtcattggcgaagtcgaacacgcagatgcagtcggggcggcgcggtcccaggtccacttcgcatattaaggtgacgcgtgtggcctcgaacaccgagcgaccctgcagcgacccgcttaaaagcttggcaatccggtactgttggtaaagccaccatggtcttcacactcgaagatttcgttggggactgggaacagacagccgcctacaacctggaccaagtccttgaacagggaggtgtgtccagtttgctgcagaatctcgccgtgtccgtaactccgatccaaaggattgtccggagcggtgaaaatgccctgaagatcgacatccatgtcatcatcccgtatgaaggtctgagcgccgaccaaatggcccagatcgaagaggtgtttaaggtggtgtaccctgtggatgatcatcactttaaggtgatcctgccctatggcacactggtaatcgacggggttacgccgaacatgctgaactatttcggacggccgtatgaaggcatcgccgtgttcgacggcaaaaagatcactgtaacagggaccctgtggaacggcaacaaaattatcgacgagcgcctgatcacccccgacggctccatgctgttccgagtaaccatcaacagtgggagttccggtggtggcgggagcggaggtggaggcatggacgtccacgatctctttcgccggctcggcgcgggggccaaattcgacacgagacgcttctcggcagacgcagctcgattccagataggaaaaaggaaatatgactttgattcttcggaggtgcttcagggactggacttttttggaaacaagaagtctgtcccaggtgtgtgtggagcatcacaaacacatcagaagccccaaaatggagagaaaaaagaagagagcctaactgaaaggaagagggagcagagcaagaaaaaaaggaagacgatgacttcagaaattgcttcccaagaagaaggtgctactatacagtggatgtcatctgtagaagcaaagattgaagacaaaaaagttcagagagaaagtaaactaacttccggaaagttggagaatctcagaaaagaaaagataaacttcttgcggaataaacacaaaattcacgtccaaggaaccgatcttcctgacccaattgctacatttcagcaacttgaccaggaatataaaatcaattctcgactacttcagaacattctagatgcaggtttccaaatgcctacgccaatccaaatgcaagccatcccagttatgctgcatggtcgggaacttctggcttctgctccaactggatctggaaaaacattagcttttagcattcctattttaatgcagctgaaacaacccgcaaataaaggcttcagagccctgattatatcaccaacacgagaacttgccagccagattcacagagagttaataaaaatttctgagggaacaggattcaggatacacatgatccacaaagcagcagtggcagccaagaaatttggacctaaatcatctaaaaagtttgatattcttgtgactactccaaatcgactaatctatttattaaagcaagatccccccggaatcgacctagcaagtgttgagtggcttgtagtagacgaatcagataaactgtttgaagatggcaaaactgggttcagagaccagctggcttccattttcctggcctgcacatcccacaaggtccgaagagctatgttcagtgcaacttttgcatatgatgttgaacagtggtgcaaactcaacctggacaatgtcatcagtgtgtccattggagcaaggaattctgcagtagaaactgtagaacaagagcttctctttgttggatctgagaccggaaaacttctggccatgagagaacttgttaaaaagggtttcaatccacctgttcttgtttttgttcagtccattgaaagggctaaagaactttttcatgagctcatatatgaaggtattaatgtggatgttattcatgcagagagaacacaacaacagagagataacacagtccacagtttcagagcaggaaaaatctgggttctgatttgtacagccttgctagcaagagggattgattttaaaggtgtgaacttggtgatcaactatgactttccaactagctcagtggaatatatccacaggataggtcgaactggaagagcagggaataagggaaaagcaattacatttttcactgaggatgataagccattattaagaagcgttgctaatgttatacagcaggctgggtgtcctgtaccagaatacataaaaggttttcagaaactactaagcaaacaaaagaaaaagatgattaagaaaccattggaaagggagagcattagtacaactccaaaatgtttcttagaaaaagctaaggataaacagaaaaaggtcactggtcagaacagcaagaagaaagtagctcttgaagacaaaagttaa

SEQ ID NO: 88 - DNA, 3223 bp, synthetic construct
  source 1..3223: mol_type = other DNA
ggcctaactggccggtacctgagtctaaatgagtcttcggacctcgcgggggccgcttaagcggtggttagggtttgtctgacgcggggggagggggaaggaacgaaacactctcattcggaggcggctcggggtttggtcttggtggccacgggcacgcagaagagcgccgcgatcctcttaagcacccccccgccctccgtggaggcgggggtttggtcggcgggtggtaactggcgggccgctgactcgggcgggtcgcgcgccccagagtgtgaccttttcggtctgctcgcagacccccgggcggcgccgccgcggcggcgacgggctcgctgggtcctaggctccatggggaccgtatacgtggacaggctctggagcatccgcacgactgcggtgatattaccggagaccttctgcgggacgagccgggtcacgcggctgacgcggagcgtccgttgggcgacaaacaccaggacggggcacaggtacactatcttgtcacccggaggcgcgagggactgcaggagcttcagggagtggcgcagctgcttcatccccgtggcccgttgctcgcgtttgctggcggtgtccccggaagaaatatatttgcatgtctttagttctatgatgacacaaaccccgcccagcgtcttgtcattggcgaagtcgaacacgcagatgcagtcggggcggcgcggtcccaggtccacttcgcatattaaggtgacgcgtgtggcctcgaacaccgagcgaccctgcagcgacccgcttaaaagcttggcaatccggtactgttggtaaagccaccatggtcttcacactcgaagatttcgttggggactgggaacagacagccgcctacaacctggaccaagtccttgaacagggaggtgtgtccagtttgctgcagaatctcgccgtgtccgtaactccgatccaaaggattgtccggagcggtgaaaatgccctgaagatcgacatccatgtcatcatcccgtatgaaggtctgagcgccgaccaaatggcccagatcgaagaggtgtttaaggtggtgtaccctgtggatgatcatcactttaaggtgatcctgccctatggcacactggtaatcgacggggttacgccgaacatgctgaactatttcggacggccgtatgaaggcatcgccgtgttcgacggcaaaaagatcactgtaacagggaccctgtggaacggcaacaaaattatcgacgagcgcctgatcacccccgacggctccatgctgttccgagtaaccatcaacagtgggagttccggtggtggcgggagcggaggtggaggcatgtcccactgggccccagagtggaagagggcggaggctaatccaagagaccttggggccagctgggatgtcaggggcagcagaggcagtggctggagtggccccttcggccatcagggaccgagagcagcaggctcccgtgaaccaccactctgctttaaaataaagaacaatatggttggtgtggtcattggttacagtggatcaaaaataaaagatctacaacattcgacaaacactaaaatacagatcataaacggggaatctgaagcaaaagtcagaatttttggcaatagggaaatgaaagcaaaggccaaagcggctatagaaacacttattagaaaacaagaaagctacaactcagaatccagtgtggataatgctgcatcccaaacccctattggaagaaatctaggcagaaatgacattgttggagaagctgagccattgtcaaattgggatcgcattagggcagcagtcgtggagtgcgaaaagagaaaatgggcagatctaccaccagttaagaaaaacttttacatagaatccaaagcaacaagctgcatgtctgaaatgcaggtgattaactggagaaaggaaaatttcaacataacgtgtgatgacttgaaaagtggtgaaaagcgtctcattccaaaaccaacttgcaggtttaaagacgcttttcagcaataccctgatcttctgaaaagcataataagggtagggattgtaaagccaacgccaattcagtcacaggcatggccaattattctacaaggaatagatcttatagtagttgcacaaaccggaacagggaaaacattgtcctatctaatgcctgggtttattcatcttgattctcaaccaatatctagagagcaaaggaatgggcctgggatgctagtccttacacccactagagagttggctcttcacgtggaagctgaatgttcaaagtattcatataaaggtctcaaaagcatttgcatatatggtggtagaaacagaaatggacaaatagaagacattagcaaaggtgtagatatcattattgcaactcctgggaggctgaatgacctacaaatgaataactctgtcaacctaagaagcataacctacttggttatagatgaggcagataaaatgctggatatggaatttgaaccccagataaggaagattttattagatgtgcgcccagaccgacagactgttatgacaagtgcaacttggccagatactgtacgtcaactagcactttcttatttgaaagatcctatgattgtttatgttggtaatctgaatctagtggctgtaaatacagtgaagcaaaatataattgttaccacagaaaaagaaaaacgagctctcacccaagaattcgtagagaacatgtcacccaacgacaaagtcatcatgtttgtcagccaaaaacatattgctgatgacttgtcaagcgacttcaatatccaaggcatatctgcagaatcattacatggcaacagtgaacagagtgatcaagagcgagcagtagaggactttaaaagcggaaacataaagatactgattacaactgatatagtatcccgaggtcttgatcttaatgatgtcacacatgtatataattatgatttcccaaggaatattgacgtatatgtacacagagtagggtacattggacggacaggaaagactggcacatcagttaccctcatcactcagagagattcgaaaatggccggtgaattgattaaaattctggacagagcaaatcagagtgttccggaagatcttgtagtaatggctgagcaatacaagttaaatcaacaaaagaggcacagagaaacacgatcaagaaaacctggacaaagacgcaaggagttttattttttaagttga

SEQ ID NO: 89 - DNA, 3973 bp, synthetic construct
  source 1..3973: mol_type = other DNA
ggcctaactggccggtacctgagtctaaatgagtcttcggacctcgcgggggccgcttaagcggtggttagggtttgtctgacgcggggggagggggaaggaacgaaacactctcattcggaggcggctcggggtttggtcttggtggccacgggcacgcagaagagcgccgcgatcctcttaagcacccccccgccctccgtggaggcgggggtttggtcggcgggtggtaactggcgggccgctgactcgggcgggtcgcgcgccccagagtgtgaccttttcggtctgctcgcagacccccgggcggcgccgccgcggcggcgacgggctcgctgggtcctaggctccatggggaccgtatacgtggacaggctctggagcatccgcacgactgcggtgatattaccggagaccttctgcgggacgagccgggtcacgcggctgacgcggagcgtccgttgggcgacaaacaccaggacggggcacaggtacactatcttgtcacccggaggcgcgagggactgcaggagcttcagggagtggcgcagctgcttcatccccgtggcccgttgctcgcgtttgctggcggtgtccccggaagaaatatatttgcatgtctttagttctatgatgacacaaaccccgcccagcgtcttgtcattggcgaagtcgaacacgcagatgcagtcggggcggcgcggtcccaggtccacttcgcatattaaggtgacgcgtgtggcctcgaacaccgagcgaccctgcagcgacccgcttaaaagcttggcaatccggtactgttggtaaagccaccatggtcttcacactcgaagatttcgttggggactgggaacagacagccgcctacaacctggaccaagtccttgaacagggaggtgtgtccagtttgctgcagaatctcgccgtgtccgtaactccgatccaaaggattgtccggagcggtgaaaatgccctgaagatcgacatccatgtcatcatcccgtatgaaggtctgagcgccgaccaaatggcccagatcgaagaggtgtttaaggtggtgtaccctgtggatgatcatcactttaaggtgatcctgccctatggcacactggtaatcgacggggttacgccgaacatgctgaactatttcggacggccgtatgaaggcatcgccgtgttcgacggcaaaaagatcactgtaacagggaccctgtggaacggcaacaaaattatcgacgagcgcctgatcacccccgacggctccatgctgttccgagtaaccatcaacagtgggagttccggtggtggcgggagcggaggtggaggcatggcggccgacaagggcccggcggctggacctcggtcgcgagctgccatggcccagtggaggaagaagaaagggctccggaagcgccgaggcgcggcctcccaggcccgcggcagcgactcggaggacggcgagtttgagatccaggcggaagatgacgcccgggcccggaagctgggacctggaagacccctgcccaccttccccacctcggaatgcacctcggatgtggagccggacacccgggagatggtgcgtgcccagaacaagaagaagaagaagtctggaggcttccagtccatgggcctgagctacccggtgttcaaaggcatcatgaagaaggggtacaaggtgccaacacccatccagaggaagaccatcccggtgatcttggatggcaaggacgtggtggccatggcccggacgggcagtggcaagacagcctgcttcctcctcccaatgttcgagcggctcaagacccacagtgcccagaccggggcccgcgccctcatcctctcgccgacccgagagctggccctgcagaccctgaagttcactaaggagctaggcaagttcactggcctcaagactgccctgatcctgggtggagacaggatggaagaccagtttgcagccctgcacgaaaatcccgacataattattgccacgcccggacggttggtgcatgtggctgtggaaatgagcctgaagctgcagagtgtggaatacgtggtgttcgatgaagctgaccggctttttgaaatgggtttcgcagagcagctgcaggagatcatcgcccgcctccccgggggccaccagacggtgctgttctccgccacgctgcccaaactgctggtggaatttgcccgggctggcctcacggagcccgtgctcatccggcttgacgtggataccaagctcaacgagcagctgaagacctccttcttcctcgtgcgggaggacaccaaggctgccgtgctgctccacctgctgcacaacgtggtgcggccccaggaccagaccgtggtgtttgtggccacgaagcaccacgccgagtacctcactgagctgctgacgacccagcgggtgagctgcgcccacatctacagtgccctagacccgacagcccgcaagatcaatctcgccaaattcacgcttggcaagtgctccactctcattgtgactgacctggccgcccgaggcctggacatcccgctgctggacaatgtcatcaactacagcttccccgccaagggcaaactcttcctgcaccgcgtgggccgtgtggctcgggctggccgaagtggcacagcctactccttggtggcccctgatgaaatcccctacctgctggatctgcacctgttcctgggccgctccctcaccctcgcccgacccctcaaggagccctcaggtgtggccggtgtggatggcatgctgggtcgggtgccacagagtgtggtggacgaggaggacagtggtctgcagagcaccctggaggcatcgctggagctacggggcctggcccgcgttgctgataacgcccagcagcagtatgtgcgctcacgcccggcgccctcgcctgagtccatcaagagggccaaggagatggaccttgtggggctgggcctgcaccccctcttcagctcgcgttttgaggaggaggagctgcagcggctgaggctggtggacagcataaagaactaccgctcccgggcgactatctttgagatcaacgcctccagccgagacctgtgcagccaggtgatgcgcgccaagcggcagaaggaccgcaaggccatcgcccgcttccagcagggacagcaggggcggcaggagcagcaggagggcccagtgggcccagccccgagccgcccagcactgcaggagaagcagcctgagaaggaggaggaggaggaggcgggagagagtgtggaggacattttctcagaggtcgtgggccggaagcggcagcggtcaggacccaacaggggagccaagaggcggagggaggaggcccggcagcgggaccaggaattctacatcccctaccggcccaaggactttgacagcgagcggggcctgagcatcagcggggaagggggagcctttgagcagcaggcagctggcgctgtcctggacttgatgggggatgaagcccagaacctgacgaggggccggcagcagctcaagtgggaccgtaagaagaagcggtttgtgggacagtcaggacaggaagacaagaagaagattaagacagagagcggccgctacatcagcagctcctacaagcgagacctctatcagaagtggaaacagaaacagaaaattgatgatcgtgactcggacgaagaaggggcatctgaccggcgaggcccagagcgaagaggtgggaagcgagaccgtggccaaggtgcatcccggccccacgccccaggcacccctgcaggccgagtccgcccggaactcaagaccaagcagcagatcctgaagcagcggcgccgggcccagaagctgcacttcctgcagcgtggtggcctcaagcagctctctgcccgcaaccgccgccgcgtccaggagctgcagcagggcgccttcggccggggtgcccgctccaagaagggcaagatgcggaagaggatgtga

SEQ ID NO: 90 - DNA, 3130 bp, synthetic construct
  source 1..3130: mol_type = other DNA
ggcctaactggccggtacctgagtctaaatgagtcttcggacctcgcgggggccgcttaagcggtggttagggtttgtctgacgcggggggagggggaaggaacgaaacactctcattcggaggcggctcggggtttggtcttggtggccacgggcacgcagaagagcgccgcgatcctcttaagcacccccccgccctccgtggaggcgggggtttggtcggcgggtggtaactggcgggccgctgactcgggcgggtcgcgcgccccagagtgtgaccttttcggtctgctcgcagacccccgggcggcgccgccgcggcggcgacgggctcgctgggtcctaggctccatggggaccgtatacgtggacaggctctggagcatccgcacgactgcggtgatattaccggagaccttctgcgggacgagccgggtcacgcggctgacgcggagcgtccgttgggcgacaaacaccaggacggggcacaggtacactatcttgtcacccggaggcgcgagggactgcaggagcttcagggagtggcgcagctgcttcatccccgtggcccgttgctcgcgtttgctggcggtgtccccggaagaaatatatttgcatgtctttagttctatgatgacacaaaccccgcccagcgtcttgtcattggcgaagtcgaacacgcagatgcagtcggggcggcgcggtcccaggtccacttcgcatattaaggtgacgcgtgtggcctcgaacaccgagcgaccctgcagcgacccgcttaaaagcttggcaatccggtactgttggtaaagccaccatggtcttcacactcgaagatttcgttggggactgggaacagacagccgcctacaacctggaccaagtccttgaacagggaggtgtgtccagtttgctgcagaatctcgccgtgtccgtaactccgatccaaaggattgtccggagcggtgaaaatgccctgaagatcgacatccatgtcatcatcccgtatgaaggtctgagcgccgaccaaatggcccagatcgaagaggtgtttaaggtggtgtaccctgtggatgatcatcactttaaggtgatcctgccctatggcacactggtaatcgacggggttacgccgaacatgctgaactatttcggacggccgtatgaaggcatcgccgtgttcgacggcaaaaagatcactgtaacagggaccctgtggaacggcaacaaaattatcgacgagcgcctgatcacccccgacggctccatgctgttccgagtaaccatcaacagtgggagttccggtggtggcgggagcggaggtggaggcatggagcatgtgacagagggctcctgggagtcgctgcctgtgccgctgcacccgcaggtgctgggcgcgctgcgggagctgggcttcccgtacatgacgccggtgcagtccgcaaccatccctctgttcatgcgaaacaaagatgtcgctgcagaagcggtcacaggtagtggcaaaacactcgcttttgtcatccccatcctggaaattcttctgagaagagaagagaagttaaaaaagagtcaggttggagccataatcatcacccccactcgagagctggccattcaaatagacgaggtcctgtcgcatttcacgaagcacttccccgagttcagccagattctttggatcggaggcaggaatcctggagaagatgttgagaggtttaagcaacaaggtgggaacatcattgtggccactccaggccgcttggaggacatgttccggaggaaggccgaaggcttggatctggccagctgtgtgcgatccctggatgtcctggtgttggatgaggcagacagacttctggacatggggtttgaggcaagcatcaacaccattctggagtttttgccaaagcagaggagaacaggccttttctctgccactcagacgcaggaagtggagaacctggtgagagcgggcctccggaaccctgtccgggtctcagtgaaggagaagggcgtggcagccagcagtgcccagaagaccccctcccgcctggaaaactactacatggtatgcaaggcagatgagaaatttaatcagctggtccattttcttcgcaatcataagcaggagaaacacctggtcttcttcagcacctgtgcctgtgtggaatactatgggaaggctctggaagtgctggtgaagggcgtgaagattatgtgcattcacggaaagatgaaatataaacgcaataagatcttcatggagttccgcaaattgcaaagtgggattttagtgtgcactgatgtgatggcccggggaattgatattcctgaagtcaactgggttttgcagtatgaccctcccagcaatgcaagtgccttcgtgcatcgctgcggtcgcacagctcgcattggccacgggggcagcgctctggtgttcctcctgcccatggaagagtcatacatcaatttccttgcaattaaccaaaaatgccccctgcaggagatgaagccccagagaaacacagcggaccttctgccaaaactcaagtccatggccctggctgacagagctgtgtttgaaaagggcatgaaagcttttgtgtcatatgtccaagcttatgcaaagcatgaatgcaacctgattttcagattaaaggatcttgattttgccagccttgctcgaggttttgccctgctgaggatgcccaagatgccagaattgagaggaaagcagtttccagattttgtgcccgtggacgttaataccgacacgattccatttaaagataaaatcagagaaaagcagaggcagaaactcctggagcaacaaagaagagagaaaacagaaaatgaagggagaagaaaattcataaaaaataaagcttggtcaaagcagaaggccaaaaaagaaaagaagaaaaaaatgaatgagaaaaggaaaagggaagagggttctgatattgaagatgaggacatggaagaacttcttaatgacacaagactcttgaaaaaacttaagaaaggcaaaataactgaagaagaatttgagaagggcttgttgacaactggcaaaagaacaatcaagacagtggatttagggatctcagatttggaagatgactgctga

SEQ ID NO: 91 - DNA, 2971 bp, synthetic construct
  source 1..2971: mol_type = other DNA
ggcctaactggccggtacctgagtctaaatgagtcttcggacctcgcgggggccgcttaagcggtggttagggtttgtctgacgcggggggagggggaaggaacgaaacactctcattcggaggcggctcggggtttggtcttggtggccacgggcacgcagaagagcgccgcgatcctcttaagcacccccccgccctccgtggaggcgggggtttggtcggcgggtggtaactggcgggccgctgactcgggcgggtcgcgcgccccagagtgtgaccttttcggtctgctcgcagacccccgggcggcgccgccgcggcggcgacgggctcgctgggtcctaggctccatggggaccgtatacgtggacaggctctggagcatccgcacgactgcggtgatattaccggagaccttctgcgggacgagccgggtcacgcggctgacgcggagcgtccgttgggcgacaaacaccaggacggggcacaggtacactatcttgtcacccggaggcgcgagggactgcaggagcttcagggagtggcgcagctgcttcatccccgtggcccgttgctcgcgtttgctggcggtgtccccggaagaaatatatttgcatgtctttagttctatgatgacacaaaccccgcccagcgtcttgtcattggcgaagtcgaacacgcagatgcagtcggggcggcgcggtcccaggtccacttcgcatattaaggtgacgcgtgtggcctcgaacaccgagcgaccctgcagcgacccgcttaaaagcttggcaatccggtactgttggtaaagccaccatggtcttcacactcgaagatttcgttggggactgggaacagacagccgcctacaacctggaccaagtccttgaacagggaggtgtgtccagtttgctgcagaatctcgccgtgtccgtaactccgatccaaaggattgtccggagcggtgaaaatgccctgaagatcgacatccatgtcatcatcccgtatgaaggtctgagcgccgaccaaatggcccagatcgaagaggtgtttaaggtggtgtaccctgtggatgatcatcactttaaggtgatcctgccctatggcacactggtaatcgacggggttacgccgaacatgctgaactatttcggacggccgtatgaaggcatcgccgtgttcgacggcaaaaagatcactgtaacagggaccctgtggaacggcaacaaaattatcgacgagcgcctgatcacccccgacggctccatgctgttccgagtaaccatcaacagtgggagttccggtggtggcgggagcggaggtggaggcatggaggactctgaagcactgggcttcgaacacatgggcctcgatccccggctccttcaggctgtcaccgatctgggctggtcgcgacctacgctgatccaggagaaggccatcccactggccctagaagggaaggacctcctggctcgggcccgcacgggctccgggaagacggccgcttatgctattccgatgctgcagctgttgctccataggaaggcgacaggtccggtggtagaacaggcagtgagaggccttgttcttgttcctaccaaggagctggcacggcaagcacagtccatgattcagcagctggctacctactgtgctcgggatgtccgagtggccaatgtctcagctgctgaagactcagtctctcagagagctgtgctgatggagaagccagatgtggtagtagggaccccatctcgcatattaagccacttgcagcaagacagcctgaaacttcgtgactccctggagcttttggtggtggacgaagctgaccttcttttttcctttggctttgaagaagagctcaagagtctcctctgtcacttgccccggatttaccaggcttttctcatgtcagctacttttaacgaggacgtacaagcactcaaggagctgatattacataacccggttacccttaagttacaggagtcccagctgcctgggccagaccagttacagcagtttcaggtggtctgtgagactgaggaagacaaattcctcctgctgtatgccctgctcaagctgtcattgattcggggcaagtctctgctctttgtcaacactctagaacggagttaccggctacgcctgttcttggaacagttcagcatccccacctgtgtgctcaatggagagcttccactgcgctccaggtgccacatcatctcacagttcaaccaaggcttctacgactgtgtcatagcaactgatgctgaagtcctgggggccccagtcaagggcaagcgtcggggccgagggcccaaaggggacaaggcctctgatccggaagcaggtgtggcccggggcatagacttccaccatgtgtctgctgtgctcaactttgatcttcccccaacccctgaggcctacatccatcgagctggcaggacagcacgcgctaacaacccaggcatagtcttaacctttgtgcttcccacggagcagttccacttaggcaagattgaggagcttctcagtggagagaacaggggccccattctgctcccctaccagttccggatggaggagatcgagggcttccgctatcgctgcagggatgccatgcgctcagtgactaagcaggccattcgggaggcaagattgaaggagatcaaggaagagcttctgcattctgagaagcttaagacatactttgaagacaaccctagggacctccagctgctgcggcatgacctacctttgcaccccgcagtggtgaagccccacctgggccatgttcctgactacctggttcctcctgctctccgtggcctggtgcgccctcacaagaagcggaagaagctgtcttcctcttgtaggaaggccaagagagcaaagtcccagaacccactgcgcagcttcaagcacaaaggaaagaaattcagacccacagccaagccctcctga

SEQ ID NO: 92 - DNA, 3970 bp, synthetic construct
  source 1..3970: mol_type = other DNA
ggcctaactggccggtacctgagtctaaatgagtcttcggacctcgcgggggccgcttaagcggtggttagggtttgtctgacgcggggggagggggaaggaacgaaacactctcattcggaggcggctcggggtttggtcttggtggccacgggcacgcagaagagcgccgcgatcctcttaagcacccccccgccctccgtggaggcgggggtttggtcggcgggtggtaactggcgggccgctgactcgggcgggtcgcgcgccccagagtgtgaccttttcggtctgctcgcagacccccgggcggcgccgccgcggcggcgacgggctcgctgggtcctaggctccatggggaccgtatacgtggacaggctctggagcatccgcacgactgcggtgatattaccggagaccttctgcgggacgagccgggtcacgcggctgacgcggagcgtccgttgggcgacaaacaccaggacggggcacaggtacactatcttgtcacccggaggcgcgagggactgcaggagcttcagggagtggcgcagctgcttcatccccgtggcccgttgctcgcgtttgctggcggtgtccccggaagaaatatatttgcatgtctttagttctatgatgacacaaaccccgcccagcgtcttgtcattggcgaagtcgaacacgcagatgcagtcggggcggcgcggtcccaggtccacttcgcatattaaggtgacgcgtgtggcctcgaacaccgagcgaccctgcagcgacccgcttaaaagcttggcaatccggtactgttggtaaagccaccatggtcttcacactcgaagatttcgttggggactgggaacagacagccgcctacaacctggaccaagtccttgaacagggaggtgtgtccagtttgctgcagaatctcgccgtgtccgtaactccgatccaaaggattgtccggagcggtgaaaatgccctgaagatcgacatccatgtcatcatcccgtatgaaggtctgagcgccgaccaaatggcccagatcgaagaggtgtttaaggtggtgtaccctgtggatgatcatcactttaaggtgatcctgccctatggcacactggtaatcgacggggttacgccgaacatgctgaactatttcggacggccgtatgaaggcatcgccgtgttcgacggcaaaaagatcactgtaacagggaccctgtggaacggcaacaaaattatcgacgagcgcctgatcacccccgacggctccatgctgttccgagtaaccatcaacagtgggagttccggtggtggcgggagcggaggtggaggcatgaccaccgagcagcgacgcagcctgcaagccttccaggattatatccggaagaccctggaccctacctacatcctgagctacatggccccctggtttagggagggttattctggactttatgaagccattgaaagttgggatttcaaaaaaattgaaaagttggaggagtatagattacttttaaaacgtttacaaccagaatttaaaaccagaattatcccaaccgatatcatttctgatctgtctgaatgtttaattaatcaggaatgtgaagaaattctacagatttgctctactaaggggatgatggcaggtgcagagaaattggtggaatgccttctcagatcagacaaggaaaactggcccaaaactttgaaacttgctttggagaaagaaaggaacaagttcagtgaactgtggattgtagagaaaggtataaaagatgttgaaacagaagatcttgaggataagatggaaacttctgacatacagattttctaccaagaagatccagaatgccagaatcttagtgagaattcatgtccaccttcagaagtgtctgatacaaacttgtacagcccatttaaaccaagaaattaccaattagagcttgctttgcctgctatgaaaggaaaaaacacaataatatgtgctcctacaggttgtggaaaaacctttgtttcactgcttatatgtgaacatcatcttaaaaaattcccacaaggacaaaaggggaaagttgtcttttttgcgaatcagatcccagtgtatgaacagcagaaatctgtattctcaaaatactttgaaagacatgggtatagagttacaggcatttctggagcaacagctgagaatgtcccagtggaacagattgttgagaacaatgacatcatcattttaactccacagattcttgtgaacaaccttaaaaagggaacgattccatcactatccatctttactttgatgatatttgatgaatgccacaacactagtaaacaacacccgtacaatatgatcatgtttaattatctagatcagaaacttggaggatcttcaggcccactgccccaggtcattgggctgactgcctcggttggtgttggggatgccaaaaacacagatgaagccttggattatatctgcaagctgtgtgcttctcttgatgcgtcagtgatagcaacagtcaaacacaatctggaggaactggagcaagttgtttataagccccagaagtttttcaggaaagtggaatcacggattagcgacaaatttaaatacatcatagctcagctgatgagggacacagagagtctggcaaagagaatctgcaaagacctcgaaaacttatctcaaattcaaaatagggaatttggaacacagaaatatgaacaatggattgttacagttcagaaagcatgcatggtgttccagatgccagacaaagatgaagagagcaggatttgtaaagccctgtttttatacacttcacatttgcggaaatataatgatgccctcattatcagtgagcatgcacgaatgaaagatgctctggattacttgaaagacttcttcagcaatgtccgagcagcaggattcgatgagattgagcaagatcttactcagagatttgaagaaaagctgcaggaactagaaagtgtttccagggatcccagcaatgagaatcctaaacttgaagacctctgcttcatcttacaagaagagtaccacttaaacccagagacaataacaattctctttgtgaaaaccagagcacttgtggacgctttaaaaaattggattgaaggaaatcctaaactcagttttctaaaacctggcatattgactggacgtggcaaaacaaatcagaacacaggaatgaccctcccggcacagaagtgtatattggatgcattcaaagccagtggagatcacaatattctgattgccacctcagttgctgatgaaggcattgacattgcacagtgcaatcttgtcatcctttatgagtatgtgggcaatgtcatcaaaatgatccaaaccagaggcagaggaagagcaagaggtagcaagtgcttccttctgactagtaatgctggtgtaattgaaaaagaacaaataaacatgtacaaagaaaaaatgatgaatgactctattttacgccttcagacatgggacgaagcagtatttagggaaaagattctgcatatacagactcatgaaaaattcatcagagatagtcaagaaaaaccaaaacctgtacctgataaggaaaataaaaaactgctctgcagaaagtgcaaagccttggcatgttacacagctgacgtaagagtgatagaggaatgccattacactgtgcttggagatgcttttaaggaatgctttgtgagtagaccacatcccaagccaaagcagttttcaagttttgaaaaaagagcaaagatattctgtgcccgacagaactgcagccatgactggggaatccatgtgaagtacaagacatttgagattccagttataaaaattgaaagttttgtggtggaggatattgcaactggagttcagacactgtactcgaagtggaaggactttcattttgagaagataccatttgatccagcagaaatgtccaaatga

SEQ ID NO: 93 - DNA, 3187 bp, synthetic construct
  source 1..3187: mol_type = other DNA
ggcctaactggccggtacctgagtctaaatgagtcttcggacctcgcgggggccgcttaagcggtggttagggtttgtctgacgcggggggagggggaaggaacgaaacactctcattcggaggcggctcggggtttggtcttggtggccacgggcacgcagaagagcgccgcgatcctcttaagcacccccccgccctccgtggaggcgggggtttggtcggcgggtggtaactggcgggccgctgactcgggcgggtcgcgcgccccagagtgtgaccttttcggtctgctcgcagacccccgggcggcgccgccgcggcggcgacgggctcgctgggtcctaggctccatggggaccgtatacgtggacaggctctggagcatccgcacgactgcggtgatattaccggagaccttctgcgggacgagccgggtcacgcggctgacgcggagcgtccgttgggcgacaaacaccaggacggggcacaggtacactatcttgtcacccggaggcgcgagggactgcaggagcttcagggagtggcgcagctgcttcatccccgtggcccgttgctcgcgtttgctggcggtgtccccggaagaaatatatttgcatgtctttagttctatgatgacacaaaccccgcccagcgtcttgtcattggcgaagtcgaacacgcagatgcagtcggggcggcgcggtcccaggtccacttcgcatattaaggtgacgcgtgtggcctcgaacaccgagcgaccctgcagcgacccgcttaaaagcttggcaatccggtactgttggtaaagccaccatggtcttcacactcgaagatttcgttggggactgggaacagacagccgcctacaacctggaccaagtccttgaacagggaggtgtgtccagtttgctgcagaatctcgccgtgtccgtaactccgatccaaaggattgtccggagcggtgaaaatgccctgaagatcgacatccatgtcatcatcccgtatgaaggtctgagcgccgaccaaatggcccagatcgaagaggtgtttaaggtggtgtaccctgtggatgatcatcactttaaggtgatcctgccctatggcacactggtaatcgacggggttacgccgaacatgctgaactatttcggacggccgtatgaaggcatcgccgtgttcgacggcaaaaagatcactgtaacagggaccctgtggaacggcaacaaaattatcgacgagcgcctgatcacccccgacggctccatgctgttccgagtaaccatcaacagtgggagttccggtggtggcgggagcggaggtggaggcatgtttgttccaagatctctaaaaatcaagaggaatgctaatgatgatggcaaaagttgtgtggctaagataattaaaccagacccagaagaccttcagttggacaaaagcagagatgttcccgttgatgctgtagctacagaagcagccacaatagacaggcacatcagcgaatcatgccctttccccagcccaggtggccagttggcagaggttcattcagtaagtcccgagcagggtgcgaaggacagccatccttctgaagagcccgttaagtcattttccaaaacacagcgctgggcagaaccaggggaacccatctgtgttgtctgtggtcgttatggagagtatatctgtgataagacagatgaagatgtgtgtagtttggagtgtaaagcgaaacatcttctacaagttaaggaaaaggaagagaaatcaaaactcagcaatccacagaaggctgattctgagccagagtctccactgaatgcttcctatgtctacaaagagcacccctttattttgaaccttcaggaagaccagattgaaaatcttaaacagcagctgggaattttagttcaagggcaagaagtcaccaggcccattattgactttgaacattgtagtctccctgaggtcttaaatcacaacttgaagaaatcaggctatgaggtgccaactcccattcaaatgcagatgattcctgtgggacttctgggaagagacattctggccagtgcagatactggctcaggaaaaacagctgcttttcttcttcctgttatcatgcgagctttattcgagagcaaaactccatctgcgctcattcttacaccaaccagagagttagccattcagatagagagacaagctaaagaattgatgagtggcctgccacgcatgaaaactgtgcttcttgtagggggcttacccttacccccacagctttatcgtctgcaacaacatgttaaggttatcatagcaacccctgggcgacttctggatataataaagcagagctctgtagaactctgtggtgtaaagattgtggtagtagatgaagctgataccatgttaaagatgggttttcaacaacaagtgcttgacattttggaaaacattcctaatgattgtcagaccattttggtttcagccacaattccaactagcatagaacagctagcaagccagcttctgcataatcctgtgagaattatcactggagaaaagaacctaccttgtgccaatgtacgtcagattattttgtgggtagaagacccagccaaaaagaaaaaattatttgaaattttaaatgataagaaactctttaagcctccagtgttagtatttgtggactgcaaactaggagcagatcttttgagtgaagccgttcagaaaatcacagggctgaaaagcatatctatacattcagagaagtcgcaaatagaaaggaaaaacatattgaagggattacttgaaggagactatgaagttgtagtgagcacaggagtcttgggacgaggcctagacttgatcagtgtcaggctggttgtcaattttgatatgccttcaagtatggatgagtatgtccatcagattggaagagtaggaagattaggtcaaaatggaacagcgattactttcatcaataataattcaaaaagactcttctgggatattgcaaaacgagtaaagcccacaggatccattcttccccctcagttattaaattccccataccttcatgaccagaagagaaaggaacaacagaaagataaacagacacagaatgatctggttacaggagctaatcttatggatattatcagaaaacatgataaaagtaattctcagaaatga